European Patent Specification EP 3 887 512 B1, published January 14, 2026. Title: BIOCATALYTIC TECHNIQUES. Applicant: Hypha Discovery Ltd. UCL Business PLC. The sequence listing filed with the application follows.

SEQUENCE LISTING (257 sequences)

SEQ ID NO: 1 - DNA, 3195 bp, Streptomyces rimosus
atgaccgagacgatcccgttcgaagcagtcgacggcgcggtgcgcccgtccgaggaggtgccggtcgtcgacctgtcggccaccggcctcagcgacacccccctccagcaggccatgggcctggcccgcgagcacggcgcggtgtaccggcggcggctgcacggccatgaggcactgctcgtgtcctccctggagctggtcaccgaactggccgacgagaaccgcttcgccaagggcgtctcggtcgccctggagaacgtccgcgagttcgccggcgacggcctgttcaccgcgtacaacgacgaaccgaactgggccaaggcgcacgacatcctcatgccggccttcgccctcggctcgatgcgcacgtaccacccggcgatgctgaaggtcgcccgccgggtgatcggcagctgggaccggcgcgcggccgacggcacacccgtcgacgtccccgacgacatgacccggatgacgctcgacaccatcggcctggcgggcttcggcttcgacttcgagtccttctcccgcgcgaccatgcaccccttcgtcgaggcgatggtgcgttgcctggaatggagcatgaaacgcctcggccgggagccggacggcgactacaccgaggaggacgctgccttccgggccgacgcggactacctcgcctcggtcgtggacgaggtcatcgcctcccgtacgggtgcggacggcaccccgggcgaggaggcgggcgacgacctcctcggcctgatgctcggcgccacccaccccgccgacggcaccacgctcgacctcgccaacatccgcaaccaggtcatcaccttcctcatcgccggtcacgaaacgacctccggcgcgctgtccttcgccctgtaccacctgctcaaggacccggccgccctgcgcctggcgcagcgcgaggccgacgagctgtggggcgaccagaccgaccccgacccgtccttcgaggacatcggccgactgccctacacccgccaggtcctcaacgaggcgctgcgcctgtggcccaccgccgccgccttctcccgccaggcccgtacggacaccctgctcggcggccgcatcccactgaaggcgggccagctggtcaccgtcctcacgccgatgctgcaccgcgacccggcctggggcgacaacccggagctgttcgaccccacgcggttcgcgccggaggccgaggcggcccgctccccgcacgcgtacaagcccttcggtacgggcgagcgggcctgcatcggccgccagttcgcgctgcacgaggcgacgatgctgctcgccatgctggtgcaccgctaccgcctcatcgaccacagcgactaccgcctgagcatcaaggaaaccctgaccctcaagccggacggcttcaccctcaccctcgcccggcgcacccccgccgaccgcgcgggcctgcgcgccgccctcgccgtactgcccggcggagccgcggagccggacggcaccgagtccggtacggacgacggcctgccgacgcgggtccgccaggacaccgccctgctcctcctccacggcaccaactacggcacctgccgcgacttcgccgagcgcatcgccgacgaggccaccggcctcggcttcaccaccgaggtggccccgctggacgccgcgaccggcgcgctccccacggaccgcccggtcgtgatcgtcaccgcgtcctacaacggacagccgaccgatgacgcggcgcgcttcgtcgaatggctttccggcgacgaagcccgggccgaaggcgtcccctacgccgtcctcggcgtcggcgaccgcaactgggccgccacctaccagcgcgtgcccacgcttttggacgagcggctggccgccctcggcgccgagcggctcctcccgcgcggcgaggccgacgcatccggcgacctgaacggcgccgtcaaggcgttcacggccaccctgcgcaccgaactgctcgtacgctacggcgatcccgcgaccatcggcgcgagcacaccggccgacgccacggacgcgtcctacaccgtccgcgaggtcaccggcggccccctggacgcactcgccgcccgccacggcctccagccgatgaccgtcaccgaggcgtacgacctcaccgcccccggctacccgcgcgtcaagcgcttcctgcgcctcaccctccccgaaggcgttacgtaccgtacggccgaccacctcgccgtacttcccgccaacggcgcggcggcggtcgaacgcgccgcgcaggtgctgggcgtatcactggaagcggtcctcgacatccgcgcgggcgctggtcgcggcggccgggacacgctccccgtggaccgcccgctcacggtacgtcagctcctcacccaccacctggagctgaacgcccgaccgactgccgcgcaacgggcggtgctcgccgaccacaacccctgtccgcccgagcgtgccgccctccaggccatccccgacgacgacccgcgcaccaccctggacctcatcgaggaacacccggccctgcgcggtgtgctgccctggccggtactcctcgacctgctcccggccctgcgcatccgccactactccctctcgtcctcgcccgccgccgacccccgccacgccgacctgatggtctcgctgctccccggcggcaccggctccggccacctgcacacactgcggcccggcgacacggtcctggcccgggtccagccctgccgggaggcgttccgcctcgacccggccgacccgacaccggtcatcctggtagcggccggcaccggcctggcgcccttccggggcgcggtcgccgaccgcctggccgccacccaacttgcccctgctctgctctacttcggctgcgatgccctcgaagccgactacctgcacgccgaagaactccaggccgccgaggcagccggggccgtgtccctgcgccccgcgttcagcgcccgcccggtggacggctgccgttacgtccagcaccgcatcgccgccgaggcggaggaagtgggggcgctgctggacgccggagcccgggtgtacgtctgcggcgacggcaaccggatggccccgggcgtacgcgccgccttccgcgagctgtacgcggcccgtaccggcgccacgcaggaggaggccgaggtctggctgcgagagctcacggcggccggccggtatgtggaggatgtctatgtgacggggtaa

SEQ ID NO: 2 - protein, 1064 aa, Streptomyces rimosus
MTETIPFEAVDGAVRPSEEVPVVDLSATGLSDTPLQQAMGLAREHGAVYRRRLHGHEALLVSSLELVTELADENRFAKGVSVALENVREFAGDGLFTAYNDEPNWAKAHDILMPAFALGSMRTYHPAMLKVARRVIGSWDRRAADGTPVDVPDDMTRMTLDTIGLAGFGFDFESFSRATMHPFVEAMVRCLEWSMKRLGREPDGDYTEEDAAFRADADYLASVVDEVIASRTGADGTPGEEAGDDLLGLMLGATHPADGTTLDLANIRNQVITFLIAGHETTSGALSFALYHLLKDPAALRLAQREADELWGDQTDPDPSFEDIGRLPYTRQVLNEALRLWPTAAAFSRQARTDTLLGGRIPLKAGQLVTVLTPMLHRDPAWGDNPELFDPTRFAPEAEAARSPHAYKPFGTGERACIGRQFALHEATMLLAMLVHRYRLIDHSDYRLSIKETLTLKPDGFTLTLARRTPADRAGLRAALAVLPGGAAEPDGTESGTDDGLPTRVRQDTALLLLHGTNYGTCRDFAERIADEATGLGFTTEVAPLDAATGALPTDRPVVIVTASYNGQPTDDAARFVEWLSGDEARAEGVPYAVLGVGDRNWAATYQRVPTLLDERLAALGAERLLPRGEADASGDLNGAVKAFTATLRTELLVRYGDPATIGASTPADATDASYTVREVTGGPLDALAARHGLQPMTVTEAYDLTAPGYPRVKRFLRLTLPEGVTYRTADHLAVLPANGAAAVERAAQVLGVSLEAVLDIRAGAGRGGRDTLPVDRPLTVRQLLTHHLELNARPTAAQRAVLADHNPCPPERAALQAIPDDDPRTTLDLIEEHPALRGVLPWPVLLDLLPALRIRHYSLSSSPAADPRHADLMVSLLPGGTGSGHLHTLRPGDTVLARVQPCREAFRLDPADPTPVILVAAGTGLAPFRGAVADRLAATQLAPALLYFGCDALEADYLHAEELQAAEAAGAVSLRPAFSARPVDGCRYVQHRIAAEAEEVGALLDAGARVYVCGDGNRMAPGVRAAFRELYAARTGATQEEAEVWLRELTAAGRYVEDVYVTG

SEQ ID NO: 3 - DNA, 2013 bp, Streptomyces rimosus
atgaccggcgtatccgcccgcgaacccgcagcgggccgcaccgacgcctcccggtggctgctgcgccgccgggtgctgtcggaccccgcgctgcggctgatctgcttcccgcacgccgggggcgccgcgaccttcttccacgggtggcaggaccgggtaccggccggtaccgaggtcggcgcggtctgctatccggggcggcagaaccggatcgccgagccgccgctcacctccatggacgacctcgccgaccaggcgcacgcggcgctgcgcgggctgctcgaccgcccgctggcgctcttcgggcacagcatgggcgcggtcgtcgcgtatgaggtggccgtgcggctcgccgaacgcgacggcaccgcaccggtggccctgctggtgtccgggcacggcgccccgtatctgtgcgtggccgggccgccgccggacaccgcggcggacgaccgggagatcgccgagctggcgatggccgccgacccggcgctgcgcggctcgccccagctgctggacctggtcatgccggtgctccgcgccgaccacgcgctgctccgcgcctaccggcccgtacgcaccccgcggatcaccgcgccgatcgtcgcctaccgtggcgcggacgaccccagggcgagcgaggacgacatgtggtcctggcgcgcgatgaccggcgccgccttccggctccgtacgctgcccggcaaccacttctacctggccaccgaggaggccgggctggtggccgatgtcatggacgcctgtcggggcggtgcgaacggcgccgccggaagcaccgcgaccggcccggccaccgcctccgccgtaccgctgttcgtacgccgctccggcgcctgccccttcgacccggcggaggacttcgcccggctgcgcgccgagcggcccgtggtccgcaccaccttgccgaccggggcccgcgcctggatggtcacgcgctacgccgacgcccgccgcgtcatcgccgaccagcggcgcttcagctcccgggccgccgtgaacggcccggtgccgcccccggaaccgcccgaaggctttccgccgccgcggcccggcgtcttctacacgtacgagcccgaggagcacggccgcatccgccggatgctcaccccggagttcagcgcccagcgtgcccgcgtcctggagccgcgcgcggaaaccctggccgaccggcacctcgacgccatcgagcgggccgggccgcccgccgacctgatcgccgacttcgtgctgccggtgccccggctgctgttcctggaactgctgggcgtgcccctccaggacgccgggcgcctccaccacgacctggcgctcctgcacgacttccaccccatccacgaggcgcaggcgggagcgttccgccggctcgacgcgtacctgcgggaactggtggaaaccgcacgcgccacacccggcgacaacgtcctgggccacctggtcgccgcgcacggcgccgagctgagcgacgacgaactcgccggaatcgcctgccagttgctgctggccggatacgcgacgatcgccggcaccctgggcctgtccctgctcgccctgatcctcgaccccgtacaggcggagctggtgcgcgacgggcgcgcccggcccgaccggatggccgaggaactgatccgccacctgtcggtggtgaccttcggcaaggtcttccaggcgaaggaggacgtcacgatcgcggaccaggacatcgcggcgggcgagtacgtgctgtgccatctgccgtccgccaaccgcgatccggcgctggccgacggcctcgaccgcctcgacgtcacccgtgagccgacgccccacctcgccctcggccacggcgcgcaccactgcctgggcgccgaactggcccggatggaactgcgggtctgcgtgccccgtgtcctgcggcggctgccgggtctgcgcttgcgcgtccccgtcgaggagctgcgcttcacaccactgaacgccgcgtacggagtggaatccctgccggtcgcctggtaa

SEQ ID NO: 4 - protein, 670 aa, Streptomyces rimosus
MTGVSAREPAAGRTDASRWLLRRRVLSDPALRLICFPHAGGAATFFHGWQDRVPAGTEVGAVCYPGRQNRIAEPPLTSMDDLADQAHAALRGLLDRPLALFGHSMGAVVAYEVAVRLAERDGTAPVALLVSGHGAPYLCVAGPPPDTAADDREIAELAMAADPALRGSPQLLDLVMPVLRADHALLRAYRPVRTPRITAPIVAYRGADDPRASEDDMWSWRAMTGAAFRLRTLPGNHFYLATEEAGLVADVMDACRGGANGAAGSTATGPATASAVPLFVRRSGACPFDPAEDFARLRAERPVVRTTLPTGARAWMVTRYADARRVIADQRRFSSRAAVNGPVPPPEPPEGFPPPRPGVFYTYEPEEHGRIRRMLTPEFSAQRARVLEPRAETLADRHLDAIERAGPPADLIADFVLPVPRLLFLELLGVPLQDAGRLHHDLALLHDFHPIHEAQAGAFRRLDAYLRELVETARATPGDNVLGHLVAAHGAELSDDELAGIACQLLLAGYATIAGTLGLSLLALILDPVQAELVRDGRARPDRMAEELIRHLSVVTFGKVFQAKEDVTIADQDIAAGEYVLCHLPSANRDPALADGLDRLDVTREPTPHLALGHGAHHCLGAELARMELRVCVPRVLRRLPGLRLRVPVEELRFTPLNAAYGVESLPVAW

SEQ ID NO: 5 - DNA, 1483 bp, Streptomyces rimosus
atgccggacgagtcccagcaccagttcgaccacgcccgccgggcgggcttcggcccgtcggacgacatccgccggcagcgcgcccagggcgccctcgtccgggaagaggtggccccggcgcccggcgccgcacccgagcccatctggatggccctgagctacgaggccgtgcgccaggtcatgggcgaccacgtccgcttcagcaaccagcgccggttccgcgcccaggccatccgcggcgggagcaagcaccgcccgcaggagatgtccggccacctcatggactacgaccagcccgagcacacccggctgcgcaagatgctcacgccggagttcacggtccgccgcatccagcggctcaagccggtgaccgaggcgatcgcggaacgctgcctggacgccatggagcgcaaggggcggcccgccgacctcgtcgagctgtacgcgagcccgatctccggcgcggtgctgtgcgaactgctcggcgtgccccgcgacgaccggcgcgagttcctggtcaagcaccagtggcagctggagcaggaccgcagccgcaaggagcgcgccgcggctcaggcgtacacctccaactacctgcgcgcgctggtcaaacggcagcgcaaggaccccgacgagggcttcatcggccagctcatccgcgaccacggcgacaacttcgacgacgaggaactgatcggcatctgcggcctgatggtgctggccggcctggacaacgtcaacggcatgatcagcctcggtgtgctggccctcctggaacacccggaccagctcgccgtcctgctggcggaccccgagaacaccgtggaccgggtggtggacgaactgctgcgcttcctgtccgtggcgcacgcgccgaccccgcgcaccgccgtcgaggacgtggtcgtggccgggcagctgatcaaggcgggggaggaggtcgtctgctcgatcccgatggccaaccgcgacccggtactcgcccccgacgtcgaccggttcgacgtcaaccgcgagccgctgccgcacatcgccttcgggcacggcatccaccactgcatcggcgccgcgctcggccggatggaactgcgcaccgcctacctggcgctgtggcgccggttcccggacctgcggctggccgtgcccgccgaccaggtgccgcacaagacgaattccatcgcgtacggcctggagcgcctgccggtcgcctggtgacggcggcccggccacggcgcgcggcgcccgcggaagaggagggacgatggtcgaggtacgggtcgacgcggagatctgcgcggcgtccggcatgtgcacgctgctggtgcccgcggtcttcgaccagtcggaggaggacggcacggtggtgctcgccgatccggcgccgcccgcggaactggcggcgaaggtgcggacggcggcgctgcggtgcccggccggcgcgatctcggtgcacgagcgggaggcggacggcccgggtacgtaa

SEQ ID NO: 6 - protein, 404 aa, Streptomyces rimosus
MPDESQHQFDHARRAGFGPSDDIRRQRAQGALVREEVAPAPGAAPEPIWMALSYEAVRQVMGDHVRFSNQRRFRAQAIRGGSKHRPQEMSGHLMDYDQPEHTRLRKMLTPEFTVRRIQRLKPVTEAIAERCLDAMERKGRPADLVELYASPISGAVLCELLGVPRDDRREFLVKHQWQLEQDRSRKERAAAQAYTSNYLRALVKRQRKDPDEGFIGQLIRDHGDNFDDEELIGICGLMVLAGLDNVNGMISLGVLALLEHPDQLAVLLADPENTVDRVVDELLRFLSVAHAPTPRTAVEDVVVAGQLIKAGEEVVCSIPMANRDPVLAPDVDRFDVNREPLPHIAFGHGIHHCIGAALGRMELRTAYLALWRRFPDLRLAVPADQVPHKTNSIAYGLERLPVAW

SEQ ID NO: 7 - protein, 73 aa, Streptomyces rimosus
MVEVRVDAEICAASGMCTLLVPAVFDQSEEDGTVVLADPAPPAELAAKVRTAALRCPAGAISVHEREADGPGT

SEQ ID NO: 8 - DNA, 1368 bp, Streptomyces rimosus
atggcgagccgtacccgtatcgatacgcctggtcgtaacgagcaccggctgcacaccgtccccctgcgccatgtcctcggcggcctgcgggcgggtggtccgctggggctgatggaacgtaccgggcgccggtcgcagggcgcgctgacccggctggagctgggcgccttccggcccttcctggtcacccaccccgatcatctgcggcacgtcctgcgcgaccacggtgcgaactaccgccggggcaccgcgatgtggaaggcgatggggcggctgacggggatggggatcgcgggcgaggggccgcagtggcgggccagccgtgagctgtggtgccggggactgtcgggcggtgcgcacgtcttcgccgacgggacggccgacgcggtcgccggggcggtggcggacctggagcggcgggtggcggcgggcgcgacggtggacgcgctgacggagatgacccgtgtcgtgctccgggtcgtgaatccggcgttcttcggctcgcgcattccgcagggggagtgcgaccggctcgccgcggcggtcgccgtcgcgttcgactcgctgctgtggcgcatggcgctgcctttcgtaccgctcgccgtgccgttgccgggcgatcgcgccttcacccgcgccacccgtacggtcaacggcatcctgctgccgctgatccgccgggcacggcacgcgcaccaccgcggcccggacctgatgagcacgctgctcgacggggcggacgcggacggccgggcgctgggcgacgcgcatgtggcccaggacatcgtggccatgttcgtggcgggttcggagtccagcgccctgacgctgacgtgggcctgggtcgccctcgccgggcatgccgacatcgcggcggaggtgcgccgggaggccgacgcggtgctcggcggcgggccgccccggcccgagcacgcccgccggctggtgttcacccggagggtgctggccgaggtctgccgcctgtacgcgatggcgtgggcggtgccgcggacggccgtcgccgaggacgtcatcggcggggtgaccgttccggccggcgccacgctggtgctgtccccgtacctgacccaccggctgcccgccttctgggagcggccgctgcgcttcgaccccggccgtttcaccgacgagcgcgtacggggccggcacccgctggcgtacctgccgttcggcgacggaccccaccagtgcgtcggccagtcgttcttcttccagcaggcggccctcgtcgtggccacgatgatgagccgtttccgtatcgccgtgccgacgccggccgagcccagggccgcggtcgcgctgcgcccgcggagccgtgtcgatctggcgctcaccccgcgcggctaa

SEQ ID NO: 9 - protein, 455 aa, Streptomyces rimosus
MASRTRIDTPGRNEHRLHTVPLRHVLGGLRAGGPLGLMERTGRRSQGALTRLELGAFRPFLVTHPDHLRHVLRDHGANYRRGTAMWKAMGRLTGMGIAGEGPQWRASRELWCRGLSGGAHVFADGTADAVAGAVADLERRVAAGATVDALTEMTRVVLRVVNPAFFGSRIPQGECDRLAAAVAVAFDSLLWRMALPFVPLAVPLPGDRAFTRATRTVNGILLPLIRRARHAHHRGPDLMSTLLDGADADGRALGDAHVAQDIVAMFVAGSESSALTLTWAWVALAGHADIAAEVRREADAVLGGGPPRPEHARRLVFTRRVLAEVCRLYAMAWAVPRTAVAEDVIGGVTVPAGATLVLSPYLTHRLPAFWERPLRFDPGRFTDERVRGRHPLAYLPFGDGPHQCVGQSFFFQQAALVVATMMSRFRIAVPTPAEPRAAVALRPRSRVDLALTPRG

SEQ ID NO: 10 - DNA, 1483 bp, Streptomyces rimosus
atgtcgtacaacccgacggcccccgacaccaccgccgacggcaccaccggagaaccgcccaccctgcccaccgaccggcgcaccggctgccccttcgacccgcccggcgaactcaccgcgctgagcgaccggcccctgcgccgcatgcgctacgccgacgggcacataggctggctggccaccggccacgccgccgcccgcgcggtcctgtccgacccgcgcttcagctcccgctacgaactcctgcacctgccggtaccgatgccgggcatggaggggatgacggcggtgccgccggcgccgaccggcgacttcctcggcctcgacgcccccgagcacacccgctaccggcggctgctcaccggcaagttcacggtccgccggatgcgtcagctctccgaacgcgtggagcagttcacccacgagtgcctggacgccatggagcaggccgggcccaccgtcgacctggtggaggcgttcgcgcggccggtgcccgcgctcatgatctgcgaactgctcggcgtgccgtacgccgaccgggaccgcttccaggagcatgtggcgaccctcttcgaccaggccgcggacgcggaggcgaggggcgcggcgttcgccgccgtcggccgcttcatgggcgaactcgtggccgccaagcgcgccgagcccaccgacgacctgctcagcgacctgaccacctccgacctcacggaggaagagctgatcggggtcggcggggtgctcctggccgccggtctcgacaccaccgccaacatgctcgggctcggcaccttcgccctgctcagcaaccccgaccagctggacgccctgcgcgccgacccgggcctcgccgggcagaccgtcgaggagctgctgcgctacctcagcgtggccgaccccatcccgcgcgccgccctggaggacgtcgagatcgaaggccggctggtcagggccggtgagacggtgaccgtctcggtccaggccgccaaccgcgacccgctgaagttccccgaccccgaccggttcgacatccaccgcaaggccaccgggcacgtctccttcggccacggcccccaccagtgcctcggccagcagctcgcccgcgtcgagatgaccgtcgcgttcccggcgctcttcgcccgcttccccaccctgcgcctcgcggttccgccgcaggaggtgccgctgcgcgaccgcgccaacatctacggcgtgatcagcctgcccgtcacctgggacaaggagtaaccccatgagcgagccacaagagcggctgcgtctgagcgtcgaccgtgaccgctgcgtcggcgccgggatgtgcgccctgaccgctcccgaggtcttcgaccaggacgacgaagagggcctggtggtgctcaagcaccccgtaccggcccccggcagcctggccgccgcccggatggccgccggcctctgccccgccggagccatcaccctccactccccggaacccacggacccgtaa

SEQ ID NO: 11 - protein, 414 aa, Streptomyces rimosus
MSYNPTAPDTTADGTTGEPPTLPTDRRTGCPFDPPGELTALSDRPLRRMRYADGHIGWLATGHAAARAVLSDPRFSSRYELLHLPVPMPGMEGMTAVPPAPTGDFLGLDAPEHTRYRRLLTGKFTVRRMRQLSERVEQFTHECLDAMEQAGPTVDLVEAFARPVPALMICELLGVPYADRDRFQEHVATLFDQAADAEARGAAFAAVGRFMGELVAAKRAEPTDDLLSDLTTSDLTEEELIGVGGVLLAAGLDTTANMLGLGTFALLSNPDQLDALRADPGLAGQTVEELLRYLSVADPIPRAALEDVEIEGRLVRAGETVTVSVQAANRDPLKFPDPDRFDIHRKATGHVSFGHGPHQCLGQQLARVEMTVAFPALFARFPTLRLAVPPQEVPLRDRANIYGVISLPVTWDKE

SEQ ID NO: 12 - protein, 77 aa, Streptomyces rimosus
MSEPQERLRLSVDRDRCVGAGMCALTAPEVFDQDDEEGLVVLKHPVPAPGSLAAARMAAGLCPAGAITLHSPEPTDP

SEQ ID NO: 13 - DNA, 1230 bp, Streptomyces rimosus
atgagcgacccggccgcggtacgccgggccctgcgcgcgctgttcagcccgctgggctgccccgacccgtacccgcactacgcggtgctgcgggagcacgggccggtctcccggctgccggacggcaccgtcgtcgtcagccggcacgccgactgcgaccgcgtgctgcgcgatccgctcttccgggtcgaggacgacgcgtacctcgcccgtacctggcccgagggccgcgaccacctcagcgtcttctccctgatgggcgagatggtcaaccagaactcgccgcaccacgagcggctgcgccgcctggtgggccgcgccttcaccccgcgccgggtggccgggctgcggcccgcggtggagaagctggtcgacggcctgctggacggcctcgccgaacgggccgccgggggcgctccggtggatctgatggagcacttcgcgctgccgctgccgatcaccgtcatcggcgagctgctcggcatccccgaggaggaccgcgcctggttcgcgccgcgcgtgcaggccgtcacctccgcgatcgagcagaacctcgccggggaggcgctggagcgcgcggacgaggccaccgcggagctgtgggaccggctcggcgcgctggccgcccggcgccaggaggacccgcgcgccgacctggtcagcacgctcatcgcggtacgcgaggaggacggcgaccggctcacccggcgcgaactgctcgccaacctggtgctgctgtactccgccggctacgagaccaccagcaacctcatcggcaacggcacggccgtcctgctggaccgcccggacctgctcgcgcggctgcgcggcgagccggagcggatcgacgcctgggtcgaggagatgctgcgcttcgacccgcccatccagatcgcctcccgctgggcgggggaggacaccgagctgggcggggtggccgtggcgcagggctcccaagtggtggccctgctcgccagcgccaaccgcgatcctgcgcgccacggggacccggacgtcttccggccggaccgggcgccgggcggctcgctcaccttcggcgcgggcgcgcactactgcctgggcgccgcactggcccgcctggaggcggccatcgccttcccccggctgctggcccgcttcccctcgatcgcgcacgcgggcaccggggcgccgcgcaaccgtatgacgtccctgcgcggctacgccgagctgcccctgctcctgtcgtaa

SEQ ID NO: 14 - protein, 409 aa, Streptomyces rimosus
MSDPAAVRRALRALFSPLGCPDPYPHYAVLREHGPVSRLPDGTVVVSRHADCDRVLRDPLFRVEDDAYLARTWPEGRDHLSVFSLMGEMVNQNSPHHERLRRLVGRAFTPRRVAGLRPAVEKLVDGLLDGLAERAAGGAPVDLMEHFALPLPITVIGELLGIPEEDRAWFAPRVQAVTSAIEQNLAGEALERADEATAELWDRLGALAARRQEDPRADLVSTLIAVREEDGDRLTRRELLANLVLLYSAGYETTSNLIGNGTAVLLDRPDLLARLRGEPERIDAWVEEMLRFDPPIQIASRWAGEDTELGGVAVAQGSQVVALLASANRDPARHGDPDVFRPDRAPGGSLTFGAGAHYCLGAALARLEAAIAFPRLLARFPSIAHAGTGAPRNRMTSLRGYAELPLLLS

SEQ ID NO: 15 - DNA, 1260 bp, Streptomyces rimosus
atggacatcgatggcgcggagcccggcggcggcccttccggtgagtacggctcgtgtgtgcgcctcgacccggaagcgcgcgatccccgctcccgcccggacccgctgtgcgccgcgggccctgtggtgcccgtcctgctgccgggtggggtgacggcctggctggtgacccggcatcaggccgggaaggcggtgctggcggacggccgcttcgtcaaggacatcggggcctggcgcgcctggcgcggcggcgaggtcccgcgctcctggccgctggcgccgctgctgaccgtcgcgaacatgaccaccgcgacggcgggcgaccacacccggctgcgcgcgccgctggcccgcgcgttcaccgcgcgccgcgtggcggggctgcggccgcgcgtcgaggagctggccggggagctgctggacggcctcgccgccgaggggccggcgggccccgtcgagctgcgggcccgcttcgcccacccgctgccgatacgggtcatctgcgagctgttcggcgtgtccgacgaccgccgtccccggctgcagtcgctgtgccaggccctgttcgccgccccggcgggcccggccgatgccctggccacccaccgcgagctgcgggccgcgctcgccgatctgctccgcgccaagcgcgaggaccccggggacgacctgacgagcgcgctggtggcccccggccacggcctcagcgggagcgaactcgtcgacacgctgttgctgatgattgtcgcgggccatgagaccacggtgaacctgctggtcaacgcggtgtacgcgctgctgacccaccccggtcagctcactctcgtacgcggcgggcaggtgccctggagcgcggtggtcgaggagacgctgcgctgggacccgccggtcgccaacttcccgttccgctacgcgctgtgcgacgtggacctggccggccggaccattcgcgcgggcgatccggtgatgctgtcgtacgccgccttcggccgcgacccgcggcagcacgggcccggggccgaccgcttcgacgtcacccggccgcccacccgccatctggccttcgggcacggcatccaccactgcctcggtgcgccgctcgcccgcctggaggcggcggtcgccctccccgcgctgttcgaccgcttccccggcctcgccctggacgaccccgggcagcgtccgctccgccgcccgtccatggtcttcaacggcctgcgggagctgccggtcgtcctcggcccgcccggcggttcataa

SEQ ID NO: 16 - protein, 419 aa, Streptomyces rimosus
MDIDGAEPGGGPSGEYGSCVRLDPEARDPRSRPDPLCAAGPVVPVLLPGGVTAWLVTRHQAGKAVLADGRFVKDIGAWRAWRGGEVPRSWPLAPLLTVANMTTATAGDHTRLRAPLARAFTARRVAGLRPRVEELAGELLDGLAAEGPAGPVELRARFAHPLPIRVICELFGVSDDRRPRLQSLCQALFAAPAGPADALATHRELRAALADLLRAKREDPGDDLTSALVAPGHGLSGSELVDTLLLMIVAGHETTVNLLVNAVYALLTHPGQLTLVRGGQVPWSAVVEETLRWDPPVANFPFRYALCDVDLAGRTIRAGDPVMLSYAAFGRDPRQHGPGADRFDVTRPPTRHLAFGHGIHHCLGAPLARLEAAVALPALFDRFPGLALDDPGQRPLRRPSMVFNGLRELPVVLGPPGGS

SEQ ID NO: 17 - DNA, 1200 bp, Streptomyces rimosus
atggctgagtccacccacactgcccgcaccgcccacgccgtcccgccgctgcccaccgggccccgggccggctgccccttctccccgccgaaggaactgctcgacgcccgcgagcagggcccgatcggccactacacccaccccggcggcaagcccggctggatgatcaccgggtacgacatggtgcggtccgtgctcgccgacccgcggttcagctcgcgcaaggagctgatgaacgtggtcgatttcgagattccgccgccgccacccggcgagttcgtcctcatggacgacccgcagcaccggcgctaccgcaagccgctgatggggaagttcaccgtgcggcggatgcggctgctgaccgagcgcatcgagcaggtcaccgccgagtgcctggacgccatggagaaggcgggcccgccggtggacctggtggccgcgttcgccaagcccatccccgccatcgtgatctgcgagctgctgggcgtgccgtacgaggaccgcggcttcttccaggggcggatcgactcgttcatgaacggtgagacgagcgacgaggacctgatggcggcctacaccgaggtccagaactacctcgcggacctggtggccgccaagcgcgcgaaccccaccgacgacgtgctcagcgacctcaccgacaccgacctcaccgacgaggagttgaagggcatcagcctggtcctgctgacggccgggctcgacacgaccacgaatgtgctggggctgggcaccttcgcgctgttgcagcaccctgagcaactggccgcgctgcgcgccgatcccgcgcttgtcgacggagcggtggaggagctgctgcggtacctcagcgtcggcaagcagttctggcgtacggcgctggaggatgtcgagctgggcggtcagaccgtgaaggccggcacgacggtcgccctgtcgctcagcaccgccaaccgcgaccccgagcgcttcgccgaccccgatgtgctcgatctccggcggcagggcggcggacacctggccttcggtcacggcgttcaccagtgccttgggcagcaagtggcccgcatcgagctgcgggtggcgttctccgcgctgttcgaccgcttccccacgctgcgtctggccgtaccggccgaagaggtcgaactgcgtccggagtccgcggacgtcttcggggtgaagcgtcttccggtcgcctgg

SEQ ID NO: 18 - protein, 402 aa, Streptomyces rimosus
MAESTHTARTAHAVPPLPTGPRAGCPFSPPKELLDAREQGPIGHYTHPGGKPGWMITGYDMVRSVLADPRFSSRKELMNVVDFEIPPPPPGEFVLMDDPQHRRYRKPLMGKFTVRRMRLLTERIEQVTAECLDAMEKAGPPVDLVAAFAKPIPAIVICELLGVPYEDRGFFQGRIDSFMNGETSDEDLMAAYTEVQNYLADLVAAKRANPTDDVLSDLTDTDLTDEELKGISLVLLTAGLDTTTNVLGLGTFALLQHPEQLAALRADPALVDGAVEELLRYLSVGKQFWRTALEDVELGGQTVKAGTTVALSLSTANRDPERFADPDVLDLRRQGGGHLAFGHGVHQCLGQQVARIELRVAFSALFDRFPTLRLAVPAEEVELRPESADVFGVKRLPVAWDV

SEQ ID NO: 19 - DNA, 2743 bp, Streptomyces rimosus
atgaccccctctcccgcttcccccgccaccgccgccgcaccggcgcttcccgtgcagccgccgcagggctgcccgttcgacccgcccgccgagttcgcgcggctgcgcaccgaggcgccgctgtcgaagatctccctgccggacggcaccgaagcctggctcgccacccgctacgccgacatccgcgccatcctcggcgacacccgcttcagctccgacaccacccgccccggctacccgctcagcggcatgaccggcggcgccaccaccgaacaccgcggcttcatccgcatggacccgcccgagcacacccggctgcgccgcatggtcacccgggagttcatggtcaagcgcgtcgaggcgatgcgcccggagatccagcgcctgaccgacgaactgtgcgacgccatggagaagcgcgccggccaggacgtggacctcatcgaggcgctggccctgccggtgccgtcgctcgtcatcagcctgctgctcggcgttccgtacgacgatcacgagctgttccagcggctgaccggcaccctgctgtcccgtacggtcaccgacgcggagcgggagagcgcgcgggccgaactgcgcgcctacctgcaccagttggtgagcgccaaggaggccgcgcccggcgacgacatcctcggccgcctgatcgccgagcagcaggtaccgggcgagatcacccacgacgacgtggtcgccttcgccgccctgctgctcatcgcgggccacgagaccaccgccaacatgatcggcctgagcgcgctgaccctgatgcgcgaccgggagaccgcggaccggctgcgcgccgaacccgccctgatccgcggcgccgtcgaggaactgctgcgcttccacagcatcatccgcaacgggccgcgccgcgccgccaccgaggacatcgagatcggcgggcagctgatccgggccggggagggcgtcgtggtggccgtaccgtccgccaaccgcgacccggaggtcttcgcggaccccgacgcgctcgacgtctgccgccccaacgcccagcaccacgtcgccttcggctacggcatccaccagtgcctcggccaggccctggcccgcgtcgagctccaggtcgtcatcggcaccctgctgcgccgcttcccggagatgcggcccgcggtcccggtggacgagatcccgttccgcagcgacatggcgatctacggctgccacaccctgcccgtcacctggtgacaccccgcccgaccgttccccttcctcctcaggagtctcctgccatgaacatcaccctcgacgccgacaagtgctgcgccgcaggccagtgcgtactgatcgcccccgaggtcttcgaccagcgggacgaggacggcatcgtcgtcctcctggacgccgctccgcccgccgaccagcacgacgcggtccgcgaggccgccgccatctgtccggccgcggtcatcaaggtggacgagtgagcccccgccgcatcgccgtcgtgggcgcctcggcggcgggcctcgccgccgccgaggccctgcgccgcttcggctggaccggcaccctgaccctcgtcggcgacgagccccacccgccgtacgaccgtccgccgctgtccaagcagctccttcagggcgcctggcagcccgacaagctgcatctgcgcgccgccgaacagctcgacgcgctcggcctcgacctgcgcctgggcacccgggcgaccggcctggacaccgcgacccgcaccctgaccctggacggtggcgagcggctggcctgcgacggcgtgatcgtcgcgaccggcgtcgcggcccgcaccctcccggcggccgccgggctcgacggcgtgcacacgctgcgcaccctggacgacgcgctcgccctcaaggaacggctgtccggtaccggccatcgcctggtcgtcgtcggcaacggcgtactgggctgcgaggccgcggccgtggcccgcgagctgggtcacgaggtcacactcgtcgggcgcgaggcgctgccgatggcccgtacggtcggcacggagatcggcgagctgctggcggccgagcaccgggagcgcggcgtccagctgcgcaccgcggccgtcgacggcttcgaggcggacggggacgggcccgcgcggcacgtgagcgccgtacggctggccgacggcacccgcctgcccgccgacaccgtgctcgtcgccatcggctcggagcccgccgtcggctggctgcacggcgacccggccctggacaccaccgacggactgcgctgcgacgcgtactgcgccgccgcacccggcgtctacgcggccggtgacgtggcccgctggcagcacccggtacacggccgccacctgcgcgtcgagcaccggatgaacgccaccgagcagggcatggccgccgcccgcaacctcctagccgaactggaggagaccctgccgggggacgaggcactggcccccgccgcgggccgcgagcgccgccccttcacaccggtgccgtacttctggtccgaccagtacggcctgaagctccaggcgtacggcgtgctgtccggcgccgaccggtccgagacgaccgtcctggacccggacgccaggaaggccgtggccctctacggcagtgacggccaggccaccggcgtactggcgatcggtgtgccgccgcgccaggtccggggcctgcgggcgctgatcgccacgcccgtgccctgggaagaagctcgcgaggggctgcacaacgcccgcgcgtaa

SEQ ID NO: 20 - protein, 409 aa, Streptomyces rimosus
MTPSPASPATAAAPALPVQPPQGCPFDPPAEFARLRTEAPLSKISLPDGTEAWLATRYADIRAILGDTRFSSDTTRPGYPLSGMTGGATTEHRGFIRMDPPEHTRLRRMVTREFMVKRVEAMRPEIQRLTDELCDAMEKRAGQDVDLIEALALPVPSLVISLLLGVPYDDHELFQRLTGTLLSRTVTDAERESARAELRAYLHQLVSAKEAAPGDDILGRLIAEQQVPGEITHDDVVAFAALLLIAGHETTANMIGLSALTLMRDRETADRLRAEPALIRGAVEELLRFHSIIRNGPRRAATEDIEIGGQLIRAGEGVVVAVPSANRDPEVFADPDALDVCRPNAQHHVAFGYGIHQCLGQALARVELQVVIGTLLRRFPEMRPAVPVDEIPFRSDMAIYGCHTLPVTW

SEQ ID NO: 21 - protein, 64 aa, Streptomyces rimosus
MNITLDADKCCAAGQCVLIAPEVFDQRDEDGIVVLLDAAPPADQHDAVREAAAICPAAVIKVDE

SEQ ID NO: 22 - protein, 425 aa, Streptomyces rimosus
VSPRRIAVVGASAAGLAAAEALRRFGWTGTLTLVGDEPHPPYDRPPLSKQLLQGAWQPDKLHLRAAEQLDALGLDLRLGTRATGLDTATRTLTLDGGERLACDGVIVATGVAARTLPAAAGLDGVHTLRTLDDALALKERLSGTGHRLVVVGNGVLGCEAAAVARELGHEVTLVGREALPMARTVGTEIGELLAAEHRERGVQLRTAAVDGFEADGDGPARHVSAVRLADGTRLPADTVLVAIGSEPAVGWLHGDPALDTTDGLRCDAYCAAAPGVYAAGDVARWQHPVHGRHLRVEHRMNATEQGMAAARNLLAELEETLPGDEALAPAAGRERRPFTPVPYFWSDQYGLKLQAYGVLSGADRSETTVLDPDARKAVALYGSDGQATGVLAIGVPPRQVRGLRALIATPVPWEEAREGLHNARA

SEQ ID NO: 23 - DNA, 1374 bp, Streptomyces rimosus
atgaccctcaccacacgatccggcccggcgataccgggcccccggggcgtaccgttcctgggctcgatgttcgacctgcggcgcagcacgctcgacacgttcgcgcgcgcccgccgtgaccacggcgacctggtgcgcttcacggccggtccgcccggcctgcgcagcgtcttctacggcgtgttctcgcccgagggcagtcagcggatcctcgcctccgaggccgccaacttccgcaaggaccacccgttctacgaagaggtccggcagtcgttcggcaacggcctgctgaccagccaggacgacgactatctccgccagcggcggatcgtgcggccgctgttcaccaagcgccgggtcgacggctacgcgtcggccgtggccgcggatgcgcaggccgtcgccgagcgctggcggaccccgcccggcggcacggtcgacctggtgggcgagatgaaccggctcgcgctgcgcaccgtctcccgcatcctgttcggcacggacgtggaggccgcggtcgccaccgtgcaccgctgcttcccggtgatcaactcgtatgtcgtacggcgcggcttctcgccgcgcaacccgccgcgccactggcccacccccgccaaccgccgggccgccgccgcgacggccgaactgcactcggtctgcgaccggatcgtggccgggcggcagaccgccggcgcactggaggacggcgccgacctgctgtccctgctcacccgcgcgggcaacgcggcggacggcggcctggacgccaccgagatccgcgatcaggtcctggtcttcctgctcgccggccacgagacgaccgcgacgtccctggccttcaccctccacctgctcgcccggcatccggaggaacaggtcctggtacgggaggagatcgacgccgtactgggggaccgggagccggaagccgccgacctggagcggttgccgcggctgacgatggccctcaaggaggccatgcggctgtacccggcggcgcccgtggtgagccggcgcggcgtcgcggccaccgagatcggcggccaccggataccggacggcgccgatgtgatcgtctcgccgtgggtgacccaccggcaccccggcctgtgggaggacccggagcgcttcgatccgcggcggttcaccccggagcgggaggcggcgcgccaccgctacgcgtggttcccgttcggcggcggcccgcgggcgtgcatcgggcagcacttctcgatgctggagtcggtgctggcggcagcggtactgctgcgctcgtacgagctgacggcggtcgaccgggaggtgccgctcaccgcgggcatcaccttgcaggcggcgggcccggcgcgggtgcggctgaggggagtgggctaa

SEQ ID NO: 24 - protein, 457 aa, Streptomyces rimosus
MTLTTRSGPAIPGPRGVPFLGSMFDLRRSTLDTFARARRDHGDLVRFTAGPPGLRSVFYGVFSPEGSQRILASEAANFRKDHPFYEEVRQSFGNGLLTSQDDDYLRQRRIVRPLFTKRRVDGYASAVAADAQAVAERWRTPPGGTVDLVGEMNRLALRTVSRILFGTDVEAAVATVHRCFPVINSYVVRRGFSPRNPPRHWPTPANRRAAAATAELHSVCDRIVAGRQTAGALEDGADLLSLLTRAGNAADGGLDATEIRDQVLVFLLAGHETTATSLAFTLHLLARHPEEQVLVREEIDAVLGDREPEAADLERLPRLTMALKEAMRLYPAAPVVSRRGVAATEIGGHRIPDGADVIVSPWVTHRHPGLWEDPERFDPRRFTPEREAARHRYAWFPFGGGPRACIGQHFSMLESVLAAAVLLRSYELTAVDREVPLTAGITLQAAGPARVRLRGVG

SEQ ID NO: 25 - DNA, 1540 bp, Streptomyces rimosus
atgacgcacaccgaaccggccgcgccggccacctgcccggtcacgggagcgacggccggggccacggacacgacggattcgaccgggcacggaacggacccgctggtcgtcgactttccgctgcgcgcgcccggcatacccttcccgccgcccgaatacgccgattaccgcgacaagaaggggctggtgctctcgcacctgcccgacggcaaacgggtgtggctggtcacccggcacgaggacgtacgcgccgtcctgaccaacccggccatcagctccaacccccagcacccgggctttcccaatgtcggcgagacgatcggcgtacccaggcaggaccagatacccggctggttcgtgggaatggactcgcccgaacacgaccggttccgcaaggccctcatcccggagttcaccgtgcggcgcgtccgcgcgatgaaacccgcgatcgagcgcacggtggacgcgcaactggacgcgatgctggccgcgggcaacaccgccgacctcgtcgccgacttcaccctgcccattccctccctggtgatctcggcactgctcggcgtgccgcccgccgaccgcgagttcttcgaatccaggacccgcgtcctggtctcgttccgtgcgtactccgacgaggaccgcctggccgccggcaaggacctcatgcggtacatcaaccggctgatcgagatcaagaagaactggggcggcgacgacatcgtcacccggctgctggccaccggcgccatcggtgcccacgaaatgtccggcgtactgatgctgctgctcatcgccggccacgagaccacggccaacaacatcgcgctcggtgtggtcaccctgctgaagaatccccagtggatcggtgacgaacgggccgtcgaggaaaccctgcgcttccactcggtcgccgacctggtgtccctgcgggtggccgtcgaggacgtggagatcgccgggcagcacatcaaggcgggcgagggcatcgtgccgctggtcgccgccgccaatcacgacgaggaactcttcgcgtgcccccacgcgttcgacccctcccgctccgcccgcggccatgtggccttcggctacggcgtacaccagtgcctggggcagaacctggtacgggtcgagatggaggtcgcgtaccgcaagctcttcgagcgcattcccaacctccggctcgacgtgcccgaggacggactgaacatcaagtacgacggcgtgctctacggcctgcacgagctgcccgtccgctggtgacctgaccagagaacccgcgcccgcccggcggcacgcctcaccggccgccgggcggcccccatccaccgcaggagagaaacccgacatgcgtatcaccgttgactccgaccgctgcgtcggggcgggccagtgcgtactgaacgcgcccgcggtcttcgaccaggacgacgacgggctcgtcacccttctcgccgagcccggcgccgaccaggaggccgccgccaaactggccggtgccctgtgcccgtccggggccatcaccgtgcacgagggctaa

SEQ ID NO: 26 - protein, 420 aa, Streptomyces rimosus
MTHTEPAAPATCPVTGATAGATDTTDSTGHGTDPLVVDFPLRAPGIPFPPPEYADYRDKKGLVLSHLPDGKRVWLVTRHEDVRAVLTNPAISSNPQHPGFPNVGETIGVPRQDQIPGWFVGMDSPEHDRFRKALIPEFTVRRVRAMKPAIERTVDAQLDAMLAAGNTADLVADFTLPIPSLVISALLGVPPADREFFESRTRVLVSFRAYSDEDRLAAGKDLMRYINRLIEIKKNWGGDDIVTRLLATGAIGAHEMSGVLMLLLIAGHETTANNIALGVVTLLKNPQWIGDERAVEETLRFHSVADLVSLRVAVEDVEIAGQHIKAGEGIVPLVAAANHDEELFACPHAFDPSRSARGHVAFGYGVHQCLGQNLVRVEMEVAYRKLFERIPNLRLDVPEDGLNIKYDGVLYGLHELPVRW

SEQ ID NO: 27 - protein, 63 aa, Streptomyces rimosus
MRITVDSDRCVGAGQCVLNAPAVFDQDDDGLVTLLAEPGADQEAAAKLAGALCPSGAITVHEG

SEQ ID NO: 28 - DNA, 1432 bp, Streptomyces rimosus
atgaccgaggcgctgcccttcccgcaggaccggacctgtccctacgacccgcccgccggctaccagcccctgcgcgacagccgccccctgtcccgcgtgacgctctacgacgggcgccccgcctgggtggtgaccgggcacgccgaatcgcgggcgctgctcaccgacccgcgcctgtccgccgaccggcagaatccggcgttcccctcccccgccccgcgcttcgagacgctgcgcaaggtgcggaccccgctgctgggcgtcgacgaccccgaacacaacacccagcgccggatgctgataccgagcttcagcgtcaagcgcgccgccgcgctgcgcccccgcatccaggagatcgtggaccggctgctggacgccatggagcagcagggcccgcccgccgagctggtgtccgccttcgcgctgccggtgccgtccatggtgatctgcgcgctcctcggcgtcccgtacgccgaccacgagctgttcgagggcctgtcccggacgctcctgcagagcgccgacccgcaggaggtcaccgaggcccgcgacaagctggaggactacttcaccgccctggtggagcgcaaacggaaggagccgggcgacggcctgctggacgagctgatcgccgagcggctggactccggcgagctgggccaccgcgaactggtccggatggccatgctgctgctggtggccggccacgagaccacctccaacatgctgtccctgggcaccttcacgctgctggaacaccccgagcagttcgccgccctgcgcgccgacccgtcgctgctcccggccgcggtcgaggagctgctgaggttcctgtccatcgccgacggcatggtgcgggtggcgaccgaggacatcgagatcggcggcgtgacgatccgggcggacgacggcgtgatcttctccacctcggtcgtcaaccgggacggcgccgcctacgcctcgccggacaccctggactgggagcgctccgcccgccaccacgtcgccttcggcttcggcgtccaccagtgcctgggccagaacctggcccgcgcggagatggagatcgccttcggggcgctcttcgcccgcttccccggtctgcgcctggcggtgcccgccgccgagatacccgtcaaacccgcccacgccctccagggcctggtcgaactgcccgtcacctggtagcggcggaccgccgcccacaccctgtacccgtcaacggaggagagccaccatgaagatcgacatcgatacgtccgtgtgcatcggctcgggccagtgcgtgctgaccgcgccgggggtgttcacccaggacgacgacggtttcagcaccctgctgcccggccgcgaggacggcacgggcgacccgctcgtacgcgaggccgcccgcgcttgtccggttcaggcgatcgcggtcacggacgactaa

SEQ ID NO: 29 - protein, 395 aa, Streptomyces rimosus
MTEALPFPQDRTCPYDPPAGYQPLRDSRPLSRVTLYDGRPAWVVTGHAESRALLTDPRLSADRQNPAFPSPAPRFETLRKVRTPLLGVDDPEHNTQRRMLIPSFSVKRAAALRPRIQEIVDRLLDAMEQQGPPAELVSAFALPVPSMVICALLGVPYADHELFEGLSRTLLQSADPQEVTEARDKLEDYFTALVERKRKEPGDGLLDELIAERLDSGELGHRELVRMAMLLLVAGHETTSNMLSLGTFTLLEHPEQFAALRADPSLLPAAVEELLRFLSIADGMVRVATEDIEIGGVTIRADDGVIFSTSVVNRDGAAYASPDTLDWERSARHHVAFGFGVHQCLGQNLARAEMEIAFGALFARFPGLRLAVPAAEIPVKPAHALQGLVELPVTW

SEQ ID NO: 30 - protein, 64 aa, Streptomyces rimosus
MKIDIDTSVCIGSGQCVLTAPGVFTQDDDGFSTLLPGREDGTGDPLVREAARACPVQAIAVTDD

SEQ ID NO: 31 - DNA, 1200 bp, Streptomyces rimosus
atgaccgcggccgcgcaggaactggaaatcgcccgcgcctgcccctactccccgaatgcgcagcacatcgcattccagcagcagggccgccccgtcaaggtcaccctggcgaccttggggccgggtgcgccggtctgggcggtgagcaatcacgccgatatccgcaccatgctcaacgacgcccgattcagcgccgaccggcagcagcagggctttcccttccaggtcgacgggcagccgggcaacttccgccggacgatgatttccatggacggggcggaacaccgggaagtccgccgttccgtgaccggcgaattcaccctcaagcgcatgaaggccctgcagccgcggatccagcagatcgtggacgactgcatcgacaccatgctggccggtccgaaacccgctgacctggtcagcgcgctcgcgctccccgttccctcgctggtgatctgtgaacagctcggtgtgccctacgaaggccacgacttcttccagtcccggtcccacatgctgttgctacgcggcgcttcggcggaagagcggctgcgcgcgctggacgaactcatcgattttctcggcgacctcatcaccgagaaggaggccgagccgaccgacgacctgctcgggcgccagatcgtgaagctgcgcgaggcggggacgtaccgccaccaggacctggcgcgcatggcctttctgctgctggtcgccggacacgagaccaccgcgaacatgatttcgctgggcaccatggccctgctcgaccgccccgcggacgcggacgccctgcgcgcggacccgagcaagctcccggtcgcggtggaggaactcctgcggtacttcaccatcgccgagttcattcccacgcgcgtcgccaccgaggacgtggaactgggcggcagcctcatcaaggcgggcgatgtcctcgtggcgctgtgcaatgtggccaaccgcgacccctcggtgtttcccgacggcgacacactggacctgcaacgcggagcccgtcaccaactggcgttcggcttcggggctcatcagtgcctggggcagaatctcgcccgcatggaactggagatcgtctatgcgacgctgctccggcggataccgacgctgcgctccgcgataccgacccgtgaactgccgttcaagcacgacgcggacatctacggtatccacgcattcccggtcacctggtaa

SEQ ID NO: 32 - protein, 399 aa, Streptomyces rimosus
MTAAAQELEIARACPYSPNAQHIAFQQQGRPVKVTLATLGPGAPVWAVSNHADIRTMLNDARFSADRQQQGFPFQVDGQPGNFRRTMISMDGAEHREVRRSVTGEFTLKRMKALQPRIQQIVDDCIDTMLAGPKPADLVSALALPVPSLVICEQLGVPYEGHDFFQSRSHMLLLRGASAEERLRALDELIDFLGDLITEKEAEPTDDLLGRQIVKLREAGTYRHQDLARMAFLLLVAGHETTANMISLGTMALLDRPADADALRADPSKLPVAVEELLRYFTIAEFIPTRVATEDVELGGSLIKAGDVLVALCNVANRDPSVFPDGDTLDLQRGARHQLAFGFGAHQCLGQNLARMELEIVYATLLRRIPTLRSAIPTRELPFKHDADIYGIHAFPVTW

SEQ ID NO: 33 - DNA, 1433 bp, Streptomyces rimosus
atgaccgagacctccaccgccttcccggcccaagacgctcctgccttccccagcgaccgtacctgcccgtacgggctgcccgagacgtacgcacggttacgcgacagcgaggacgcgctgcgccccgtgaccctcttcgacggccgcaccgcctgggtcgtcaccaagcacgagaccgcccgcaccctgctcgccgacccgcggctctcctcgaaccgcacccaccccgacttccctctcacctccccgcgcctggcgggcctgcgcgatcgccgccccgccttcatcagcatggacccgcccgagcacgggccccggcgccggatgacgatcagcgaattcaccgtcaagcgcatcaagggcatgcgaccggacatcgagcgaatcgtgcacggcttcctcgacgagatgctcgccgcgggcccgcccgccgacctggtcagccggttcgcgctgccggtgccctccatggtgatctgccaactgctcggtgtcccctacgccgaccacgacttcttccaggacgccagtcggcgcctggtgcagtcgaccagcgcggaggaggcgaccggcgcgcgcgacgacctggaacgctacctggacgggctgatcaccaccctggagtccgagcccgggcccggactcctcggcgcgctggtcacccggcagctcgcggacggcgccatcgaccgcgacgaactgatctcgaacgcgctgctgctgctcgtcgccggccacgagaccaccgcctccatgacctccctgagcgtcatcaccctgctcgaacaccccgagcagcacgccgccctgcgcgacgatccgtccctgatcccgggcgcggtcgaggaactgctgcgctacctcgccatcgccgacgtggcgggcgcccgcgtcgccaccgccgacatcgaagtggacggacaggtcatccgggccggcgagggcgtgatcgtcgtccactccatcgccaaccgcgacgccggggtgttcgagaacccggacaccttcgacattcaccgctcggcccgccaccacctctccttcggctacggcgtccaccagtgcctcggccagaatctggcccgcctcgaactcgaaatcatcctgagcgcgctgttcgaacgcatccccacgctgcggctggccacaccggtcgagcgcttgaccctgcggcccggcagcaccatccagggcgtcaacgaactccccgtcacctggtgagcggggcgaagggagcgaccatgcacgtgaccgccgaccgcgacgtgtgcgtcggtgccgggatgtgcgccctgaccgcgcccggcgtcttcgaccaggacgacgacgggctcgtcaccgtcctgacctccgatatcggagagaacgaccgggacgccgtgcgcgaggccggcatgctgtgcccgtccggggcccttcgggtcacggagtaa

SEQ ID NO: 34 - protein, 406 aa, Streptomyces rimosus
MTETSTAFPAQDAPAFPSDRTCPYGLPETYARLRDSEDALRPVTLFDGRTAWVVTKHETARTLLADPRLSSNRTHPDFPLTSPRLAGLRDRRPAFISMDPPEHGPRRRMTISEFTVKRIKGMRPDIERIVHGFLDEMLAAGPPADLVSRFALPVPSMVICQLLGVPYADHDFFQDASRRLVQSTSAEEATGARDDLERYLDGLITTLESEPGPGLLGALVTRQLADGAIDRDELISNALLLLVAGHETTASMTSLSVITLLEHPEQHAALRDDPSLIPGAVEELLRYLAIADVAGARVATADIEVDGQVIRAGEGVIVVHSIANRDAGVFENPDTFDIHRSARHHLSFGYGVHQCLGQNLARLELEIILSALFERIPTLRLATPVERLTLRPGSTIQGVNELPVTW

SEQ ID NO: 35 - protein, 63 aa, Streptomyces rimosus
MHVTADRDVCVGAGMCALTAPGVFDQDDDGLVTVLTSDIGENDRDAVREAGMLCPSGALRVTE

SEQ ID NO: 36 - DNA, 1356 bp, Streptomyces rimosus
atggctgcacacgccgatgagccgatccgcctggcggtgggggaactggcacggtttctcggcgcggacgtcgacgaccccgcctttctgaccgatcctcacagatgtctgacgcccgggatacgcgagaaatccgtgcaccggctgcccggaggcgccctggccgttctcggttacacggcgtgcgccgaggtgctgcgtgatacacggttcggccacggtgcccgcgaactgtacgagaccaccctgctggggctgccggcccggtcttttctccaactggacgcaccggggcacacccggctgcgcggccaggtcgcgcggcatttcaccgcacggcgagtacgggccttggccgagaacgtcgggtattacagcactgctctcgtacgggagcacgcgggccgcccgggggatttcgtggcggatttcgccgagccgctggcgatgtcggtcatcagcgacgtactgggcgtgccgcccgaggatcgccccgccttccaccgtgacgcccggctggtcgtccgcggactggaccagccggcccgcgccatggacgaacgggccgtcgcccaggcgcggttccgcttcgtacggttcttccgccgccgggcgcaggcgcgccgccaggccgggacgcggcaccgggcgccccgggacggcctgctggacgccttgtcgcaccggccggacggcagcccggccgacatccgcgagctggtcaccacgtgcagcctgctgctgagcgccggatacgacaccacggtcagcctgctgtcgcacgcggtggcggaactgggcggcgcaccgtccgggcaggggtgggcgctggcccgggacccgcagacggtgggcgcggtcgtggaggaggtgctgcgtctgcactctcccgtgcagatcgctccgcgcgccgcggtgcgtgacgcggccctggacgggctgccggtggcccgcggcacgatcgtgctgcccctgctgccggcggccaaccgggacccggacatcttcgacagcccgcacaccttccggccccggcgctatctcgccccggcagctcaaggccgttcgacagcaaggcatttggcgttcggagcgggcgcgcatttctgtctgggggcggccctggcccggctgaccgcccacagcgcgctggctgttctggccgcctgcccgcccagaccgcgcgacgcgccccgtacgtacagcgaaggcgtcgtcgtacgcggcctgcgcagtctgccggtcacctggccgcaccggcccgcggaacggcccccgcaccctccggccgacggcgcggccgcgtacgtcgagccgtcgtgccccatcccccacgcgcaaaggagcgtcacataa

SEQ ID NO: 37 - protein, 451 aa, Streptomyces rimosus
MAAHADEPIRLAVGELARFLGADVDDPAFLTDPHRCLTPGIREKSVHRLPGGALAVLGYTACAEVLRDTRFGHGARELYETTLLGLPARSFLQLDAPGHTRLRGQVARHFTARRVRALAENVGYYSTALVREHAGRPGDFVADFAEPLAMSVISDVLGVPPEDRPAFHRDARLVVRGLDQPARAMDERAVAQARFRFVRFFRRRAQARRQAGTRHRAPRDGLLDALSHRPDGSPADIRELVTTCSLLLSAGYDTTVSLLSHAVAELGGAPSGQGWALARDPQTVGAVVEEVLRLHSPVQIAPRAAVRDAALDGLPVARGTIVLPLLPAANRDPDIFDSPHTFRPRRYLAPAAQGRSTARHLAFGAGAHFCLGAALARLTAHSALAVLAACPPRPRDAPRTYSEGVVVRGLRSLPVTWPHRPAERPPHPPADGAAAYVEPSCPIPHAQRSVT

SEQ ID NO: 38 - DNA, 1341 bp, Streptomyces rimosus
atgccgggcgccttgcccctcgtcgggcacgcgcccgcgctcattcgtgatcccttcggcttcttcctgtcgctgcgggaccacgccgacgaccgcggcctggtccgcatccggctcggctcgatgcccgtctacatggccaccacccctgagcggctgcacgaggtcctggtggacaaggggcggtggttcgagaagggccggttcttccagcgcctcaagcggctggccggcgaggggctgagcaccgcggacggggagctgcacaaacgtaaccgccgcttcctcgcgccccttttcggcgcgcagcgcatcaaggactactccctggtcatgagccgcaatgcccggcgcctgtcccagtcctggcagccggatcagcaggtggacatctacaaggaggccgccgcttattccatcgactccatcgccatgtcgctgttcagtacagacgtcggaacgccggcggtggaaacgatccgtaccgaactgccggtgctgctggacatgctcctcaagcgcgctgcctcaccgaagatcctggatcgcctgccggtacgctacaaccgcgttttcgaccgggcgtccgcgcagttgaccggggtgatcgaccaggtcatcaccaccgcacacgccggcggccacgccgaggagcacgacgacctgctcgcgcagctgctgcgggcgcaggtccacgacgacgttccggtccgcctcagtgacgttcagatccgcgacgaggtggccacgctgctgttcgccggggccgagaccacggcgtcgaccctggcctgggcctggcactacctggcgcaccaccccgaggtcgaccggcaggtggtggacgaggtcctggaggtcgtgggccccgaccgcgcggtgaccatcgaagacgtcccccggctgaccgtgatccgccgggtgctggacgaggtgatccgcctgcacggtgtcacgttcctgatgcgccgcagcaccgcgccggtgaccctcgccgatgtcacgctgcccgcgggcaccgaggtggcgttcagcatgtacgccatccaccgtgatcccgaggctttcgaggacccccacaccttcaacccggaccggtggctggaccccggggccaaacggtcgttcatgcccttcggcggcggcaaccgcaagtgcatcggcgatcagttcgccctggccgagaccaccatcgccgtcgcggaggtgctgcgcgactggcgcatgacccccgccggcggccacactccgcagcaggtgatctccgctgtcgcccggcccgaccgggtacccatgaccgtacggccgcgtaaccccgcacccagccggccgagcaactaa

SEQ ID NO: 39 - protein, 446 aa, Streptomyces rimosus
MPGALPLVGHAPALIRDPFGFFLSLRDHADDRGLVRIRLGSMPVYMATTPERLHEVLVDKGRWFEKGRFFQRLKRLAGEGLSTADGELHKRNRRFLAPLFGAQRIKDYSLVMSRNARRLSQSWQPDQQVDIYKEAAAYSIDSIAMSLFSTDVGTPAVETIRTELPVLLDMLLKRAASPKILDRLPVRYNRVFDRASAQLTGVIDQVITTAHAGGHAEEHDDLLAQLLRAQVHDDVPVRLSDVQIRDEVATLLFAGAETTASTLAWAWHYLAHHPEVDRQVVDEVLEVVGPDRAVTIEDVPRLTVIRRVLDEVIRLHGVTFLMRRSTAPVTLADVTLPAGTEVAFSMYAIHRDPEAFEDPHTFNPDRWLDPGAKRSFMPFGGGNRKCIGDQFALAETTIAVAEVLRDWRMTPAGGHTPQQVISAVARPDRVPMTVRPRNPAPSRPSN

SEQ ID NO: 40 - DNA, 1194 bp, Streptomyces rimosus
atgccggtccagctccccggcggcatccccggccacgccgtgacccgccaccacgccctgcgcgacttcctcacccacccggaagtggccaaggacgcctgccacttcgccgcgctgcgcgagggccgcatcccgcccggctggccgctcaccaccttcgcgaccgtggacgggatgacgacggccgacggcgcggaccaccggcggctgcgggaaccggccgtcaaggcgctctcgccccggcgggtggcggcgctgcggccgcgggtggagcggctgaccgccgagctgctcgacgggctgcccgccctggccgcgcggggcggcgggacggtcgatctccggcacgccttcgcctatccgctgcccatgcgggtgatcagtgaactcatcggcgtggacgaggagttccgggaccggctgcaccagctgtccgggctggtcgtgagcaccgtcatcgacccggaggcggcgctggcggccaaccgggagctggtcggggtcctcgggcaggtcgtggcggcccgccgcgcggcgccgggcgacgacctgaccagcgcgctcatcgcggcctgtgacgaggcggacgcccggctgagcgaacgggagctgatcggcaccctgttgctgatgatcgccgccgggcaccagaccaccctcgacttgatcaccaacgccgtacgggccctctgcgcccaccgcgaccagctggacctggtccgcgcggggcgggcggactgggcggacgtggtcgaggagacgctgcgccacgacagcccggtggcccacttcccgttccgctacccgacccgggacctggacgtcggcggcacggtgatcccccgggggacgccggtgctcgcctcgtacgcggcggccgggcgcgacccggaggcgtacgggccggacgcggaccgcttcgacgtgacgcgacggcccgccgtccggcacctgtccttcgggcacgggccgcatgtctgtccgggcgcaccgctggcccgcttggaggcgcggatcgccctgcgcgcgctgttcacccgcttccctgatctggccctggccgtaccggaggcggacctgcggccgctgcccacgttcgtgggcaacagcgtcgcggagcttccggtacggccgggtcgggacgtcgggacggccggtcaggacgcgtcggccaccagccccggcgccgggtaa

SEQ ID NO: 41 - protein, 397 aa, Streptomyces rimosus
MPVQLPGGIPGHAVTRHHALRDFLTHPEVAKDACHFAALREGRIPPGWPLTTFATVDGMTTADGADHRRLREPAVKALSPRRVAALRPRVERLTAELLDGLPALAARGGGTVDLRHAFAYPLPMRVISELIGVDEEFRDRLHQLSGLVVSTVIDPEAALAANRELVGVLGQVVAARRAAPGDDLTSALIAACDEADARLSERELIGTLLLMIAAGHQTTLDLITNAVRALCAHRDQLDLVRAGRADWADVVEETLRHDSPVAHFPFRYPTRDLDVGGTVIPRGTPVLASYAAAGRDPEAYGPDADRFDVTRRPAVRHLSFGHGPHVCPGAPLARLEARIALRALFTRFPDLALAVPEADLRPLPTFVGNSVAELPVRPGRDVGTAGQDASATSPGAG

SEQ ID NO: 42 - DNA, 1224 bp, Streptomyces rimosus
atgacgaccgttcccgatcttcccgacgccacagaggcgctggagcacttccccttcgacgacggccgtggcatcgaggtccacgagcggttccgggagctgcgggagcgcgcggggctgctccgggtgcggctcgactacggtgaacccacctggctggtcacccgttacgcggacgcccggctggtgctgggcgacgcgcggttcagccgtgccatgtcggtcggccgggacttcccgcgccaggaggaagcgacggaactggccgggctgatcaccatggacgcccccgaacacacccggctgcgcacactgttggtcaaagccctcagcaaatcccgtatcgacgcgcagcgcccgacggtgcgcgcgacggcggacgcgctgctgtcgtcggcgatggacgccgggccgggcatggacatcgtggtggactacgcgcagcagatgagcgtgctgtccatctgcgacctgctcggcgtgccggcctcggaccgggaggcgttcgagtcgaccagcgcggcactgctccccggcagcgccgtcggcgccgaggacatgatgcggcggttcggtgagctgcgcgcctgcaccgagcggctcatcgccgagcgccgggcccgcccccgcgacgacctgatgtcggcgatgatccaggcccgggacgaggaggaccggctcaccgacgccgagctgatcgagctggtcgtcagcatgctgctggccaggttcgaggcgatcatcacccagatcccgaactgcgtctacgttctcacgcggggcgaccgggcgctctggaaccggctgcgtgcgaatccggccgagctgcccgcggcggtcgaggagctgctgcgcaacaacgcctccgccggcgcgggcctgttcgtccgctatgcgcgggaggatgtcaacgtcggcggcacgctggtgcgcgcgggcgaagccctgaccatcgccgtcgagtcggccaaccacgacccggcccggttcgaggaccccgacgcgatcgatttcacccggccacccggcgggcacctcaccttcggttatggcgcgcactactgcgtcggcgcccagctcgggcgcatcgacctccaggaagggctgcgggtgctgctcaccagggccccggagctgaccgtccgcgacctcacgtggagagtacggccgcacatccggggaccggtggcgatgcgcgtgacctggcagggcgacccggaataa

SEQ ID NO: 43 - protein, 407 aa, Streptomyces rimosus
MTTVPDLPDATEALEHFPFDDGRGIEVHERFRELRERAGLLRVRLDYGEPTWLVTRYADARLVLGDARFSRAMSVGRDFPRQEEATELAGLITMDAPEHTRLRTLLVKALSKSRIDAQRPTVRATADALLSSAMDAGPGMDIVVDYAQQMSVLSICDLLGVPASDREAFESTSAALLPGSAVGAEDMMRRFGELRACTERLIAERRARPRDDLMSAMIQARDEEDRLTDAELIELVVSMLLARFEAIITQIPNCVYVLTRGDRALWNRLRANPAELPAAVEELLRNNASAGAGLFVRYAREDVNVGGTLVRAGEALTIAVESANHDPARFEDPDAIDFTRPPGGHLTFGYGAHYCVGAQLGRIDLQEGLRVLLTRAPELTVRDLTWRVRPHIRGPVAMRVTWQGDPE

SEQ ID NO: 44 - DNA, 1224 bp, Streptomyces rimosus
atgcagaacaccgccgagaccggccccgacgacctcattgacgtgacgcagcttctggacgatccgcacgccgggtacgcggtgttgcgggaggcggggcccgtccatcggattgccgggccggacgggcagcccgcgtggctggtgacgcggtacgaggatgtgcggcggtgtctgtccgatccgcggctttccctggacaagcggaacgcgcggggcggctatcgcgggttcgcgctgccgcccgcgctggacgcgaatctgctcaacatggatccgccggaccacacccgggtgcgccggctggtggccaaggcattcacgcccgcgcgggtcgagaagctgcgggagcccgtacggcggctggcggacgggttgctggacgcggtcgcggacgccgggcgggccgacctgatggagtgttacgccggtccgctgcccatcatcgtcatctgcgacctgctgggcgtaccggaggacgaccggccggacttccgggcctggacggacgcgctgatcacgcccgacccggcccggccggagcgggcgaaggaggccgtcggggcgatgatgcgctactacacggggctgatcacggccaagcgggccgcgccgggggacgatctgctctccgacctgatcctggtgcgggacggcgcggcggcggagggtggcgcgggggaccggctcggtgaggacgagctgacctcgttggcgttcctcctgctcttcgccggttacgagaacaccgttcacctcatcggtaactcagtcctcgccctgctcgaccaccccgaacacctcatggcgttgcgtacgaatccagccgaactgtcggcggccgtggaagagttcgcacgctatgacggaccggcctcgctggccatccgccggttccccctggaggacgtggaaatcggcggcgtacgggtgcccgcgggcgagagtgtgctgctctcccttgcctcggcgaaccgcgacccgcaccgcttcgccgaccccgggacgctcgatccgggccgcgacgccacgggtcagctgatgttcgggcacggcatccactactgcctcggcgcggccctggcgcgcctgcagaccgagaccgcgctgaccgctctcatcagccgttttcccgggttgcggctggatgtgccacggtcggaactgcgccaccgccgcaccctgcgggcacgtggcttgatctcgctccccgtcgcctggtaa

SEQ ID NO: 45 - protein, 407 aa, Streptomyces rimosus
MQNTAETGPDDLIDVTQLLDDPHAGYAVLREAGPVHRIAGPDGQPAWLVTRYEDVRRCLSDPRLSLDKRNARGGYRGFALPPALDANLLNMDPPDHTRVRRLVAKAFTPARVEKLREPVRRLADGLLDAVADAGRADLMECYAGPLPIIVICDLLGVPEDDRPDFRAWTDALITPDPARPERAKEAVGAMMRYYTGLITAKRAAPGDDLLSDLILVRDGAAAEGGAGDRLGEDELTSLAFLLLFAGYENTVHLIGNSVLALLDHPEHLMALRTNPAELSAAVEEFARYDGPASLAIRRFPLEDVEIGGVRVPAGESVLLSLASANRDPHRFADPGTLDPGRDATGQLMFGHGIHYCLGAALARLQTETALTALISRFPGLRLDVPRSELRHRRTLRARGLISLPVAW

SEQ ID NO: 46 - DNA, 1212 bp, Streptomyces rimosus
atgccggaaatcatcgacctgggcgcgtacggcccggacttcgtcgccgacccgcatccgtactacgccaagctgcgcgcccagggcccggtccaccgggtccgcgccccggagatggagccggagttcccgcaggcctggctgatcgtcggatacgacgaagcgcgggccgtgctggccgacaaccgcttcgccaaggactggtcccgggcgaacggctccctcgccgacagcgaggtcctggccgagtggcagctgatgaacatgctcgacgccgacccgccgcagcacacccggctgcgcaagctggtggcccgggagttcaccacccgccgcgtcgaggcgctgcgcccgcgcgtccagcagatcaccgacgagctgctggacgccatgctggccgccccggacggccgcgccgacctcgtggaggcgctcgccttcccgctcccgatgaccgtcatctgcgaactcctcggcgtgcccgacatcgagcgggacaccttccgcgcctggtccaacgaactggtctcgccgaccgacaacgaggcgacgatgaccgccgcccgcgagatggccgcctatctggacggcctgatcgaaagcaagcggagctcgccgggcgaggacctgctgagcgcgctggtgcgcacgagcgatgaggacggcgaccagctctcccggcaggaactgctcggcatggccttcctcctgctcgtggccggccacgaaaccaccgtcaacctgatctccaacggcgtacgggccctgctccagcaccccgcgcaactggccgcactgcgcgccgatccctcgcttctcgacaacgccgtcgaggagatgctgcgctacgacggccccgtggagaccgccacctggcgcttcaccgccgagcccgtcgggatcggcggcgtggagatcccggccggtgagatcgtcctcgtcggcctggccggggcggaccgcgacccggagcgcttcgaggcccccgacaccttcgacatcacccgcgagacccgcggccacgtcgccttcggccacggcattcacttctgcctcggcgccccactggcccgcgtcgagggccgtatcgcggtgcgcactctcctggaccgctgcccggacctggccctggacaccgctcccgaggcgctgacctggcgcgcgggcatgacgatacgagggccccagcacctgccggtgcggtggcggtaa

SEQ ID NO: 47 - protein, 403 aa, Streptomyces rimosus
MPEIIDLGAYGPDFVADPHPYYAKLRAQGPVHRVRAPEMEPEFPQAWLIVGYDEARAVLADNRFAKDWSRANGSLADSEVLAEWQLMNMLDADPPQHTRLRKLVAREFTTRRVEALRPRVQQITDELLDAMLAAPDGRADLVEALAFPLPMTVICELLGVPDIERDTFRAWSNELVSPTDNEATMTAAREMAAYLDGLIESKRSSPGEDLLSALVRTSDEDGDQLSRQELLGMAFLLLVAGHETTVNLISNGVRALLQHPAQLAALRADPSLLDNAVEEMLRYDGPVETATWRFTAEPVGIGGVEIPAGEIVLVGLAGADRDPERFEAPDTFDITRETRGHVAFGHGIHFCLGAPLARVEGRIAVRTLLDRCPDLALDTAPEALTWRAGMTIRGPQHLPVRWR

SEQ ID NO: 48 - DNA, 1263 bp, Streptomyces rimosus
atgtcagtgccgagccgcccgccggccaccgtgctcgacaacccgctgcacgccctgctcgaccgggaggtgctcgcgaacccctacccgctgttcgagcggtggcgggagcaaggtccgatgtggacgtcggacggttccctgctgctgagcgaccacgccagttgtctggcggtgctcaagagccacccgaccatgggcagtgacacgttcaacgcgccggggatgcgggaactcttcggcgaccgcggcgacgagccggtgctcaactcgatcttcttcatggacgatcccggacacgggcggcagcggaacctggtcagcaaggcattcacaccacggatcaccgcgcgcttcgagccgtggatccgcgagatcgtggacgaactgcttcgcgactgcctggccgacggcgagttcgacggcgtgcaggacctggccgcggtgctctcgctgcgggtcatcgcgacgctcctgggcatcccgcgcgaggacatcccgatgctgcgggagtggtccagcgacatggcgctgtccacggagctgcccacgctggtggccagcttccactccaccgcgatgttcgaccgcgaggaactcgtccgcatcatccgtaccaccaccgaactgcacggctacttcgcgaacctcatccacaagcgccgccgcaaccccggcgaggacctcatctccagtctgatctccacgcaggagaacgggcgcggactgagccggcgtgaggtgacgaacgtcgtggtgaccgtgttcaccgcggcccacgagtccaccacgaacctgatcaccaacggcctgctcgcgatgtcgcgccacccggagcagttccagctgctccggcagaacccggcgatcgtcggcgacgtggtcggcgaggcgctgcgctacgactgcccgatcatgctgaccggccgggtcgcgctgcggtccgaccggatcaacggcatcgacatccccgagggctcggtggtcaccctggtcctcgcgtccggcaacagggacgagcgggtgcacccgaaggcggatcggttcatcgcggaccggaagccggccgtgatgaacctcgccttcggcgccggcgcgcacttctgcctcggtagcagtctggcccggctggaggcggagatcgtgttcggtgagctggctcgccggctgcgcggctttcacgtgcacgaggactcactgagctatcgcaggcacgtggtcgtccgcggcctcgacaccgaacggatcactttccaactctaa

SEQ ID NO: 49 - protein, 420 aa, Streptomyces rimosus
MSVPSRPPATVLDNPLHALLDREVLANPYPLFERWREQGPMWTSDGSLLLSDHASCLAVLKSHPTMGSDTFNAPGMRELFGDRGDEPVLNSIFFMDDPGHGRQRNLVSKAFTPRITARFEPWIREIVDELLRDCLADGEFDGVQDLAAVLSLRVIATLLGIPREDIPMLREWSSDMALSTELPTLVASFHSTAMFDREELVRIIRTTTELHGYFANLIHKRRRNPGEDLISSLISTQENGRGLSRREVTNVVVTVFTAAHESTTNLITNGLLAMSRHPEQFQLLRQNPAIVGDVVGEALRYDCPIMLTGRVALRSDRINGIDIPEGSVVTLVLASGNRDERVHPKADRFIADRKPAVMNLAFGAGAHFCLGSSLARLEAEIVFGELARRLRGFHVHEDSLSYRRHVVVRGLDTERITFQL

SEQ ID NO: 50 - DNA, 1365 bp, Streptomyces rimosus
atgaccacatcgcccaccgagtccaccacggccaccccgcccgactccaccaccgcctccgcccccggcaccccgccggacgccctgccgtcctacgtcggcctgcacccgggcgagccgaacgtgatggagccggagctgctcaacgacccgtacgccggttacgggaagctgcgcgaacagggcgccctggtgcgcggccggtttctcgacgactcgcccgtctggctcgtgacccgcttcgacgtggtacgcgaggtcatgcgcgacccgcggttcatcaacaacccgtcccgcctgcccggccgcacggagaaggacccgcgcgcccagctgatcgagctgttcggcatccccgaccacatggcccggtacctggtggacaccatcctcaccagcgacccgccggaccacacccggctgcggcgcctggtctcgcgggccttcaccgcccgccgcatccaggacctgcggccgcgggtggaggcgatcaccgacgagctgctggaccggttgccggcccacgcgcaggacggcgtcgtcgacctcgtcgagcacttcgcgtacccgctgcccatcaccgtgatctgcgaactggtcggcatcgacgaggaggaccggccgctgtggcggcagttcggcgccgacctcacctccctggagccgaagcggatcggcgccacggtaccggccatggtcgagcacatccacaaggtgatcggcgagcgccaatcggccctgcgggacgacctgctcagcgcgctcatccgggcccgggacgacgacggcggccggctgagcgagaccgagatggtcaccatggtcctcacgctggtactggccggccacgagaccaccgcccacctcatcagcaacggcaccctcgccctgctcacccaccccgaccagcggcgcctgctcaccgaggacccgggcctgctcccccgcgcggtccacgagctgatgcgctggtgcgggccgatccaggccacccagctgcggtacgcctccgaggacgtcgaggtggccggcacccaggtccacaagggcgacgccctgatgttcagcctcgtggcggccaaccacgacccgcgccactacaccgagccggaaaaactcgacctgacacgccagccggcgggccgcgccgaggaccacgtcggcttcggacacggcatgcactactgcctgggcgcctcactcgcccggcaggaaggcgaagtcgccttcggcaagctgctcgcacgctatccggaggtggcactcgccctgccccatgagcagctggaggagcaagagcgcatacgccagcccgggtcctggcgactgcggcggctgccgttgcggctgcgtccggaggactaa

SEQ ID NO: 51 - protein, 454 aa, Streptomyces rimosus
MTTSPTESTTATPPDSTTASAPGTPPDALPSYVGLHPGEPNVMEPELLNDPYAGYGKLREQGALVRGRFLDDSPVWLVTRFDVVREVMRDPRFINNPSRLPGRTEKDPRAQLIELFGIPDHMARYLVDTILTSDPPDHTRLRRLVSRAFTARRIQDLRPRVEAITDELLDRLPAHAQDGVVDLVEHFAYPLPITVICELVGIDEEDRPLWRQFGADLTSLEPKRIGATVPAMVEHIHKVIGERQSALRDDLLSALIRARDDDGGRLSETEMVTMVLTLVLAGHETTAHLISNGTLALLTHPDQRRLLTEDPGLLPRAVHELMRWCGPIQATQLRYASEDVEVAGTQVHKGDALMFSLVAANHDPRHYTEPEKLDLTRQPAGRAEDHVGFGHGMHYCLGASLARQEGEVAFGKLLARYPEVALALPHEQLEEQERIRQPGSWRLRRLPLRLRPED

SEQ ID NO: 52 - DNA, 1245 bp, Streptomyces rimosus
atgaccgccgagaaccacaccgcgcagccccaggcgcccgcgcccgacgggatcccgtacgacgagccccttccgcactaccccttcagcaccaagggggaccggctcgcccccgaactcgacgagctgcgcagccgctgccccgtggcccgggtcagcaccaactccggtgaacaggcgtggctggtgaccgactacgggctcgcccagcacgtactgcgggaccgcgccttcgcccgctccgtgctgggcgaggcggacagccccgcccaggacgccccgatcctcgcgcccgaactgctcgacgccatgaaccacctccagcaggccgggctgcgtgccgaagtgctccgctcgctcggccgcgaccagcccgacctgcccgccgactgggtcgcgcgggtcaccggcgaagggctggacgcgatgatccgcgaaggcgcccccggcgacctccagcgccacttcgctgagtgggtcgccgcccagtgcatgtgccgcctcctcggcgtgcccttcgaggaccatgcctggctcgccgtacgggcggacctggacctgaccatggtcacccccacccccgaggaactcgcccgcaactgggaggagatccgcgcctacatggccgcgcacatgacggcccgccgccccggcgagccccgaggcctcgtggaccgcctcgccgacctcaacgccgcgcaccaagggctgacggagcggcagctgtcgaacatcgtgtccgtcctcttcgtcagcggctacgaggacttcgcgagcttcctgggcgtcgcggcctacaacctgctccagcacccggagaccatcagcgcggtgcgcgccgagccggagaccatgccgcagtgcgtggaggagctgctgcggtgcagcgtcgtgctgggcaacgcgattccccgctttgtcaccgccgacgcgcggatcggcccgtcccaggtcaaaaagggcgacatggtcctgctctccctggacgcggtcaactacgactcgaccgcgttccccgaccccaagaccttcgaccccacccgctcacccaacccccacctgcgcttcggctacggccgccaccactgccccggcgcccacctggtccgccgccagtccgaggtcgccttccgcgtcctcctcgaccgcctgcccggcatccacctggtggtgccgccgcaagaggttccctggcacccgaaccgcatggcgatcatggcggcggagattccggtggcgtggtaa

SEQ ID NO: 53 - protein, 414 aa, Streptomyces rimosus
MTAENHTAQPQAPAPDGIPYDEPLPHYPFSTKGDRLAPELDELRSRCPVARVSTNSGEQAWLVTDYGLAQHVLRDRAFARSVLGEADSPAQDAPILAPELLDAMNHLQQAGLRAEVLRSLGRDQPDLPADWVARVTGEGLDAMIREGAPGDLQRHFAEWVAAQCMCRLLGVPFEDHAWLAVRADLDLTMVTPTPEELARNWEEIRAYMAAHMTARRPGEPRGLVDRLADLNAAHQGLTERQLSNIVSVLFVSGYEDFASFLGVAAYNLLQHPETISAVRAEPETMPQCVEELLRCSVVLGNAIPRFVTADARIGPSQVKKGDMVLLSLDAVNYDSTAFPDPKTFDPTRSPNPHLRFGYGRHHCPGAHLVRRQSEVAFRVLLDRLPGIHLVVPPQEVPWHPNRMAIMAAEIPVAW

SEQ ID NO: 54 - DNA, 1215 bp, Streptomyces rimosus
atgccgcaggacacctcccgccggttcgagcgagcgcccagggccgccttcggccccgacgcccacacccgcgagctgcacgggaaagcaccggtcagcaaagtcgacatgggcccgatacccgactcggacgccggccgcgccacggtctggctggtcacgggctaccacgaggtacgccaggtcctcggcgaccacgtacggttcggcaacggcttcgcctccggcccggtgtacgggaccgcgagccgcttccggcccccggaggtcgtcgggcacctgatggactacgacccgccggagcacacccggctgcgccggatgctgaccccggcgttcacggtccggcggatgcggcagctggagccccgtatcgaagaggtcgtggcgcgctgcctggacggcgtggcgaaggccgggcagcccgccgacctggtggaacggttcgcccgcccggtgtcgggcgaggcgctgtgcgaactgctcggggtgccgcgcgacgaccgtacggacttcgtgcgccgcgtccagtggcagctggagcaggaccggccgcgcaggcagcgggccgacgcgggcgagtcctacctgcgctacctcggcgcgatggtgcgccgccgtcgcaaggaccccgacgacagcttcatcggcacgctcgtacgcgagcacggcgacagcatcaccgacgaggaactgcgcggcgtctgcggcctgatgatgctcgccgggctcgacaacgtctccggcatgatcagcctgggcatcctcgtcctgctccagcaccccgaccagctcgccgcgctgcacgccggcaccgcgtccgcggaccgcgtggtcgacgagctgctgcgctacctgtcggtggcgcacgcaccgcagcggcggatcgccctggcggacgtcaccgtcgcgggccaggtgatcaaaaagggggagcaggtcctgtgctccctccagatggccaaccgcgacccggccttcctcccgcaccccgaccgcttcgacgccacccgcgaccccgcgccccacgtcgccttcggccatggcatccaccactgcatcggcgccgcgatgtccaggatggaactgcgcatcgcctaccgcgccctgtggcaccgcttccccggactgcggctggccgtccccgtggaggagatcgcgtatcggaccaatgcggtggcggacggggtggtgaggctgcctgtggtgtggtaa

SEQ ID NO: 55 - protein, 404 aa, Streptomyces rimosus
MPQDTSRRFERAPRAAFGPDAHTRELHGKAPVSKVDMGPIPDSDAGRATVWLVTGYHEVRQVLGDHVRFGNGFASGPVYGTASRFRPPEVVGHLMDYDPPEHTRLRRMLTPAFTVRRMRQLEPRIEEVVARCLDGVAKAGQPADLVERFARPVSGEALCELLGVPRDDRTDFVRRVQWQLEQDRPRRQRADAGESYLRYLGAMVRRRRKDPDDSFIGTLVREHGDSITDEELRGVCGLMMLAGLDNVSGMISLGILVLLQHPDQLAALHAGTASADRVVDELLRYLSVAHAPQRRIALADVTVAGQVIKKGEQVLCSLQMANRDPAFLPHPDRFDATRDPAPHVAFGHGIHHCIGAAMSRMELRIAYRALWHRFPGLRLAVPVEEIAYRTNAVADGVVRLPVVW

SEQ ID NO: 56 - DNA, 1254 bp, Streptomyces rimosus
atggatgagtcgcccgtcttcgtcctggatcccgcaggccgtgaccggcacggtgaggacgcccggttgcgcgcccgtggcccgctcacccgggtggacgtgctcggcgtcgaagcctgggcggtctccgaccctgttctgctgcgtcggctcctcatggacccgcgcgtctccaaggatgcccgccgtcactggcctgcctatcccggccggatcgcgggggtctggccgctggagctgtgggtggcggtggacaacatgttcaccgcctacggtgacgaacaccgtcggctccgccgcatcatcagccaggtcttcaccgcgcggcacgtcaacgccctggcacccgtcatcgaacgcatcgccggagagctgctcgacggccttgctgccacaccgcccggtacgccggtggacctgcgtgaacgcttcgcgtcgccgttgccgatcagggtcgtcagccacttggtgggcctgtccgaagcggacgggccacgcttccgccgtaccgtcgacaaggtcttctccaccagtctggacccggtggaggcaggcgccaacgtcgctgaactgtacgcgctgctgaccggcctggtcgccgcgaaacgggccgagcccggcgacgacctggcctccaagctcatcaccgcgcgggacagtgagggcgacggatcacgtctcaccgagaccgaactgatcgacactctcctcctggtgatcaacgccgggttcgagaccaccgtcaacctgatcgaccaagccgtcacggccttgctcacccaccccggccggctcgccctcgcgcgagcgggccgcgtcggctggcaggacgtcgtggaggagacgctgcgctgggaggccccggtaccgtacctgcccatgcgctacgcggtggaggacatcccgctgcccggccacggcccgacgatccgcaaaggggacgcgatcctcgcctcgtacggcgccgccaaccggcacccggacctccacggtcccaccgccgatcagttcgaccccgccaggacggacaaatcccacctctccttcggacacggagtgcacgcctgcctgggtgccgcactcgcccggctggaaggcacgatcgccctgcgcggcctcttcgaacgcttccccgatctcgctctcgccgtcccggcacaccggctgcgccccctgccgagcttcgtctccaacggccaccgcgaactaccggttgtgctccgctccgcgccggccggggaagcagggggataa

SEQ ID NO: 57 - protein, 417 aa, Streptomyces rimosus
MDESPVFVLDPAGRDRHGEDARLRARGPLTRVDVLGVEAWAVSDPVLLRRLLMDPRVSKDARRHWPAYPGRIAGVWPLELWVAVDNMFTAYGDEHRRLRRIISQVFTARHVNALAPVIERIAGELLDGLAATPPGTPVDLRERFASPLPIRVVSHLVGLSEADGPRFRRTVDKVFSTSLDPVEAGANVAELYALLTGLVAAKRAEPGDDLASKLITARDSEGDGSRLTETELIDTLLLVINAGFETTVNLIDQAVTALLTHPGRLALARAGRVGWQDVVEETLRWEAPVPYLPMRYAVEDIPLPGHGPTIRKGDAILASYGAANRHPDLHGPTADQFDPARTDKSHLSFGHGVHACLGAALARLEGTIALRGLFERFPDLALAVPAHRLRPLPSFVSNGHRELPVVLRSAPAGEAGG

SEQ ID NO: 58 - DNA, 1377 bp, Streptomyces rimosus
atggagactgccccgctccgccccgtacccggcccgcgcggcctgccgtggctcggaaacctgcccgccttcggcaaggacccgctggcgttcctgacccggctgcgggacgccggcgacgccgtgacgtggtccctcggcccgcggcgcagcctgttcctctcccacccgcagcacatcgccgaattcctcggctcccggggcggcgcctacgacgtcctgcgaatcggctgggccatgcaccagctcgtcggcgagagcgtcctgctcaccgcgggggccgagtggcgccgcaagcgcggcatggtccagccgaccgtccgcccgcgccaggtccgccgcttcgcccggaccatggtcgacagcgccctcgcggcggtcggcggctggcgcgacggcgaccgcttcgacctgcggcgggagatgacgctcatcactcagcgcatcgtgctccgtacgctgttcggcaacgacctcggggaccggacccaggccctcggcgaggcgatggcgacggccgaacgcgcggtcgccaccgagatccgcggcctgcctctgatcctcccgccatgggtgccgctgccctaccgccggcgtcatctcggcgccgtcgccaccatcgacgccgagatgcggcggctgatcgacgcccggcgggccggggcggacggcggggacggtgccggtgcggacggcggccagggcggcgatctgctgacccggctgctcgcggcgcgggacgaggaagggcgcccgctgtccgccaaagaggtccaggacgaggcggtgacgctctgggcggccggtcacgagacgacctccaccgcgttgacgtggacctggtacctgctgtcccggtcgcccgaggcgcgggcccggctggacgacgaggtcgaccgcgtcctgggcggccgcccacccaccgaggaggactacgaacggctggtctggacccggcagatcgtcaaggagagcctgcggatgtatccgccggtctggctcgtccccgccgtggccaaggagggcgtcgtcctgggcggccgcgccattcccgccggtacgacggtgtggtgcagccagtggacggtccaccgggacccgcgctggttccgcgacccccaggtgttccgccctgaacgctgggacgccgacgctcccgacgtcatccccgaacacgcttggttcccgttcggcggcggctcccgcggctgtatcggcgcccggttcgcccagatggaggcggctttgctcatcgccgccgtggcgcagcgcttccacctggacgtgacgccgaaggaggcgacgccgcgcatgggcatggtcattcagccggccgtgccgctgatcgccacggtgcgcgctcgttcgcgtccgtaa

SEQ ID NO: 59 - protein, 458 aa, Streptomyces rimosus
METAPLRPVPGPRGLPWLGNLPAFGKDPLAFLTRLRDAGDAVTWSLGPRRSLFLSHPQHIAEFLGSRGGAYDVLRIGWAMHQLVGESVLLTAGAEWRRKRGMVQPTVRPRQVRRFARTMVDSALAAVGGWRDGDRFDLRREMTLITQRIVLRTLFGNDLGDRTQALGEAMATAERAVATEIRGLPLILPPWVPLPYRRRHLGAVATIDAEMRRLIDARRAGADGGDGAGADGGQGGDLLTRLLAARDEEGRPLSAKEVQDEAVTLWAAGHETTSTALTWTWYLLSRSPEARARLDDEVDRVLGGRPPTEEDYERLVWTRQIVKESLRMYPPVWLVPAVAKEGVVLGGRAIPAGTTVWCSQWTVHRDPRWFRDPQVFRPERWDADAPDVIPEHAWFPFGGGSRGCIGARFAQMEAALLIAAVAQRFHLDVTPKEATPRMGMVIQPAVPLIATVRARSRP

SEQ ID NO: 60 - DNA, 1350 bp, Streptomyces rimosus
atgcgcgatccggtccgctacttcgagacgttgcgccggcgctacggtccggtgttccgtatgaaattgctcggcttcccgccccaggtcgtggtctcgaccgcggagctggccgcggagatctaccgtatggacggcgacggcaaccgcgccggagcgctgcgcgcggggtacgtgccgtgggtcggacagcactcgctgctcaccaacgacggcgaggaatggtggcgccaccgcaagctgctcagccccaccctgcacggcaggtccatcgcgaactatcccgagctgatcgccgagatcgccgcgaaggacatcgggacgtggccgctcggcaggccgttcaccctgcgcgagcacatgcaggccatcaccctggaggtcatcctgcggctggtcttcggggtccgggacaccgagcagggggcccggttacgggccggtctcatcgacctgtccaaggccaccggctccgccgccctgttcctgacgcccgcccggctgcgggcctgggcgcaacggtctccgctggcgatgcgcctgccgttcctgccgacgacccgcgccgcgcaggccgtcgagacggtggaccacatcctgttcgccgagatcgcccggcgccgggccgaggaggacgcggacgccgacgacgtcctggggcggctgctccgcgcccgggacgaccagggccgcccgctcagcgaccaggagatccgcgacgaactgctcaccctgctggaggccggcctggagaccacggcgaccggcctgtcatggaccttcgagcggctgatgcgcaatccgcgggtgctcgcgcggctccaggaggaggtggagcagggcgaggacgacacctacctcgacgcggtcgtcaaggaggcgctgcggtcccgtccggtgatcttcggcatggggcggctgctggacaagccgttgcgggtcggtgggttcgaggtgccggccggctgggtggccatcccgatgttctcgctgatcctccaggaccgtgcggtgtacccggacgccggggagttccggccggaacgcttcctcggtgagggcgccaaggcggcgcagaagtcgttcctgccgttcggcggcggccgccgttactgcgtcggcgcccaactcgccacgctggagatgaagatcatcactcgcgaggtgctccggcacgtccatctggcccccgccgaccccgcgccggaggcccagcgcatgtggcacgccaccctcatccccggcaagcaggtcgtcgcggtggcccgcaagcaaccgccgaagcggcgggcgccggtccaggaggcgaagtgccccgtacatccggctctttcggacgacgcggggtaa

SEQ ID NO: 61 - protein, 449 aa, Streptomyces rimosus
MRDPVRYFETLRRRYGPVFRMKLLGFPPQVVVSTAELAAEIYRMDGDGNRAGALRAGYVPWVGQHSLLTNDGEEWWRHRKLLSPTLHGRSIANYPELIAEIAAKDIGTWPLGRPFTLREHMQAITLEVILRLVFGVRDTEQGARLRAGLIDLSKATGSAALFLTPARLRAWAQRSPLAMRLPFLPTTRAAQAVETVDHILFAEIARRRAEEDADADDVLGRLLRARDDQGRPLSDQEIRDELLTLLEAGLETTATGLSWTFERLMRNPRVLARLQEEVEQGEDDTYLDAVVKEALRSRPVIFGMGRLLDKPLRVGGFEVPAGWVAIPMFSLILQDRAVYPDAGEFRPERFLGEGAKAAQKSFLPFGGGRRYCVGAQLATLEMKIITREVLRHVHLAPADPAPEAQRMWHATLIPGKQVVAVARKQPPKRRAPVQEAKCPVHPALSDDAG

SEQ ID NO: 62 - DNA, 1269 bp, Streptomyces rimosus
atgttcacaccccgcacgtacgccaccgcggtcccgtacgaactcttcagggaactgcgggcgacccggccggtgtgctggatcgaggaaccggcggtcgacggctggcccgccgggcccggctactgggccgtgctgcggcacgccgacgtcaaacacgtcctgcgtacccccgagatctactcctcgtacctgggcgcgacccagatccgcgaccccgacaccgaggaggacctcgcgttcgtccgggcgatgatgctcaaccaggaccctccggaccacgcgcgcatccggcgtgtcgtcgccgcggccttcaccccgcgcgcggtacgggaactggcggacgtcatcgacgcgcgggcacgggagctggtggcggaggtggcacgggcgggcgaggcggacttcgtgaccgtggccgccgacctgccggtgtggacgctggcgcacgtcatgggcgtcccggaggaggaccggcagctgctcttcgactggtcgaaccgcgtcatcggctaccaggacgacgcgtacgccacctccagcactgccgaccccgcccgcctcagcccgatgggacgggccgccctgcgccaccggcccgcaccggcgctccgcccggacggacgcccggtcaacccgcgctcgcgccgcgcactggccgacatgttcgcgtacgcccacgcgctggccgagcacccgcgccccggcaccgtgatggcccacctacgggaaggcggcctgacccgcgccgagttcgagaacacgttcttcctcttcgccgtggccggcaacgaaaccctgcgcaacggcatcccgggcggcctgctcaccctcctccagcacccggaccagttcgcccgcctccgccgggaaccggacctgaccgacagcgcggtggaggaaatgctgcgctactggcccccggtgatcgacttccgccgcaccgccacccgcgacaccgaactcgccggacagcacatccgccgcggcgacaaggtcgtcgtctaccacgcctccgccaaccgcgacgaaaccgtcttccccacccccgaccacttcaacatcacccgcacccccaacgaccacctcagcttcggcttcggcccacacttctgcctgggcagccacctcgcccgcctccagatgcgggcggtactccggcatgtgctggagcggctgccgggggtggagctggcgggggagccggtgcggttggtttccaactttcagaacgggttgcggcggttgccggtgcgggtgggggcgtaa

SEQ ID NO: 63 - protein, 422 aa, Streptomyces rimosus
MFTPRTYATAVPYELFRELRATRPVCWIEEPAVDGWPAGPGYWAVLRHADVKHVLRTPEIYSSYLGATQIRDPDTEEDLAFVRAMMLNQDPPDHARIRRVVAAAFTPRAVRELADVIDARARELVAEVARAGEADFVTVAADLPVWTLAHVMGVPEEDRQLLFDWSNRVIGYQDDAYATSSTADPARLSPMGRAALRHRPAPALRPDGRPVNPRSRRALADMFAYAHALAEHPRPGTVMAHLREGGLTRAEFENTFFLFAVAGNETLRNGIPGGLLTLLQHPDQFARLRREPDLTDSAVEEMLRYWPPVIDFRRTATRDTELAGQHIRRGDKVVVYHASANRDETVFPTPDHFNITRTPNDHLSFGFGPHFCLGSHLARLQMRAVLRHVLERLPGVELAGEPVRLVSNFQNGLRRLPVRVGA

SEQ ID NO: 64 - DNA, 1227 bp, Streptomyces rimosus
atgaccacggacgacgacgaagaagaggatcagcggatgcccgagacacccgagattcccgcgcactaccggcgggaccgcttcgacccggtacccgaactcgtccggatggccagggagacgccgctggtcgagaccgacgtcacgatcggtccctccgagcaggtgggctgggtggccaccgggcacgccgaggtgcgggcggtgctggccgacgcggagcggttcagcacccgcccgcccgccgacagcgaggaggacgccgagagcctggtccaggccgggaacctgctccagtacgacccgcccgaccacacccggctgcgcaagctgctcacgccggagtacacggtgcgcaagatgcgccgcctggagccccgcatcgaggagatcgtccaggactgcctggacaccatggagcgcgtcggccgcccggccgacctcgtacgctacttcgcctggccgatcccgggcctcgccagctgcgaactgctcggcgtcccccgcgacgaccagacggaactggcgcgctacctggacatcacccgggacgtgggccgcagccaggaacagcagctggccgccgggaaggcgtactgggcgtacatgggccagctcgccgagcgccgccgccgcaaccccggcgacgacatgctcggcagtctcgtccgcgaacagggcgcggccgtctccgacgcggaactggcgggcatcggcgcgacggtgatggccgccggcttcgaacaggtcgccagcatcctggggctgggcaccctgctgctgctggaacaccccgaccagctcgccctgtggcgcgaacagcccgaactgaccgaccgcgcggtcgaggaagtgctgcgctacctcacggtcatccacaccgcctcgccccgtacggcactggtggacgtgacgatcggcgggcagaccatcaaggccggggagagcgtggcctgttcgctgctggccgccaaccgcgtaccggcccccggtgagcccgccgaccgcttcgacatcacccgtgagccggccacccacatggccttcggccacggcatccaccactgcctcggcgccccgctggcccggatggaactgcgcatcgccttcccggccctgctgcgccgcttcccggacctgcggctcgccgtgccgcacgagcgggtccggttccggcccgcccggtcccgccagtacgccctggaatcgttgcccgtcgcatggtaa

SEQ ID NO: 65 - protein, 408 aa, Streptomyces rimosus
MTTDDDEEEDQRMPETPEIPAHYRRDRFDPVPELVRMARETPLVETDVTIGPSEQVGWVATGHAEVRAVLADAERFSTRPPADSEEDAESLVQAGNLLQYDPPDHTRLRKLLTPEYTVRKMRRLEPRIEEIVQDCLDTMERVGRPADLVRYFAWPIPGLASCELLGVPRDDQTELARYLDITRDVGRSQEQQLAAGKAYWAYMGQLAERRRRNPGDDMLGSLVREQGAAVSDAELAGIGATVMAAGFEQVASILGLGTLLLLEHPDQLALWREQPELTDRAVEEVLRYLTVIHTASPRTALVDVTIGGQTIKAGESVACSLLAANRVPAPGEPADRFDITREPATHMAFGHGIHHCLGAPLARMELRIAFPALLRRFPDLRLAVPHERVRFRPARSRQYALESLPVAW

SEQ ID NO: 66 - DNA, 1179 bp, Streptomyces rimosus
atgttgatgccgctgcggcgtcaggggctggacccggtgggcgagctggcgacggtgcgcgagcaggagcccatctccaagctgccggtgccgatcgccgccaatgtgtggctcgtcaccgggtacgacgaggtcaaggcggtactgggcaaggccaacgccttcagctcggacttcaccaacctcatcggccaggccggtgccagcaccgaccagaaccccggcggcctcggattcgccgacccgccggtgcacacccggctgcgccgtctgctgacccccgaattcaccatgcgccggctcgggcggctcacgccccgtatccacgagatcgtggaggagcggctggacgccatggagaaggccggcagctccggcgagccggtcgacatcgtggaaacctttgcgctgccgattccgtccttggtcatttgcgaactgctcggtgtgccgtacgaggaccgcgcggacttcgagcggctgagcgccgcgcgcttcgacctcttcagcggcgccaacgcgtccttcggcgccatatcggaatcgctcgcctatttccgtgaggtggtcaagaagcagcggcagaacccgggcgacggcctgctcggcatgatcgtcaaggaacacggcgactcggtcagcgacgaggagctggcgggcctggccgacggcgtgctgaccggcggcttcgagaccaccgcgagcatgctggcgctgggcgccctggtcctcctccaggaccccgagcacttcgccgccctcaaggacggcgacgaggcggccgagcgctacgtcgaggagctgctgcgctacctcaccgtcgtccaggtcgccttcccccgcttcgcgcgcgaggacatggagatcgccggtgtgccgatcgccaagggcgacgtggtgctgtgctcgctcagcggcgccgaccgggacggcaagctcggtcccgacatggagcgcttcgacccgtcccgcaacgttccctcgcacctggccttcggctacggcatacaccgctgcgtcggcgccgagctggcccgtatggagctgcgcgccgcctaccccgcgctggtacggcggttcccgaacatgcggctcgcggtggagccggacgcgctggaattccgcaagctgtcgatcgtgtacggaatcgagtcgctgccggtgcacctcggcggctaa

SEQ ID NO: 67 - protein, 392 aa, Streptomyces rimosus
MLMPLRRQGLDPVGELATVREQEPISKLPVPIAANVWLVTGYDEVKAVLGKANAFSSDFTNLIGQAGASTDQNPGGLGFADPPVHTRLRRLLTPEFTMRRLGRLTPRIHEIVEERLDAMEKAGSSGEPVDIVETFALPIPSLVICELLGVPYEDRADFERLSAARFDLFSGANASFGAISESLAYFREVVKKQRQNPGDGLLGMIVKEHGDSVSDEELAGLADGVLTGGFETTASMLALGALVLLQDPEHFAALKDGDEAAERYVEELLRYLTVVQVAFPRFAREDMEIAGVPIAKGDVVLCSLSGADRDGKLGPDMERFDPSRNVPSHLAFGYGIHRCVGAELARMELRAAYPALVRRFPNMRLAVEPDALEFRKLSIVYGIESLPVHLGG

SEQ ID NO: 68 - DNA, 1035 bp, Streptomyces rimosus
atgctcggcgacgcccggttcagctccgaccgctcgcacccggacttcccgtggatgcgcgtcggcgagaccgttttccccggcttcaggccctcgctgatcgagatggacccgcccgagcacggccccgcccgtcgtgcggtcgccggcgagttcaccatccaccgcatgcgggagctgcgccccaagattcagcgcattgttgacggtctgctcgacgatgtgctggccggtgccaagcccgccgacctggtgtccgcgctggccgtgccgctgtccggtctggtgctgtgtgagctgctcgggatcccgaccggttaccgggaggagctcaccaccaacaccgcggtgttggtggcccacgactccgctgatgcggatcgcgccgagtccttccgctccctgagcgagtatttcgacgcgctgtgtgccacgaagatgaccgagcggcccggggacctgctgggcaggctggcgggccaccggctcttcagcggtgacgagagtcgctgggccatggtcgaactgtgcatactcctggtcgtcgcgggcctggagaccaccgccacgatgaccgcactcggaatcctggctctcctcgaacaccccggccagctcgccctcctcaccgccgacccgggcctgaccccgggagcggtggatgaattgctgaggttcttctccattgccgagctgtccctgatgcgccgcgccacggcggacgttgagatcggcggcactctggtacgtacgggtgagggcgtcgccgccctgtccgccgccgccaaccgcgaccccgcggtcttcgccgacccggacacgttcgatgtcaccagggacaaccgcaggcatctggctttcggttcgggaccgcaccagtgcctcggcaagaacctggcccggatggagctgcgcatcgttctcgataccctgttccggcgcatccccactctccgcctggccacgccacgcgacgaattgcgcttcgtcaacggctccgggttctcggtatcggcactcccggtcacttggtaa

SEQ ID NO: 69 - protein, 344 aa, Streptomyces rimosus
MLGDARFSSDRSHPDFPWMRVGETVFPGFRPSLIEMDPPEHGPARRAVAGEFTIHRMRELRPKIQRIVDGLLDDVLAGAKPADLVSALAVPLSGLVLCELLGIPTGYREELTTNTAVLVAHDSADADRAESFRSLSEYFDALCATKMTERPGDLLGRLAGHRLFSGDESRWAMVELCILLVVAGLETTATMTALGILALLEHPGQLALLTADPGLTPGAVDELLRFFSIAELSLMRRATADVEIGGTLVRTGEGVAALSAAANRDPAVFADPDTFDVTRDNRRHLAFGSGPHQCLGKNLARMELRIVLDTLFRRIPTLRLATPRDELRFVNGSGFSVSALPVTW

SEQ ID NO: 70 - DNA, 1194 bp, Streptomyces rimosus
atggacacacaccccgaacccatcgattaccctttttccgagccgtccgggctcaccgtcgatccggaatacgaggactgccgcagccgccccggcctgacgtggatccggccgccgtacggtgaccacgcctggctggtgacgcgctacgcggacatccgcttcgtcctgcgggaccggcggttcgtccgcacgcccccgccgggcagcgacgaggcgcggctgaccccgctgccgctgcaggacagcatcctgaacaccgatccgccccagcagccccgcctgcgcaaggccctcgcccagggcctcaagttcaacgccgagcacgtccgtgagctggaggaactggccaccggggaggcgcggcggctgctggcccgctgcacggcggagccgcccccggccgatctggccgccgcgtacaccaagccgctcaccgtggccatcctctgcccgctgatcggcatccccgaagaggacctggcggtcttcctcgactggttcgaggggttcgcgggcaccggcctgcccgccgacgtggtggagtcgcgtatcgaggagatctcccgctacacggcccggctcatcgccgaccgccggcagcggccgcgggaggacctggtcagccgcctggtggcccggctgggccaggacgacgggctgtcgatggaggagctgggcgagctggtcaacgacatcctgctcgccgtcgacaacgtcaccacccagctcaccaacgcctgttacgtgctgctctcctcccccgcccacttccgggagctggcggccgacccggacctgctgccgcgggcggccgacgagctgctgcgctacgcgccgttcccctcgcacgtcaccttcgcccggtacgccaccgaggacgtggaggtcggcggcaccctcgtacgggccggtgagcaggtgctgcccgcgctgccggccggcaaccacgacccgcggatgttcgccgagccggagcggctggacttccaccgcggcggcaacccgcatctgtccttcggccacggcacccatcactgcatggggccgccgctggtgcggatgctggtgaaggtggccgtggccgccctgctcggccaccccggcctgcggctggccgcgccggacgaggagctgccgtggcgcgccgacctgatcatccggcggatcgaggagctgccggtcacctggtaa

SEQ ID NO: 71 - protein, 397 aa, Streptomyces rimosus
MDTHPEPIDYPFSEPSGLTVDPEYEDCRSRPGLTWIRPPYGDHAWLVTRYADIRFVLRDRRFVRTPPPGSDEARLTPLPLQDSILNTDPPQQPRLRKALAQGLKFNAEHVRELEELATGEARRLLARCTAEPPPADLAAAYTKPLTVAILCPLIGIPEEDLAVFLDWFEGFAGTGLPADVVESRIEEISRYTARLIADRRQRPREDLVSRLVARLGQDDGLSMEELGELVNDILLAVDNVTTQLTNACYVLLSSPAHFRELAADPDLLPRAADELLRYAPFPSHVTFARYATEDVEVGGTLVRAGEQVLPALPAGNHDPRMFAEPERLDFHRGGNPHLSFGHGTHHCMGPPLVRMLVKVAVAALLGHPGLRLAAPDEELPWRADLIIRRIEELPVTW

SEQ ID NO: 72 - DNA, 1230 bp, Streptomyces rimosus
atgacgcagccggacaccaggacgaaccagccggacaccgggccgggccggcccgagcagatacccgcccacctgcggcgggaccgtttcgacccggttcccgaactccggcggcaggtccgggaggcgccgctcgtggtggccgacgtcgaattcgggctcttcggccgggtgaagtgggtggccaccggcgaggccgaaatccgggaggtgctgggcgacctgaaacgtttcagctcccggctgcccgacgacggccaggacacgtccggggcccgcgccgcacccggcaacctcctgcagtgcgacccacccgaccacacccgcctccggcgcatggtggcaccggaattcacggcgcggcggacccggcggctggaaccgcgcatcaccgcgatcgtcgaagagtgcctggacatcatggagcgcgtcggaccgccgaccgacttcatgcgaaacttcgcctggcccgtggcagggctgatcacctgcgagctgctgggcattccccgcgacgaccgggcggaactgtcccgctatctcgacatcgcccaggacgaatccgcgcccccggaacagcagacggccgtcggcaaggcgtactgggcctatatggtgcggctcgccaaacggcagcgccgcagccccggcgacggcctcttcggccacgtggtgcgcgagcacggcgcggacatcggcgacgacgaactggcgggtgtcggcgcgaccttcgtctccgacggcttcctccaggtctccagcatgctggggctgggcgcgctggcgctgctggaccaccccggccagctgcggctgctgcgggaacggccggagctgatcgaccgggccgtggaagaactgctgcgctacgtcaccgtcatccacaccgtctcgccccgcaccgccctggaggacgtgaccatcgggaaccaggtgatcaaggcgggcgagatggtcgcctgctcgctgttcgccgtcaaccgggcgcagggcggaccgggggcggacgcgttcgacatcacccgcgagtccgccccgcacctggccttcggccacggcatgcaccactgcgtcgccgcgccgctggtcaagctggagatgcgcatcgcctacccggcactgctgcgccggttccccgggctgcggcccgcggtggcgccggacggcatccgcttccggtccgcgcagacgcggcagttcagcctggacgcgctgcccgtcgcctggtaa

SEQ ID NO: 73 - protein, 409 aa, Streptomyces rimosus
MTQPDTRTNQPDTGPGRPEQIPAHLRRDRFDPVPELRRQVREAPLVVADVEFGLFGRVKWVATGEAEIREVLGDLKRFSSRLPDDGQDTSGARAAPGNLLQCDPPDHTRLRRMVAPEFTARRTRRLEPRITAIVEECLDIMERVGPPTDFMRNFAWPVAGLITCELLGIPRDDRAELSRYLDIAQDESAPPEQQTAVGKAYWAYMVRLAKRQRRSPGDGLFGHVVREHGADIGDDELAGVGATFVSDGFLQVSSMLGLGALALLDHPGQLRLLRERPELIDRAVEELLRYVTVIHTVSPRTALEDVTIGNQVIKAGEMVACSLFAVNRAQGGPGADAFDITRESAPHLAFGHGMHHCVAAPLVKLEMRIAYPALLRRFPGLRPAVAPDGIRFRSAQTRQFSLDALPVAW

SEQ ID NO: 74 - DNA, 1278 bp, Streptomyces rimosus
atgccggacgccggacgtctccctcgataccctttcgccttccggggcgaccagctcgcgcccgagctggccgcatcggtggtccaccgcccgatccagcgcgtacggaccaacaccggtaccgacgcctggctggtgaccggccacgagctggtgcgctcggtgctccgggaccgccgcttcagcctcaccctcacctccgacccctggatgccccggcaggaccccctcatcccaccgctctcggtcaccgacatccgcacccagtgcgagaacgcgggcctcctccaggacctcttccaaggcgtgggaccgcaccagcggtacctgacaccgggccgcgtccgggagatcgccgacgggctgctggacaccttcctggccggagagcaacccggcgacctgatggacgggttcatcatgccgctctcccgcgcgctcaccatggaactgctgggcctggacccggaaggctgcccggacaacgccgaaatcttcaacatcttccgtaccggcccggaaagcatgcagggcgtgccggagagctggaacctggcccttacgtggatgctcggacggcttcccgggctgcgcgcgtccggcgcagggctgctgggccgcctcatcaccctcagcgacgcgtccggcgtactgagcgaggaggaggtcgccgacctcttcgtcttcctcctcatctcccagttcggcaaccccgccaccttcctcggcgcggcgaccgtggggctgatgcagcacccggaggtgacggcccggctgcggaaggaccccgggctgctgccacgggccgtcgacgagctgctgcgctggacggtcttcctgggcgacgcactgccccgcaacgcgcgcgaggacgtgctgctggacggcgttctcgtacgggagggcgacctcgtgctggtgtccaccgacgcggccaaccgcgacccgcgggtcttccccgacccgcaccgcctcgacatcgaccgggagcccggcccgcacctgcggttcagcgacgggcggcaccgctgtccgggcggcccggtctcccgcatgcaggccgcggagacgctgcgcgtactgctggggcggaccgccgatctgcgcctggccgtgcccgccgacgagatcgaatggcaccgctactacgcggtcacactgccggtggcggtgccggtcaactggacgctccccggagcggccactcccgggaccggcgacggtaagccccgcggagcggccgttcccaggcccgatggcgggacgctcactccgtaa

SEQ ID NO: 75 - protein, 425 aa, Streptomyces rimosus
MPDAGRLPRYPFAFRGDQLAPELAASVVHRPIQRVRTNTGTDAWLVTGHELVRSVLRDRRFSLTLTSDPWMPRQDPLIPPLSVTDIRTQCENAGLLQDLFQGVGPHQRYLTPGRVREIADGLLDTFLAGEQPGDLMDGFIMPLSRALTMELLGLDPEGCPDNAEIFNIFRTGPESMQGVPESWNLALTWMLGRLPGLRASGAGLLGRLITLSDASGVLSEEEVADLFVFLLISQFGNPATFLGAATVGLMQHPEVTARLRKDPGLLPRAVDELLRWTVFLGDALPRNAREDVLLDGVLVREGDLVLVSTDAANRDPRVFPDPHRLDIDREPGPHLRFSDGRHRCPGGPVSRMQAAETLRVLLGRTADLRLAVPADEIEWHRYYAVTLPVAVPVNWTLPGAATPGTGDGKPRGAAVPRPDGGTLTP

SEQ ID NO: 76 - DNA, 1188 bp, Streptomyces rimosus
atggagtcaccggagttcttccgcgacccgtacccgctgctcgccgcgctgcgcgagcgcggtcccgtccagcaggtacggtccgggccgcacggcgcgacgtggctcgtcaccggctgggccgaggcccgtacggcgctggcggagccccggctctccaaggacaccacccgctacttcgccgacaagccgtccaagcgcaacctggcgcccgccgtcagcgccaccatgctggccaccgacccgccggaccacacccggctgcgccggctggccgtcaaggcgttcacgccggcggcggtggcccgcctggagccgcgggtggcggagatcgcggacggtctgctggaccggatggccgacggcggcgattcggccgatctcgtcgaggacttcgccgtaccgctgcccatcgaggtcatcggcgacctgctcggcgttccccgcgaggaccgcccggcgctgcgccgctggtccaacgacctcttcgcggccggcgcgccggacagcatcgacgcggcctcgcacgccatcagcgactacatgacggagctgatcgcgaagaagcgcgccgaaggtaccggggccgatctgctcaccgagctgatcgccgcgcgcgacgagggcgaccggctcagcgagttcgaactggtctcgctggccgtcctgctggtcgtcgccgggcacgagacgaccaccaacctgatcggcaacggcgcgctcgcgctcctccgggacgacgcgctccgtacccgcctgcggcaggacccggcgctcatcccggacgccgtggaggaactgctccgctatgactccccgatcaccacggccacgttccggtacgcggccgaaccgctcaccctcggcggcgccgagatcgcggcgggcgatgtcgtcctggtctccccgggcgccgccaaccgtgacccggcccggttccccgacccggacacggtcacccccggccgttccgccgggcatctctccttcggccacggtccgcaccactgcctgggcgcgcccctggcccgcctggaagcccgtatcgccttccgagcgctgctcacccgcttccccggcctgcggctggccgtcccgcccggcgaactcccgtggcgccacacccgcctgatgcgcggtctgtcgcacctcccggtcacctggtccgcacaggtcacggattgttaa

SEQ ID NO: 77 - protein, 395 aa, Streptomyces rimosus
MESPEFFRDPYPLLAALRERGPVQQVRSGPHGATWLVTGWAEARTALAEPRLSKDTTRYFADKPSKRNLAPAVSATMLATDPPDHTRLRRLAVKAFTPAAVARLEPRVAEIADGLLDRMADGGDSADLVEDFAVPLPIEVIGDLLGVPREDRPALRRWSNDLFAAGAPDSIDAASHAISDYMTELIAKKRAEGTGADLLTELIAARDEGDRLSEFELVSLAVLLVVAGHETTTNLIGNGALALLRDDALRTRLRQDPALIPDAVEELLRYDSPITTATFRYAAEPLTLGGAEIAAGDVVLVSPGAANRDPARFPDPDTVTPGRSAGHLSFGHGPHHCLGAPLARLEARIAFRALLTRFPGLRLAVPPGELPWRHTRLMRGLSHLPVTWSAQVTDC

SEQ ID NO: 78 - DNA, 1209 bp, Streptomyces rimosus
atgaagtcgtccgcgacgcggtccggggccggcggacacgcccgtaccccgtgcgatgccgcggcccgcgcccactccagcggcccgctggatctcttgcgcgccgagttcgacggcgtgcacgacgtgtggcgctcggcctcgggaatggtgtacgtggccggcccggaggcggcgcgggcggtgctgggcaaccggccggccatcgtggccgagacgtccgacttctaccggacccggcacggcgtcttcgggccgcgggccgcgcaggcggagatcggccgtgcggcccgcgccctgatgcaccaccacctcgacgcccggcggtcgcagctgccccggctgatccacgagcgcctcgcgccccgcagttcctggccggacgcggggaacctgctggtccacgagcacctggcggatgtcctgctgcacccgggcgcgccgatctccctgcgtacgacggtcggcaaggtcgtcacccgcgccgtgctggcgggtgcccgcaggcgccacgcaccgccgtccaggctcctcctccgccaccgcgcgtccgccgcgctgcaggccgagatacgcgcccggcagcaccggcgacagcaccacggcggcagcgccggcccccgcgacctgctcgatgtcgtggtggacggctgcggtcccgcgacggcatccgacgatctcgccgaggtctacctgtctttcctgttcgccgcggtgggctccatcggcttcgccctcggatggtcggtccaccttctcggcacccatcccggctgcccggcggcaccggaccggatcgtgcgcgaggccctgcgcctgtggccggtggcctggctgttcgcccgtacgccgctgcgggccgtggagctcggcgggatgacggtgacacccgaggaccagctcgccgtgtgcacctacctggtgcaccggcatcccgcgtactgggagcgacccgacgagttcctcccgcagcgctgggcggcacccgtctcccgggccgcctacctccccttcgggcacgggccgcacacctgcgccggagcgaccgtcaccctgcaactcctcaaggacatcgtcggcctgctcatccatgactggcggctgtcggtcatccacgacggcggcggtcctcaggtgggcccggcgctggctccgccgcgcttcaccgcggtgctgagcccacgtgccaacagctccggaaggaggtaa

SEQ ID NO: 79 - protein, 402 aa, Streptomyces rimosus
MKSSATRSGAGGHARTPCDAAARAHSSGPLDLLRAEFDGVHDVWRSASGMVYVAGPEAARAVLGNRPAIVAETSDFYRTRHGVFGPRAAQAEIGRAARALMHHHLDARRSQLPRLIHERLAPRSSWPDAGNLLVHEHLADVLLHPGAPISLRTTVGKVVTRAVLAGARRRHAPPSRLLLRHRASAALQAEIRARQHRRQHHGGSAGPRDLLDVVVDGCGPATASDDLAEVYLSFLFAAVGSIGFALGWSVHLLGTHPGCPAAPDRIVREALRLWPVAWLFARTPLRAVELGGMTVTPEDQLAVCTYLVHRHPAYWERPDEFLPQRWAAPVSRAAYLPFGHGPHTCAGATVTLQLLKDIVGLLIHDWRLSVIHDGGGPQVGPALAPPRFTAVLSPRANSSGRR

SEQ ID NO: 80 - DNA, 1434 bp, Streptomyces rimosus
atgcgcccaccccgcctacccgaaccgctccccctctacggggaggactacaagcgcgacccgtaccccctgtacgccgagctgcgcgagcgcggccccgtccaccgggtcaggttcccgagcggcgtgcacgcctggctcgtcaccggatacgaggccgctcaccgggcgctgaacgatccccggctgggcaagcaccactcccgcggcaacgccgcctggcgcgcccgtgcctcgatcatgcccgagccgcagcattcgcggctccaggtccacctgctgcaccaggacccgccccggcacaccgccatgcggcgcctgatcaccgacgccttcgcacccaggcggatcgccggactccggccgcggttcgagcgcttggcggaggcgctgttggatgaactgccgcccgcagggccgagcggcgaaggcggtccggagcggggcgcccgcgccgacctggtcgcctcgttcgcggcgcgcttccccttcctcgtgctcgccgaggtcatcggcctgccggacgcgttcaccgcgcgcttcgaccgcgactggggcaaggtcgtccagcccgtcggcccggacgatcccggccgtccggcgtacgaggcccggctgcgcggcttgcagggctatatcgccgacctcgtacaacacaagcggcgggaacgcggcaccgacctgctctcccgtctggtcaccgcccgcgacgccggggaactggacgatgccgagctggactccatgatcttccaactcctcgtcgccggacaggaacccgtcaccaaccagatcaccacagcgctgaccgccctgctccggcacccggaacacctcgcgcggctgcgcgacgaccccgcgctcctcccccgcgcggtggaggaactgctccgctacgacagtgctttcgagctgacgacctggcggttcctcgcggcggacgcggacgtgtcgggcacgcggattccggccggcgactccgtgatcgtctcgctgtgcgcggccaaccgcgaccccgcccgcttccccgcccccgacacgctcgacttcgaccgtacgcccaacccgcatctcgccttcggccacggcatccacttctgcccgggcgccacgctcgcccgtaccgaactgcacatcgctctggaaacgctgctccgccgcctgccgggcctgcgcctggccgtgccggatgccgacttgaggtggataccggcggtgctggcgcgcggggtggatgagcttccggtctcgtacggggcggttggcggggctgcgggcagcgatggcggggtgggtacagaaccggccggatcgggtacagaaccggccggtactcctgcgggcagaggcggcgggtcgggtacagaacccgccggaccgcctccgtacgcctgccccttcagcggctctgccggagaggccgccacccgataa

SEQ ID NO: 81 - protein, 477 aa, Streptomyces rimosus
MRPPRLPEPLPLYGEDYKRDPYPLYAELRERGPVHRVRFPSGVHAWLVTGYEAAHRALNDPRLGKHHSRGNAAWRARASIMPEPQHSRLQVHLLHQDPPRHTAMRRLITDAFAPRRIAGLRPRFERLAEALLDELPPAGPSGEGGPERGARADLVASFAARFPFLVLAEVIGLPDAFTARFDRDWGKVVQPVGPDDPGRPAYEARLRGLQGYIADLVQHKRRERGTDLLSRLVTARDAGELDDAELDSMIFQLLVAGQEPVTNQITTALTALLRHPEHLARLRDDPALLPRAVEELLRYDSAFELTTWRFLAADADVSGTRIPAGDSVIVSLCAANRDPARFPAPDTLDFDRTPNPHLAFGHGIHFCPGATLARTELHIALETLLRRLPGLRLAVPDADLRWIPAVLARGVDELPVSYGAVGGAAGSDGGVGTEPAGSGTEPAGTPAGRGGGSGTEPAGPPPYACPFSGSAGEAATR

SEQ ID NO: 82 - DNA, 1218 bp, Streptomyces rimosus
atggaaggagtccaggcagtcttcgatccctggtcgccggatttcgtcgccgacccgtatcccgcctacgccgagctgcgcgcccgcggccgggtgcactatttcgcgccctccaaccagtggctcgtcccgcgccacgcggacgtcgcggcgctgctccgcgaccgccggctgggccgtacgtaccggcaccgcttcacgcacgaggagttcggccgtaccgctccgccacccgagcacgagccgttccacgtgctcaacgacaacggcatgctcgacctggaggcgcccgcccacacccgcatccgccgtctggtctcgaaggcgttcaccgcccgtacggtcgagcggctgcggccctacgtcgaagccctggcggaccggctggccgcggatctggtcgcggacggcggcggggacctggtggcgcgggtcgcggagccgctgcccgtcgcggtgatcgccgaaatgctcggcatccccgaggccgaccggcatgcgctgcgcccctggtcggccgccatctgcggcatgtacgagctgaacccgccggaggagacggcccggcgcgcggtggccgcttcgctggaattctccggctacctgcgggaattgatcgccgctcggcgcagtgcgccgggggacgacctgatctccgggctgatcgccgcgtacgacgagggcgagtcgctgagcgaacaggagatgatctcgacctgtgtcctgctgctgaacgcgggccacgaggccactgtcaacgcgacggccaacggctggtacgcgctcttccgccacccggagcagttggcggccctgcgcgcggccccggccgcgctgctgcccaccgccgtggaggagttgctgcgccacgacacgccgctccagctcttcgaacgctgggtgctggacgacatcgagatcggcggtacggtcgtgccgcgcggcagcgagatcgcgctactcttcggctcggccaaccacgacccggcagccttcgaccaccccgaacggctcgacctcgcccgtaaggacaacccgcacatctccttcagcgccggtatccactactgcatcggcgcgcccctggcccgtatcgaactggccgcctcgctggcggcgttgctccgccgggcccctgacctgcgcctggccgccactccggaacgcaagccgaacttcgtgatccgaggactgcgcgagctgctggtcgcggtgtaa

SEQ ID NO: 83 - protein, 405 aa, Streptomyces rimosus
MEGVQAVFDPWSPDFVADPYPAYAELRARGRVHYFAPSNQWLVPRHADVAALLRDRRLGRTYRHRFTHEEFGRTAPPPEHEPFHVLNDNGMLDLEAPAHTRIRRLVSKAFTARTVERLRPYVEALADRLAADLVADGGGDLVARVAEPLPVAVIAEMLGIPEADRHALRPWSAAICGMYELNPPEETARRAVAASLEFSGYLRELIAARRSAPGDDLISGLIAAYDEGESLSEQEMISTCVLLLNAGHEATVNATANGWYALFRHPEQLAALRAAPAALLPTAVEELLRHDTPLQLFERWVLDDIEIGGTVVPRGSEIALLFGSANHDPAAFDHPERLDLARKDNPHISFSAGIHYCIGAPLARIELAASLAALLRRAPDLRLAATPERKPNFVIRGLRELLVAV

SEQ ID NO: 84 - DNA, 2846 bp, Streptomyces rimosus
atgcagatcgtcgtggacctcacccgctgtcaggcgtacgcgcaatgcgtcttcctcgcgccggaggtcttccggctgcccagggaggagagcctgctgtaccgcccggacgttcccgaggaccagatggagcgcgtgcgccaggccgcggcggcgtgcccggtgcaggcgatcctgatgggagaggcggtgagtcccggtgcccggtgacctgcgggacggccggatcgtcatcgtcggcgcgtcgctggccggactgcgcgccgcggagacgctgcgcgacgagggcttcaccggttcgctgaccgtgctgggcgaggagccgtggccgccgtacgacaggccgccgctgaccaagcaggtgctcctcggcaccgcggccccggagagcaccgggctgccgatgcgccgggacgtggacgccgactggcggctcggggtacgcgccgacgggctcgatccgatcggcaagcgtgtgctgctggccggcggcgaggcgctgccgtacgaccggctgctgatcgccaccggtacccgggcgcgcccctggccccacccggaacaggccgctctggacggggtactggccgtgcgtacccgcgacgacgccgcgcatctggccgaccggctggccgccggtccgcgccgggtgctggtcatcggcggcggcttcaccggctcggagatcgcctcggcctgccgggaacgggacatcgaggtcacggtcgccgaacgcggccccggaccgctggtgggcgcgctcggcggcacgttggcgaagctcgccgccggcctgcaacgggcccacggcgtggacctgcgctgcggcgtgacggtcaccgcactgcgcggggacgacaagggccgcttcaccggggcggatctctccgacggcagccgcatcgacgcggacgtgtgcgtcatcgcgttgggcgcggtgcgcaacgtcgaatggctggcggactccgggctggcggcgggcccccacggagtcgcctgcgacgccggatgccgtgccttcacccggtacgggatcgtcaccgacgacgtcttcgtggccggtgacgtctcccgcttcccgcatccgctcttcgactaccagatgctctccctggaacattggggcaacgcggtcgcccaggccgaggtggcggcccacaacatggtcagcccggggccgctgcgccgtccgcacctcggcgttccggtgttctggtcgaaccacttcgggatcagcatcaagtccgtgggcgtccccaccttctccgaccaggtggtcgtcgcccaaggctcggtggccgaacgccggctggcggcggtctacggctaccagggccgcgtcaccgccgcggtcaccgtcgacatgggcaagtggctggagcactaccagcgactgatcgagaccgccgccccgttcccgcccgctcccggcgcggccgacggccacccgctgatcagcgaactcccggtgccctccgacgtaccggaccccgcggggctctcccacggccccaccgtcgcgctcaccggtcatctgccggaccgccggctcaccgtgcggcattccggcacctgactcctcagctctgttgtcagtccctcccgtccgaggagccgtcatggccgtcgacaccctgctggagcggatcaccgactacgccagccgtcccgacccctacccgctgtacgcggagctgcgcgaggcgggcgtggcgcggcagacggacggcagctacctgatcggcgggtatcacgacatcgtcgcgttgctgcacgacccgcggctcagttccgaccgccgcaaccgcgccgcgccctaccacggtctgcgcgaggacgaggagacgctggtccccttcctccggctcgacgaccccgagcaccaccggctgcgcgcgctggccatgcggccgttcgggccaccgcacagcccgggccgggtcgacgcgatgcgcggtgaaatcgcccgtatcacccgggaactggccgaggcgttccgcggccgtacgcacctcgacctcgtcgacgacttcgcctacccgctgcccgtcaccgtgatctgccggctgctcggcgtcccgcgcgaggacgagccggtcttccgtgactggtccaccacgatcatcgacgccttcgacgtccggtccggcgaggacgccgacaagcgtcaacgggccggtgcccaggcccgcacggagatgggccgctacctggtggacctcgccgagcggcgccgcggacagccggacgacaccatgctctccgcgttcgtcaacgccccggccgcggacggcgtgctcatccgcgaggaactggcggccaccgcagtcctgttgctggtcgccggacacgagaccaccgtcaacctgatcaccaacggcgtactcaccctgctgcgccaccccgaccagctggaccgactcctgcgggagccgcagctgatgcccacggcggtggaggaactgctgcgctacgagccacccgtacacctgctacaacgcgtacccctcgcccacatagacgtcgcgggcacaaccctccccaagggcgtgccggtggtactcgccgtggcctcgggcagccgcgaccccaggcgcttccagaaccccgaccggttcgaccccacccgccaggacaaccagcacctcggcttcggcagcggcatccacctctgctacggcgcccccctcgcccgcatagaagcccaaaccgccctcacggcactcctgccccacctcagcacagcaacgctcaccgaagacccacccccttaccgccacagcgccctcctgcgcggtcctcggcacctgcccctcgatttggcgtcgcctcgaaataaagggtaa

SEQ ID NO: 85 - protein, 408 aa, Streptomyces rimosus
MAVDTLLERITDYASRPDPYPLYAELREAGVARQTDGSYLIGGYHDIVALLHDPRLSSDRRNRAAPYHGLREDEETLVPFLRLDDPEHHRLRALAMRPFGPPHSPGRVDAMRGEIARITRELAEAFRGRTHLDLVDDFAYPLPVTVICRLLGVPREDEPVFRDWSTTIIDAFDVRSGEDADKRQRAGAQARTEMGRYLVDLAERRRGQPDDTMLSAFVNAPAADGVLIREELAATAVLLLVAGHETTVNLITNGVLTLLRHPDQLDRLLREPQLMPTAVEELLRYEPPVHLLQRVPLAHIDVAGTTLPKGVPVVLAVASGSRDPRRFQNPDRFDPTRQDNQHLGFGSGIHLCYGAPLARIEAQTALTALLPHLSTATLTEDPPPYRHSALLRGPRHLPLDLASPRNKG

SEQ ID NO: 86 - protein, 69 aa, Streptomyces rimosus
MQIVVDLTRCQAYAQCVFLAPEVFRLPREESLLYRPDVPEDQMERVRQAAAACPVQAILMGEAVSPGAR

SEQ ID NO: 87 - protein, 458 aa, Streptomyces rimosus
VPGDLRDGRIVIVGASLAGLRAAETLRDEGFTGSLTVLGEEPWPPYDRPPLTKQVLLGTAAPESTGLPMRRDVDADWRLGVRADGLDPIGKRVLLAGGEALPYDRLLIATGTRARPWPHPEQAALDGVLAVRTRDDAAHLADRLAAGPRRVLVIGGGFTGSEIASACRERDIEVTVAERGPGPLVGALGGTLAKLAAGLQRAHGVDLRCGVTVTALRGDDKGRFTGADLSDGSRIDADVCVIALGAVRNVEWLADSGLAAGPHGVACDAGCRAFTRYGIVTDDVFVAGDVSRFPHPLFDYQMLSLEHWGNAVAQAEVAAHNMVSPGPLRRPHLGVPVFWSNHFGISIKSVGVPTFSDQVVVAQGSVAERRLAAVYGYQGRVTAAVTVDMGKWLEHYQRLIETAAPFPPAPGAADGHPLISELPVPSDVPDPAGLSHGPTVALTGHLPDRRLTVRHSGT

SEQ ID NO: 88 - DNA, 1272 bp, Streptomyces rimosus
atgtccggccacggaccggcggccgtcccgccctgtccggaactgttcacgtgggagttcgccgccgacccgtacccggcgtacgcctggctgcgcgagcacgcgcccgtacaccgcacccggctgcccagcggtgtcgaagcctggctggtgacccggtacgcggacgcgcggcaggcgctcgccgacacccggctgtcgaagaacccggtgcaccacagcgaggccgcgcacggcaagggcaaggtcggcatccccggcgagcggggcgccaacctgatgacgcacctgctcaacatcgacccaccggaccacacccggctgcgccgcctggtctccaaagccttcaccccgcgccgcatcgcccggttcgcgccgcgcgtacaggaactgaccgacgcgctgatcgactccttcgcggagcgcggcgaggccgatctcatccacgagttcgccttcccgctccccatctacgccatctgcgatctgctcggtgtcccgcgcgaggaccaggacgacttccgcgactgggccgggatgatgatccggcacggcggcgggccgcgcggcggcgtcgcccggtcggtgaagaagatgcgcggctacctcgccgagctgatccaccgcaagcgcgaggccctgggggaggaaggggccgacgacctcatctccggcctgatccgcgcctccgaccacggcgagcacctgacggagaacgaggccgccgcgatggccttcatcctgctgttcgcgggcttcgagaccaccgtcaatctcatcggcaacggcgtgtaccagctgctgcgccaccctgaccagcgcgcactgctccagaaggccgctgcggcgggcgatacggagctgctcgccgccggggtcgaggagctgctgcgctacgacggcccggtcgagctggccacctggcgcttcgcgacccgggacctgaccctgggcgggcagcgcatcgccgagggagatccggtcctggtcgtgctcgccgccgccgaccgcgacccgcggcgcttcgcggaaccggacgtactggacctgcgccgccgcgacaatcagcacctcggatacggccacggcatccactactgcctgggcgcgccgctggcccgtctcgaaggccaggccgccatcgccacgctgctgacccggctgccggacctggcactcgccgccgacccggacgatctgcggtggcgcggcgggctgatcatgcgagggctgcgggccctgccggtggagttcacgcccgtacggaagtaa

SEQ ID NO: 89 - protein, 423 aa, Streptomyces rimosus
MSGHGPAAVPPCPELFTWEFAADPYPAYAWLREHAPVHRTRLPSGVEAWLVTRYADARQALADTRLSKNPVHHSEAAHGKGKVGIPGERGANLMTHLLNIDPPDHTRLRRLVSKAFTPRRIARFAPRVQELTDALIDSFAERGEADLIHEFAFPLPIYAICDLLGVPREDQDDFRDWAGMMIRHGGGPRGGVARSVKKMRGYLAELIHRKREALGEEGADDLISGLIRASDHGEHLTENEAAAMAFILLFAGFETTVNLIGNGVYQLLRHPDQRALLQKAAAAGDTELLAAGVEELLRYDGPVELATWRFATRDLTLGGQRIAEGDPVLVVLAAADRDPRRFAEPDVLDLRRRDNQHLGYGHGIHYCLGAPLARLEGQAAIATLLTRLPDLALAADPDDLRWRGGLIMRGLRALPVEFTPVRK

SEQ ID NO: 90 - DNA, 1233 bp, Streptomyces rimosus
atgccatgccccgcgctgcccgacgggttcgacttcaccgaccccgacgtctaccagagccgtgtaccgctgcccgagttcgcgcggctgcggcgtaccacccccgtctggtggaacgcccagccgcacggcatcgccgggttcggcgacgacgggtactgggtggtgacccgccacgaggacgtcaaggaggtctccacccggccggaggtcttctcggcgagcaccaacacctcgatcatccggttcaacgcggccatgacccgcgaccggatcgacgtccagaagctgatcatgctgaacatggacccgccggagcacacccgggtccgccagatcgtccagcgcggcttcacgccccgcgccatccgcgccctggaggacgcgctgcgcacccgcgcgcggaccatcgtcgccgaggcgcggcgcaaggagtccggcgacttcgtcaccgatgtcgcctgtgaactgcccctccaggccatcgccgagctgatcggcatcccccaggacgaccgggcccggatcttcgactggtcgaacaagatggtcgcgtacgacgatcccgagctggccatcaccgaggaggtcggcaacaccgcggcggcggagctgatctcgtacgcgatgaacctggccgcggaccgcaaggagtgccccgcccaggacatcgtcagccggctcgtcgcggcggaggacgagggcaacctcgcgtccgacgagttcgggttcttcgtcctgctgctggccgtcgcgggcaacgagaccacgcgcaacgcgatcacgcacggcatgcacgcgttcctgacgcaccccgaccagtgggagctgtacaagcgcgagcggccgagcaccacggccgaggagatcgtgcgctgggcgacgcccgtcgtctccttccagcgcacggccacccaggacaccaccctgggcggcgcgcggatcgaaaaggggcagcgcgtcggcctcttctacgcctccgccaaccacgaccccgaggtcttcgcgcacccggagacgttcgacatcacccgcgaccccaacccccatctgggcttcggcgggggcggcccgcacttctgcctcggcaagtcgctcgccgtcctggagatcgacctgatcttccaggccatcgccgacgccatgccggacatcgccctcgtgggcaccccgcgccggctgcggtcggcgtggctcaacggggtgaaggagctgcgggtccggtacgtgtaa

SEQ ID NO: 91 - protein, 410 aa, Streptomyces rimosus
MPCPALPDGFDFTDPDVYQSRVPLPEFARLRRTTPVWWNAQPHGIAGFGDDGYWVVTRHEDVKEVSTRPEVFSASTNTSIIRFNAAMTRDRIDVQKLIMLNMDPPEHTRVRQIVQRGFTPRAIRALEDALRTRARTIVAEARRKESGDFVTDVACELPLQAIAELIGIPQDDRARIFDWSNKMVAYDDPELAITEEVGNTAAAELISYAMNLAADRKECPAQDIVSRLVAAEDEGNLASDEFGFFVLLLAVAGNETTRNAITHGMHAFLTHPDQWELYKRERPSTTAEEIVRWATPVVSFQRTATQDTTLGGARIEKGQRVGLFYASANHDPEVFAHPETFDITRDPNPHLGFGGGGPHFCLGKSLAVLEIDLIFQAIADAMPDIALVGTPRRLRSAWLNGVKELRVRYV

SEQ ID NO: 92 - DNA, 1230 bp, Streptomyces rimosus
atggacgcgcgggtccgccacagccccgaggccgagcgcatcgacacccgcggcgaaccgccggtgtggcgcgcggagctgcccgacggctccaccgcctgggtcgcgtccgggtacgacgccgcgcgccaggtgctgacggactccggcttcgcgaaaccggccgtccggggcggcgagcgctggacggactatctggccttcaccggcaaggaggtcaccgacagcatcgtgcgcagcatgctcaacaccgacggcgacctgcaccggcagctgcgcgaactgggcgcgtcggcgttcacgcccgagcgggtgcgggagaccgccgaccgcgcggaaacgctcgccgagaccctgctcgacgagatcgcgggacgcggccgcgccgacctcgtccacgaattcgcccaccccttcgccgtccgggccatcaccgaacacctcggctatccgcccgatttcatccggcgcgccctggagctgcggcgctggggcccgtccccgctgttcgatccccccggctccccggaccgcgcgcgctacgccgccgaccgcacggccatgagcgagctgctgcacgacctggtggccttccggcgcggcagccccgggcccgacgccgtcagcgggatgatcgcgcgcgccgacgccgcgggcctggacgaagggcagctgacctccaccctcttcctgctgctcgtctccgcctacgaaccggtcgccgacttcctcacgtcgagcctgtactccctctggcaccgccccgacctgctcgccgaccccgcccgggtggccgacggcctcggcgagctgctgcgctacacctccccgctggccgccaccatgccgcgcttcgccacccgcccgatggagctgtacggcgccgagctggcgccgggggacgcggtgatcgtgcacctggccctcgccaaccgcgacccgcgccgcttcaccgcccccaaccgcctcgacctcgaccgggaaaccggccaggacctggtcttcgcgcacggcccgcacttctgcctcggcagccagttcgcggtccggctgtgccgtacggccctcggcgccgtgctgcgccgcctgcccggactcgccgccgcccggccgctcgacacactgccctggcagcgcggctccacgggcggcatcacccatctgcacgtcaccgcgggcctgacggagctgcccgtcaccttccagccccggcacgcggtggtctcctaa

SEQ ID NO: 93 - protein, 409 aa, Streptomyces rimosus
MDARVRHSPEAERIDTRGEPPVWRAELPDGSTAWVASGYDAARQVLTDSGFAKPAVRGGERWTDYLAFTGKEVTDSIVRSMLNTDGDLHRQLRELGASAFTPERVRETADRAETLAETLLDEIAGRGRADLVHEFAHPFAVRAITEHLGYPPDFIRRALELRRWGPSPLFDPPGSPDRARYAADRTAMSELLHDLVAFRRGSPGPDAVSGMIARADAAGLDEGQLTSTLFLLLVSAYEPVADFLTSSLYSLWHRPDLLADPARVADGLGELLRYTSPLAATMPRFATRPMELYGAELAPGDAVIVHLALANRDPRRFTAPNRLDLDRETGQDLVFAHGPHFCLGSQFAVRLCRTALGAVLRRLPGLAAARPLDTLPWQRGSTGGITHLHVTAGLTELPVTFQPRHAVVS

SEQ ID NO: 94 - DNA, 1518 bp, Streptomyces rimosus
atgggtatacgtggtgcggcgggcgtccgcgcggcccgcggtcccgccccgcacagctggaccgtgtcgacggcacccggcggcgtaccgctgctgggacacgcgctcccgctgtggcggcgcccgctggacttcctcgcctcgctgcccgcgcacggcgacctggtcgcgatccgcctcggaccgcagcgcgtgtggctcgcctgcgacccggcgctggtgcagcagatcctcatggacccgcgcacgtacgacaagggcggtccgctctacgacaccatgcgcatggtgctcggcaacgggctggtcacctgcacccaggacgtgcaccgcaggcagcgccggctggcccagccctgcttccgcccgtcccggatcgccgactacgcgcaggtgatgagcgccgagatcgacgccgccgtcggaaagtggcggcccggacagacgctggacgtcaccgacgcgatgatggacctctcggcccgggtcaccaccggcgtgctgatgtccacgtccctcgacccgggcctcgccgccgaggtacgcgcctgcctgtcgaccgtcatgcgcggcgtcctgctgcgcgcggtcgtcccgctcggcccgctctacagactccccacgcccggcaaccgccgcttcgaccgggctctcgcccggctgcaccacatcatcgacgggatcatcgccgaacgccgcggcagcaccgcccggcacggcgacctgctcgacaccctcctgggagccacggacgacgcccccggaccggacggccgcgccgtacccgaaggccttgcccaggactgcccccacgccaccgccgcgcccaccccccaggaggcaccccacgatcaggaaccgctcaccgaccaagaggcgcacgaccagttgatgaccttcctcgtggccggcatcgagaccaccgcgctggccctcgcctggacgctccacctcctggcggcccaccccgaggaagaacgccggctgcacgccgaggtggactccgtgctcgccggccggccgcccgcgccggacgatctgccccggctcggccacgcccggcgcgtggtcaccgaagccctgcgcatgtacccgccgggctgggccctgacccgggtgaccaccaccgagaccacgctggccggccaccggctggcaccgggaagcaccgtcctgtacagcgcgtacgtgctccaccaggacccggtggccttccccgacccccagcgtttcgaccccgaccgatggttgccggaacgggcagggggcgttccgggcggtgcgatgctcccgttcgccgccggcaaccgcaagtgcatcggcgaccacttcgcgatgaccgaagccgtgctcgtccttgccgccatcgccgcgcgctggcgcctgcgcccgccgtcccccaggaccgtacgaccggtcccggcggccgtgctgagcccgggcccgctgcccatggtctgcgcctcacgccgcggaccggacggcccagcgccggccgtgccatctgaagcaccgtaa

SEQ ID NO: 95 - protein, 505 aa, Streptomyces rimosus
MGIRGAAGVRAARGPAPHSWTVSTAPGGVPLLGHALPLWRRPLDFLASLPAHGDLVAIRLGPQRVWLACDPALVQQILMDPRTYDKGGPLYDTMRMVLGNGLVTCTQDVHRRQRRLAQPCFRPSRIADYAQVMSAEIDAAVGKWRPGQTLDVTDAMMDLSARVTTGVLMSTSLDPGLAAEVRACLSTVMRGVLLRAVVPLGPLYRLPTPGNRRFDRALARLHHIIDGIIAERRGSTARHGDLLDTLLGATDDAPGPDGRAVPEGLAQDCPHATAAPTPQEAPHDQEPLTDQEAHDQLMTFLVAGIETTALALAWTLHLLAAHPEEERRLHAEVDSVLAGRPPAPDDLPRLGHARRVVTEALRMYPPGWALTRVTTTETTLAGHRLAPGSTVLYSAYVLHQDPVAFPDPQRFDPDRWLPERAGGVPGGAMLPFAAGNRKCIGDHFAMTEAVLVLAAIAARWRLRPPSPRTVRPVPAAVLSPGPLPMVCASRRGPDGPAPAVPSEAP

SEQ ID NO: 96 - DNA, 1341 bp, Streptomyces rimosus
atgggtacgcacattcctggacccgaaccccggccggacggcggggtggatgctgtcgcggcggcgggtgggctgcaccggtatcagttgtggctgcatgccgagtacgggcccgtggtgcggttccagctgccgggggcggagacggccgtttcggtggcggatccggtgctgctggaggccacggcgcacatcgacaagcggccggagcggttgttcgagtttctggcaccgctgtgcgaggcgggcaatctgcaggtgttgccggccgaggagcacaccccgtggcgtcgggtgctgttgtcggtgctggccgggcggccgtcgcacgaacggcacttcgagcggttcaccgagctgacgacgtccctcgcggaccggtgggccgggcagggcgaacaggaaccggtcgcgttgcagaaggaactgaccgcactgtcgttgcggatgatcggtgcgtacgcgctggggggcgacgcggcggatccggagaaggtcatcgcggccttcgaggaggtgctcaccgagtatctggggcggctctaccaggtgcccgtgccgggtacggaggaggagcgcgcccggcgggcggagcaggccctcgcgtatctgcgggcgaccgtcgaccgggtgctgacggcgcaccgccctgacagccgtacggaccggagcgatctgatcggggccctcgtggcggccggtgaggacccggcgcggatccgtgacacggtgatggtggcgatgctggccgcgcaccacacgacgggcgtggccgtgtcgtggaccctgcacctgctgggacgccaccccgaggtggccgaacgcgtcgccggggagctggaccgcgtgctcggcgaccgtgcggtgcccgggtacgccgatctgcggcgcctgacgtatctggacatggtcctgaaggagtcgatgcggctgttcccgcccggtccgtacggtgcacgggagacgaccgaggcgctggtcctgggcgcgtacgaggttccggccgggacggtgatcttctatccgttctgggccgtccatctgaaccccgatcactggcccgagcccgagaggttcgtgcccgagcggttccttccggaagaggtggccaagcgtccgaggctggcgtacatcccgttcggcctcgggccgcgcagctgtgagggcgccggtctggccacggtcgaggcgcaactggtcctggccgtactgctcaagcgcttccggttccggcctgtgccagggcatgaggtgacgccgatcgagcggttcgtgctgtgggcggccgatgacatccggatgttcgtgagtcggcgggaggtgggggcggggagcccgtaa

SEQ ID NO: 97 - protein, 446 aa, Streptomyces rimosus
MGTHIPGPEPRPDGGVDAVAAAGGLHRYQLWLHAEYGPVVRFQLPGAETAVSVADPVLLEATAHIDKRPERLFEFLAPLCEAGNLQVLPAEEHTPWRRVLLSVLAGRPSHERHFERFTELTTSLADRWAGQGEQEPVALQKELTALSLRMIGAYALGGDAADPEKVIAAFEEVLTEYLGRLYQVPVPGTEEERARRAEQALAYLRATVDRVLTAHRPDSRTDRSDLIGALVAAGEDPARIRDTVMVAMLAAHHTTGVAVSWTLHLLGRHPEVAERVAGELDRVLGDRAVPGYADLRRLTYLDMVLKESMRLFPPGPYGARETTEALVLGAYEVPAGTVIFYPFWAVHLNPDHWPEPERFVPERFLPEEVAKRPRLAYIPFGLGPRSCEGAGLATVEAQLVLAVLLKRFRFRPVPGHEVTPIERFVLWAADDIRMFVSRREVGAGSP

SEQ ID NO: 98 - DNA, 1224 bp, Streptomyces rimosus
atgaccaccccccagcaccccgacgacttcctgcgtctcctgcgaatgcgcagcgcggccgaggacgggatcttccgggtcgacgaggaacggctcgccgtgttcgatccggaagcggcccgccggatcagcgccgcgaactggcaccggttcgtcatgcacgaccgcctggtcgacatggtgcggcggcgccggagtcccgaggtgcggtggagccaggtacggtccgcctggctcacccagctgcacgcgctggccacgccggaacagcacggccggctgatcgagcgcatggcacagatcatggacgcgcggctcggccgggacgtggatctcaccatgctcagccaggacgtggccgtgcggtcgctgctgccgctcgcgctgtcgggcctcaccaccggcgaggcggatctcgtccgccgggacctggagatgaagctgctgcggctggtctcgcccgacccgggcagcacctggcaccacctgcggttcgtcgcggtccagatacggtcgggactggtcgtgcgccgggtcctgcgccaacgcgcccgcgggcgccggggccgcgagccggacctcgccgacccgatcgtcgacctgctgcccgcactcggcatggaccgcgccctggacgtggtgacggccgtcctcaccgccatcggcggcccgccgggcacggccgccgcgagcgtgctgtacgagttcgcccgccgccccgagtggcagcggcggctcgccgatgagctgggcgccgtcgaccccgtcgcgttccgtacggcaccgccggacgcggccccggtgacccaccgcttcgtcaaggaagtgctgcgcctgtggagtccgccgctgctgctggtacgacgctccacggtcccgttcgacctcgggaagacacgcctggcgccgggcgactggtacttgctgagcccgcacatgatccatcgcgatgaccgcgtctggaaacggcccgacctcttcgacccggaccgatttctgcccggtgcgccccacggcccggcggaccgcacgtgctacgtgccgttcggctgggcgcccaagaagtgcatcggcgcgaacatcgccatcgtccagctgatggccctgtgccacctgctgtgcacccggtaccgcctgaccgtgcaccggccggacgaggtcacgatggccttgcgtttcgctccggtaccggagaacttccggggggagctggccttccggtaa

SEQ ID NO: 99 - protein, 407 aa, Streptomyces rimosus
MTTPQHPDDFLRLLRMRSAAEDGIFRVDEERLAVFDPEAARRISAANWHRFVMHDRLVDMVRRRRSPEVRWSQVRSAWLTQLHALATPEQHGRLIERMAQIMDARLGRDVDLTMLSQDVAVRSLLPLALSGLTTGEADLVRRDLEMKLLRLVSPDPGSTWHHLRFVAVQIRSGLVVRRVLRQRARGRRGREPDLADPIVDLLPALGMDRALDVVTAVLTAIGGPPGTAAASVLYEFARRPEWQRRLADELGAVDPVAFRTAPPDAAPVTHRFVKEVLRLWSPPLLLVRRSTVPFDLGKTRLAPGDWYLLSPHMIHRDDRVWKRPDLFDPDRFLPGAPHGPADRTCYVPFGWAPKKCIGANIAIVQLMALCHLLCTRYRLTVHRPDEVTMALRFAPVPENFRGELAFR

SEQ ID NO: 100 - DNA, 1467 bp, Streptomyces rimosus
atgactttcccttttcccgaacagcccggcaccacgtgggccgccacgccgcctccggagtgcccggcacacgcccggcccggcgccgccgacgggctggcgcggctcttcggccccgaggcggccgccgaccccatgggcctgtacgagcgcctgcgcgcccggcacggggccgtcgcgcccgtcctgctggacggcgacctgcccgcctggctcgtcctcggctaccgagagatcctggaggtcgccggtacgcccgcccgtttcagccgcgattcgcgcaactggcgctggttcagggaggggcgggtcccgccggactcgccgctgctcccgatgatcgcctggcagccggtgtgcctgttcctggacggggaggagcgcaaccggctgcgcctggccgtcaccgacagcctggaccgcttcaaccgccggggcatccggcggcacatcacccgcttcacccaccagctggtggacggcttcatcgagcgcggggaggcggacctggccgaggagttctgcgaacacctgcccatgctcgtgctgacccagctcctgggcatgccggacgagtacgggccccggctggtcgcggccagccgggacatggtggcgggcaccgcgacctcggtggccagcaacgcgttcatcgtggacaccctcatggagctggtacggagcaagcacaccacccgcgggcacgacatcacgtcctggctgatcgaccactcctcccggctgaccgacgaggaggtgtggaaccacctgcgggtcgtcctgatcgccgcgaacgagaccaccgtcaacctcctcaagagcacgctgcggatggtgctgaccgacccccggtgccacgcgtcgctggccggcgggcagatgacgctgcccgacgtggtggagcaggtgctgtggagcgaaccgccgctgatgaccatccccggccgctgggccgcggtggacacggaggtcggcggccagaagatcgaggcgggggacatgctgctgctcagcctggccgccgggaaccacgatccggccgtccggccggacccgtcgatcccgctgcacggcaaccgctcgcacctcgccttcagcagcggcccgcaggagtgccccggccagaacatcggccgcgccatcgccgacaccggcatcgacacgctgatggcacggctgcccgacgtacggctgcgcatccccgaggaggagctgcgctggacgtcgggctggatgacgcgccatctgaccagccttccggtgacgttcagcgcctcccggcccgcgcactccggcgcgaccgccggtacggccttcgaacgcccgccgggcaccaccccgcacgacggctccctgcccgcggccgagcccccggccacgcccccgcccggcccgcctccggcggctcccgtgcccagggggcgtacgtcctggtgggccgcgttgaaggcttggctgcgcggctaa

SEQ ID NO: 101 - protein, 488 aa, Streptomyces rimosus
MTFPFPEQPGTTWAATPPPECPAHARPGAADGLARLFGPEAAADPMGLYERLRARHGAVAPVLLDGDLPAWLVLGYREILEVAGTPARFSRDSRNWRWFREGRVPPDSPLLPMIAWQPVCLFLDGEERNRLRLAVTDSLDRFNRRGIRRHITRFTHQLVDGFIERGEADLAEEFCEHLPMLVLTQLLGMPDEYGPRLVAASRDMVAGTATSVASNAFIVDTLMELVRSKHTTRGHDITSWLIDHSSRLTDEEVWNHLRVVLIAANETTVNLLKSTLRMVLTDPRCHASLAGGQMTLPDVVEQVLWSEPPLMTIPGRWAAVDTEVGGQKIEAGDMLLLSLAAGNHDPAVRPDPSIPLHGNRSHLAFSSGPQECPGQNIGRAIADTGIDTLMARLPDVRLRIPEEELRWTSGWMTRHLTSLPVTFSASRPAHSGATAGTAFERPPGTTPHDGSLPAAEPPATPPPGPPPAAPVPRGRTSWWAALKAWLRG

SEQ ID NO: 102 - DNA, 1227 bp, Streptomyces rimosus
atgctggaacagctgcgcaggcagtacggggacgtcgcaccggtcctcgtccccggcgacatcccggcctacctggtcctgggatacaacgcgacacgcgatgtcatgcagagcaactcccgcgtggtctgcgactcccgccgcggccgtgtctaccaggacggccggatcccggcggaccaccccctggcgccgatgaccgcgtaccagccggtcgtggcgttcgaggacggcgtgccccacgcccgcctgcgcagcgccgtggtcgacagcctggacttcaaccggcactccctgcgccgctacatcggccggtacgccaaccgcctcatcgactgcgtcgcctcccgcggcaccgccgacctggtcagcgagtacgccgcgcagctgccggccctcgtgatggcctggatgtacggcatgcccgaggaggagagccccgccctggtggccgcggtacgggacctgaccagcggcaacgagcgggccgccgagggcaacgcgttcgtcacccgcacgatggaggaactcgtccggcgcaggcgggccggcgagggcgccgacaacaccatcggcggccgggacttcgtcagccgtctcctggaccacgaggcgggcctcagcgatcaggaggtcgtcgagcacctgcgcatgatcttcgtcgccggctacacgccgacggtcgcgctgatcgcaaacacgctgctggtgctgctgacccagcgtcagttcagccgtgacctgaccagcggccagatgacgctgcccgaggccctggaacgcgtgctctgggaccacccgccgatcgggctgctgcccacccgctgggcggccggggacatgaccatcgccggccagcagatcaaggccggagacatgatcatcctggggatcgaggctgccaacgcggaccccgccgcccgggaacccggacgccccgtagtccacaattcgggacacctcgccttctccaccggcccccacgagtgtcccggccgcgacatcggacaggccatcgcggagaccggcatcgacatcctgctgagcacgctcagggacctggaactggcggtgcccgaggcagagctgcagtggcagtcggcttgggtctcgcgtcgcctgctgtccttgccggtgacgttcactccgccgcgggtcaggggggtgcgggctccgcagccggaggctgctgtggcgggagtgggtaggtcggttggtactgcctaa

SEQ ID NO: 103 - protein, 408 aa, Streptomyces rimosus
MLEQLRRQYGDVAPVLVPGDIPAYLVLGYNATRDVMQSNSRVVCDSRRGRVYQDGRIPADHPLAPMTAYQPVVAFEDGVPHARLRSAVVDSLDFNRHSLRRYIGRYANRLIDCVASRGTADLVSEYAAQLPALVMAWMYGMPEEESPALVAAVRDLTSGNERAAEGNAFVTRTMEELVRRRRAGEGADNTIGGRDFVSRLLDHEAGLSDQEVVEHLRMIFVAGYTPTVALIANTLLVLLTQRQFSRDLTSGQMTLPEALERVLWDHPPIGLLPTRWAAGDMTIAGQQIKAGDMIILGIEAANADPAAREPGRPVVHNSGHLAFSTGPHECPGRDIGQAIAETGIDILLSTLRDLELAVPEAELQWQSAWVSRRLLSLPVTFTPPRVRGVRAPQPEAAVAGVGRSVGTA

SEQ ID NO: 104 - DNA, 1425 bp, Streptomyces rimosus
atgaacaccctccgcaccgccaagctgctcgccgccgcggccggtctcctctccgtcccgtactggctgccgcgctccgtcgtcgccgcccgcgtcgcgctcttcgcgcggatcaacggcgacgagggcatcgccttcccgagcgccgacgtccccgccgaccgcttccaggagatctactcccaccccgccgccaacggccgcagccggggcgccgccctctcggacctcttctggtactggctggcgcccggccccgaggtgcaccaggagcacctggaggacggcccgcgctacgacgaggtcgcccgtaccaccctcgccgtgctgggcggtcccagccgcgagctgtccgccgcggtggcccgccgtaccgccgccgtgctcgacgaactggtcaccggccgggccgagttggtccggctgcgcgacctgatgatgccggtgtgggcggagttcttctacggactcgtgttccgcgaaccgtgcccgccgtacgtccggcgcctgatcgtggacaacgccgccgacgtggtcaactccctgaagtgcacccggctccgccacccggcccgccgcgcccgcctcacccgccacctgcggcagcgcatcgccgccgggaccgtaccgccgcaccacctgccgggctccctcacgcccgacgagcaggcgtactacctccagggcaccttcttcaacacggccatcgtccagatgtccgaggccatggcccacctgctgctggtcctcgcccagcacccggaggcgcagcgcaggctcgccgccggaccggacgacgaccggtacttctccaacgtcctcaacgagacgctgcggctctacccgctcttcggcgtcgcccaccgcatcagcacggacgacatcccgctcggccccggcacggccatccccgccggctccgtcctgtgcttcaactaccccgactaccacgccaccggctacaccgaccccgaggtcttcgaccccgcccgctgggaccgcctggtggccaaggagcagcaccacatcccgttcggcgtcgccgccaaccggccgtgcccggcctggcggctcgccccgctggccatgcacgccgcgacccgcgaggtgctgcgccgcttcaccctccactccaccgtcgcccacacccgctccatcccgcaccgcgccccctgcctgctggtccggcgcgaccgtccgctgccgaagcaccggctgctcgccgcccgggtcttcctgagggtgcgcgaccggtgggaggacgtgtggcgcagctgcgtccagctcgtcctcggtacgtggatggtgctcgacgcccgccgcctgcgcccggccgagcgctacttcgccacccacgacacgcagggcgtcccgctgccgggcaccgcccccgccccggcgcgctgtccgtacccgcacgcctaa

SEQ ID NO: 105 - protein, 474 aa, Streptomyces rimosus
MNTLRTAKLLAAAAGLLSVPYWLPRSVVAARVALFARINGDEGIAFPSADVPADRFQEIYSHPAANGRSRGAALSDLFWYWLAPGPEVHQEHLEDGPRYDEVARTTLAVLGGPSRELSAAVARRTAAVLDELVTGRAELVRLRDLMMPVWAEFFYGLVFREPCPPYVRRLIVDNAADVVNSLKCTRLRHPARRARLTRHLRQRIAAGTVPPHHLPGSLTPDEQAYYLQGTFFNTAIVQMSEAMAHLLLVLAQHPEAQRRLAAGPDDDRYFSNVLNETLRLYPLFGVAHRISTDDIPLGPGTAIPAGSVLCFNYPDYHATGYTDPEVFDPARWDRLVAKEQHHIPFGVAANRPCPAWRLAPLAMHAATREVLRRFTLHSTVAHTRSIPHRAPCLLVRRDRPLPKHRLLAARVFLRVRDRWEDVWRSCVQLVLGTWMVLDARRLRPAERYFATHDTQGVPLPGTAPAPARCPYPHA

SEQ ID NO: 106 - DNA, 1056 bp, Streptomyces rimosus
atgcgtacgtacggtacggaacggagcgaccgggtcacggtcttcacgccgcggctcggccggctcctcagtgagcaccgcggcgcggacgtcttccggctggaggccgacacggtcggcgtcgccggacccgggctgatcgacgccgtgctgcgcagcagaccggccaacgcggccgaacggcccactttcaaacccctacagggccggcccatcagccgccccgaatcctccgcggtcatgcgggccgtttccctggacgtgcgcgcggcactggaaaagcccgacgggaaaggcggcccggcggccgatctgtcgggggaatggccgcgggtggcacacctttatctgcgggacctggttttcgggtccgatccgatgcggctgcgcgtactcgtggaccgcaagctggaatggacgcccaaactgacgtggaccgtgatcgcggcgggcgcggcgctgccgggctgcccgggggccggtgcgccggtgtcccggctggcgggtctcgccgccgccgcggccggttacggggaccggcggtacgcgatgggcctgtaccggcgggcggcggcaccggtgtgcttcaccgtgtccacgctggtcgccaacgccctctggctcgggtcgcccttcgaggaccacataccgaaccgtcacatcctgtacgagtcgatgcggctgctgccgccttcgtggaacctcctgcgcgtggcgtcaccggagttcgcggccctcgacgaccggatcggcgcgggcgacgacgtcctgctgctgccgctgctcagccaccgcgatccgcggctgtgggacgcgccggacgcgttccggcccgagcgctgggcggccctcgacgccgacgaccagcccggctacctgcccttcgggcacgcgaacgagcggtgctgggggcggcacatggtcatgccgctggccgaacggctgctggacctggtgcgggaacagggcctggcggtgagcccggagcagaagtccgccgaggtgccgctggccgggctgctcggggtgtcgcgggtgtcggtcgtacggcgctaa

SEQ ID NO: 107 - protein, 351 aa, Streptomyces rimosus
MRTYGTERSDRVTVFTPRLGRLLSEHRGADVFRLEADTVGVAGPGLIDAVLRSRPANAAERPTFKPLQGRPISRPESSAVMRAVSLDVRAALEKPDGKGGPAADLSGEWPRVAHLYLRDLVFGSDPMRLRVLVDRKLEWTPKLTWTVIAAGAALPGCPGAGAPVSRLAGLAAAAAGYGDRRYAMGLYRRAAAPVCFTVSTLVANALWLGSPFEDHIPNRHILYESMRLLPPSWNLLRVASPEFAALDDRIGAGDDVLLLPLLSHRDPRLWDAPDAFRPERWAALDADDQPGYLPFGHANERCWGRHMVMPLAERLLDLVREQGLAVSPEQKSAEVPLAGLLGVSRVSVVRR

SEQ ID NO: 108 - DNA, 1412 bp, Streptomyces rimosus
atgaccacagccgacacgatgccccttgcctacccgttcaacgacgccgacggactggctctgtccgagacctacgaacaggtccgcgaccggcccggactgctccgggtacagatggcgtacggcgaaccggcctggctcgccacccgctacgccgacgcccggctggtcctcggcgaccggcgcttcagccgcgcggaagggctcgaacgcgacgagccgcggcagtcggagggccagcgggacagcgggatactgagcatggacccgcccgaccacacccggctgcgcaccctggtcgccaaggcgttcaccgtgcaccaggtggagaaactccggccgtgggtgcgcgagttgacacacggcctgatcgacgagctggaggccgcgggcccgcccgtggacctcgtggaccgctacgcgctgcccatcccggtcgcggtgatctgccggatgctcggcgtaccggaagaggaccggcccaagttccgtacgtggagcgacgccgcactgtccaccagctcgctgacggccgaggagttcgaggccaaccgcgaggaactgcgcgcctacatggcgaagttgatcgaggatcaccgcacgacgccgcgggacgacctgatgacgcggctgatcgaggcccgggacgtcggcgaccggctctccgagctggagctgatcgacctgtgcgtcggcatcctggtcgccggacacgagacaacggccacccagatccccaacttcgtcctgtcgctgctggaccacccgggcgagctggagcggctgcgcgccgaacccgcgctgatcaagagcgccgtcgaggaactgctgcgcttcgtaccgctcggcagcggcgcgggcttcccgcgctacgccaccgaggacatcgaggtgggcggcacactcgtccgtgcgggtgaaccggtactggtcgccgtcggcgcggccaaccgggacgcgctgcgcttcgacgagccgggcaccctcaacatcacccgcgacggcaaccagcacctcggcttcggacacggcgtgcaccactgcctcggcgcgccgctggcccggctggaactccaggaggcgctgatcgccctgatcacccggttcccgaagctgcatgtggccggggacgtggtgtggaaggaccagatgctggtccgcggcccgcgcgtgatgccggtggggtggtgagccggatgacgtggaaagcggcgatcgacggacagcagtgcatggcgtccggcatgtgcgcgggcatcgccccggacctcttcgtcctggacggcccgcacgcccgaccgctccaggaggagatccccgaggacgaggccgcgctcgacgcggcggactcctgccccgccatggcgatcctgatccgggacggggagaaggtggtggggccgcggccctaa

SEQ ID NO: 109 - protein, 396 aa, Streptomyces rimosus
MTTADTMPLAYPFNDADGLALSETYEQVRDRPGLLRVQMAYGEPAWLATRYADARLVLGDRRFSRAEGLERDEPRQSEGQRDSGILSMDPPDHTRLRTLVAKAFTVHQVEKLRPWVRELTHGLIDELEAAGPPVDLVDRYALPIPVAVICRMLGVPEEDRPKFRTWSDAALSTSSLTAEEFEANREELRAYMAKLIEDHRTTPRDDLMTRLIEARDVGDRLSELELIDLCVGILVAGHETTATQIPNFVLSLLDHPGELERLRAEPALIKSAVEELLRFVPLGSGAGFPRYATEDIEVGGTLVRAGEPVLVAVGAANRDALRFDEPGTLNITRDGNQHLGFGHGVHHCLGAPLARLELQEALIALITRFPKLHVAGDVVWKDQMLVRGPRVMPVGW

SEQ ID NO: 110 - protein, 71 aa, Streptomyces rimosus
MTWKAAIDGQQCMASGMCAGIAPDLFVLDGPHARPLQEEIPEDEAALDAADSCPAMAILIRDGEKVVGPRP

SEQ ID NO: 111 - DNA, 1095 bp, Streptomyces rimosus
atggcgtggctccaggacgcggacgcgcccagttggttcgtgagccggtacgacgacgtccgtgcggtgatcggggatccacggctggtcaggccgagtgtcaacggctggtccttcatgccggagcaggaccggccggacggcatggaactgatcacgatgatggagatggagggcccgcggcacacggcgctgcgcagggccctgtccggggcgttcagcgcacggtccgtacggcgccgtctgccgcgtatccgccggagcgccgagcggctgctggacgagttcgccgacggcggcgcacccggcgatctgatcgccggttacaccgagccctttccgctgctggtggtgtgcgaatcggtgggcatcccgtacgaggaccgcgactactacctgcccatggcggacgcggctctgggggcgctgctcaccgtggaggaggcgcggcgggtcacgccgctgctacgggactacgtccggtcactgatcgtccaacggcggcgggcgcccgcggacgacatcctcggcgacctggtccgcaggtgtgaccggggcgagctggacgaggagagcgtgctcagcttcgggctgtcgatgctcgtcgccggttaccgcacgacgaccatgttcctgtccgacgccgtcctggcgctgctggccgatccggaccagtacgtccggctgcgcgacgaccgcggcctgctgcccggcgcggtggaggagttcctgcgctacgtcccggcgatgaacggggtggtggtgctgcaggccaccgaggacttcgaactgggcgggcagacgatccgggcgggggacgcggtcctgccggcactggcctccgccaaccgcgacgagaccgtgttcgatgagcccgaacggctcgatgtgtgccggcggccgaacccgcacatcgcgttcggccggggcccgcacaactgcatcggcgcccacctggcgcgggcggagctgaccgtgggcctggaaacgctcctggaccgtttcccgcacctgcgcctggccgagggacacagccccacctgggacgacgcctccccgtccaagtcgcctctcacccttccggtcagctggtaa

SEQ ID NO: 112 - protein, 364 aa, Streptomyces rimosus
MAWLQDADAPSWFVSRYDDVRAVIGDPRLVRPSVNGWSFMPEQDRPDGMELITMMEMEGPRHTALRRALSGAFSARSVRRRLPRIRRSAERLLDEFADGGAPGDLIAGYTEPFPLLVVCESVGIPYEDRDYYLPMADAALGALLTVEEARRVTPLLRDYVRSLIVQRRRAPADDILGDLVRRCDRGELDEESVLSFGLSMLVAGYRTTTMFLSDAVLALLADPDQYVRLRDDRGLLPGAVEEFLRYVPAMNGVVVLQATEDFELGGQTIRAGDAVLPALASANRDETVFDEPERLDVCRRPNPHIAFGRGPHNCIGAHLARAELTVGLETLLDRFPHLRLAEGHSPTWDDASPSKSPLTLPVSW

SEQ ID NO: 113 - DNA, 1215 bp, Streptomyces rimosus
atgagccaccccgaagccctcataccggtcccggaggtcgagcccggtaccgcggggccgccgtgcgcctacgcccggctgcggaccgaggcgcccgtggtcaaggcgcagctgcccaacggcgagacgggctggctgatcagccgctacgaggacgcccgcgccgcgttcgccgacccccggctcgtacggccgctgctgtcggcctggccgccccgcgagggaagcgacgccccgccgccgtgcctgcccaccttcctggagatgaccggcgcccaccacgaacgcgtgcgccgcaccgtactgccgctgttcggcaggcggcggctcgccttcatggagccccgcgtccgggcgatggcggaggaactcctcgacacgatggtggccggggccgacgggggagtggcggatctcgtcgcctcctacgccgagccgctgccgctgcgggtgctgtgcgcgaccgtcggcctgccgtacgaggaccgcgagacctacctgccgcacaccctcgcgctcctgggcgcgtccggcctcacgatggaggaggtactcgcggccctgtacgcgctgcaggactatgcggacgacctcatctcccgtaaggagaagacggacggcgaggacgaggactacatccggctgctgctggcggaggcacgccggccggacagcgagatcacccgcgacgacgtcgtcagcttcgtcgtcaccatgctgatggccggctacaagaccaacatccagcacaccggcaacgccctgctcgcgctgctcacccaccccgagcagctgaaggcgctgcgcgaggcgcccgagcggaccggcgccgcggtggaggaactgctgcggtacgtcccgctgatgaacgccatcaacatcctcgtcgccaccgaggacttcaccctccacgggcagaacatcagggccggggacgcggtcgtgcccgtaccggcgtccgccaaccgcgacccggacgccttcgccgaacccgaccgcctcgacctgacgcggactccgaacgcgcacatcgcgttcgggcacggcccccacgcctgcaccggcggccacctgacccgtatgcagctcggtatcgccatccaggtactgctggaacggctgcccggcatcgaactggccgtcgcggcggacaccatcccctgggacgagtccactccactgcgcgcaccggcccggctccccgtgcgctggtaa

SEQ ID NO: 114 - protein, 404 aa, Streptomyces rimosus
MSHPEALIPVPEVEPGTAGPPCAYARLRTEAPVVKAQLPNGETGWLISRYEDARAAFADPRLVRPLLSAWPPREGSDAPPPCLPTFLEMTGAHHERVRRTVLPLFGRRRLAFMEPRVRAMAEELLDTMVAGADGGVADLVASYAEPLPLRVLCATVGLPYEDRETYLPHTLALLGASGLTMEEVLAALYALQDYADDLISRKEKTDGEDEDYIRLLLAEARRPDSEITRDDVVSFVVTMLMAGYKTNIQHTGNALLALLTHPEQLKALREAPERTGAAVEELLRYVPLMNAINILVATEDFTLHGQNIRAGDAVVPVPASANRDPDAFAEPDRLDLTRTPNAHIAFGHGPHACTGGHLTRMQLGIAIQVLLERLPGIELAVAADTIPWDESTPLRAPARLPVRW

SEQ ID NO: 115 - DNA, 915 bp, Streptomyces rimosus
atgggcccgggcgcgctcaccgacccggactgggtggtgccgccggtgccccaggacgtaccggagggcgggatggcctggctgcgggcgcgggtcgcccgcttcagcagcggggaggcgcacgtacggcgccgggcgctggcggtcggcccgctcggcgggggagacgcggccgacgcgctgcgcgacaccgcccgcgtacggacgcaagcgctgctggacggggcgggggtggggccgggatcggggccggggacggtggacgtgatggcgctggtggcgcgcgtcgtgcccgtcgaagtgcttgccgatttcgtcgggctgccggtcacggcggagacggccgggctggtcgggcacgtcgcccgcgcgtaccacgcacacggcgagaccgtcccggccgccgaccgcgccctcgcccggctcgtaacggtgtgcggcggtacgtgggacgaggccacggcggcccgcatcgggctgctggtgcaggcgtacgacgcgacggcggggctgatcggcaacgcggcgcatcggatgctgtcctgcgatacaggcgatacggggagtgcgagcggtacgggggatacgccggagggctccgccgagtctgccgccgatgtcgtcaccgcctcgctcgaccggacgctgagcgccgacccacccgtacggggcaccctccgcgcccctgcgaacggcggtgatccagtacggatcgccctgctcacggacgacggatcgctcgccttcggtgccggcccgcacgcctgccccgggcgcgcccacgcccgggcgctcgcggccggagtgctggacgcgctgctcgggcgcggctgccgcctcgtccggccggacctcgcgtacgagccgtccccgaacctgcgggtgccggtgcggctggaggtgacgtgcacataa

SEQ ID NO: 116 - protein, 304 aa, Streptomyces rimosus
MGPGALTDPDWVVPPVPQDVPEGGMAWLRARVARFSSGEAHVRRRALAVGPLGGGDAADALRDTARVRTQALLDGAGVGPGSGPGTVDVMALVARVVPVEVLADFVGLPVTAETAGLVGHVARAYHAHGETVPAADRALARLVTVCGGTWDEATAARIGLLVQAYDATAGLIGNAAHRMLSCDTGDTGSASGTGDTPEGSAESAADVVTASLDRTLSADPPVRGTLRAPANGGDPVRIALLTDDGSLAFGAGPHACPGRAHARALAAGVLDALLGRGCRLVRPDLAYEPSPNLRVPVRLEVTCT

SEQ ID NO: 117 - DNA, 1146 bp, Streptomyces rimosus
atggacaatccctaccccctgtaccggcggctgcgcgaaacctcccccgttctgtgggatcccgtacgccatcactggaccgtcacccgccaccaggaagtcacccaggcactgcgctccccggccctgcacgccgtaccccgccgcctcggcccccgcacaccccccaccctgcgcctgctcaacagcgccatgctcgactccgatccgcccgagcacacccgccgccgtcgcgtcttcacccaagccttcaccccgcgcctgaccgcagacctcgcacccgccatcacccaccgcgtcgacgccctcctcgaccgcgtgcacgaaagcggccacatggacctcatcgaagacctggccactccactgcccctgcacgtcatcggccagctgctcggcatacccccgcaagaccgcccccgcctgcacgccggagcccgcggctacgcccgactgtggggcggcgacgacaccgaccagaccaccatcggccaagccgtcaccgacatcaccagagccatcgaccactgccgcgagctgatcacccagcgtcgcaacgctccccgctccgacctgatcagccgtctggcctcaccagccggccgggcgggctcgctcagcgacggcgaactggccgccaacctcttcatggtcttcaccgcaggccactacacgaccaccgacttcctgggaaactccgtcctcgcactggcacaccacccgcaccagtggcaacaactgtgcacggacccggcactggcctcctcggccgtcaccgaactgctgcgctacgaagcccccgtccagttcgtcatccgcctggccgcacaagacctcaccctcgccggccagcgcatcacagccggccagctcgtcgtccttctgctcgccgcagcgaaccgcgacccacgggccttccccgaccccgaccgcctcgacctcacacgcactcccaaccaccacctcaccctcggcttcggcatccactcctgcctgggcaccgccctggcccggctccaaggcgagatcaccctgagccgcctggccgcccgcatgccccgtctccgcccggccggcgacaccatccgctggaagaccaccaccggactccgcggacctctccgtctatccgtccactgggactaa

SEQ ID NO: 118 - protein, 381 aa, Streptomyces rimosus
MDNPYPLYRRLRETSPVLWDPVRHHWTVTRHQEVTQALRSPALHAVPRRLGPRTPPTLRLLNSAMLDSDPPEHTRRRRVFTQAFTPRLTADLAPAITHRVDALLDRVHESGHMDLIEDLATPLPLHVIGQLLGIPPQDRPRLHAGARGYARLWGGDDTDQTTIGQAVTDITRAIDHCRELITQRRNAPRSDLISRLASPAGRAGSLSDGELAANLFMVFTAGHYTTTDFLGNSVLALAHHPHQWQQLCTDPALASSAVTELLRYEAPVQFVIRLAAQDLTLAGQRITAGQLVVLLLAAANRDPRAFPDPDRLDLTRTPNHHLTLGFGIHSCLGTALARLQGEITLSRLAARMPRLRPAGDTIRWKTTTGLRGPLRLSVHWD

SEQ ID NO: 119 - DNA, 57 bp, Synthetic Sequence
attttgtttaactttaagaaggagatatacatatgaccgagacgatcccgttcgaag

SEQ ID NO: 120 - DNA, 60 bp, Synthetic Sequence
gtggtggtggtggtggtgctcgagtgcggccgctaattaccccgtcacatagacatcctc

SEQ ID NO: 121 - DNA, 57 bp, Synthetic Sequence
attttgtttaactttaagaaggagatatacatatgaccggcgtatccgcccgcgaac

SEQ ID NO: 122 - DNA, 68 bp, Synthetic Sequence
cgatccgcactcacccgcatggtcatgaattctgtttcctataattaccaggcgaccggcagggattc

SEQ ID NO: 123 - DNA, 59 bp, Synthetic Sequence
attttgtttaactttaagaaggagatatacatatgccggacgagtcccagcaccagttc

SEQ ID NO: 124 - DNA, 62 bp, Synthetic Sequence
ctacccgcagagggcggggcataagcttcctattacgtacccgggccgtccgcctcccgctc

SEQ ID NO: 125 - DNA, 58 bp, Synthetic Sequence
attttgtttaactttaagaaggagatatacatatggcgagccgtacccgtatcgatac

SEQ ID NO: 126 - DNA, 71 bp, Synthetic Sequence
cgatccgcactcacccgcatggtcatgaattctgtttcctataattagccgcgcggggtgagcgccagatc

SEQ ID NO: 127 - DNA, 59 bp, Synthetic Sequence
attttgtttaactttaagaaggagatatacatatgtcgtacaacccgacggcccccgac

SEQ ID NO: 128 - DNA, 57 bp, Synthetic Sequence
ctacccgcagagggcggggcataagcttcctattacgggtccgtgggttccggggag

SEQ ID NO: 129 - DNA, 54 bp, Synthetic Sequence
attttgtttaactttaagaaggagatatacatatgagcgacccggccgcggtac

SEQ ID NO: 130 - DNA, 68 bp, Synthetic Sequence
cgatccgcactcacccgcatggtcatgaattctgtttcctataattacgacaggagcaggggcagctc

SEQ ID NO: 131 - DNA, 70 bp, Synthetic Sequence
attttgtttaactttaagaaggagatatacatatggacatcgatggcgcggagcccggcggcggcccttc

SEQ ID NO: 132 - DNA, 71 bp, Synthetic Sequence
cgatccgcactcacccgcatggtcatgaattctgtttcctataattatgaaccgccgggcgggccgaggac

SEQ ID NO: 133 - DNA, 54 bp, Synthetic Sequence
attttgtttaactttaagaaggagatatacatatggctgagtccacccacactg

SEQ ID NO: 134 - DNA, 70 bp, Synthetic Sequence
cgatccgcactcacccgcatggtcatgaattctgtttcctataattacacatcccaggcgaccggaagac

SEQ ID NO: 135 - DNA, 61 bp, Synthetic Sequence
attttgtttaactttaagaaggagatatacatatgaccccctctcccgcttcccccgccac

SEQ ID NO: 136 - DNA, 68 bp, Synthetic Sequence
gtggtggtggtggtggtgctcgagtgcggccgctaattacgcgcgggcgttgtgcagcccctcgcgag

SEQ ID NO: 137 - DNA, 63 bp, Synthetic Sequence
attttgtttaactttaagaaggagatatacatatgaccctcaccacacgatccggcccggcga

SEQ ID NO: 138 - DNA, 89 bp, Synthetic Sequence
cgatccgcactcacccgcatggtcatgaattctgtttcctataattagcccactcccctcagccgcacccgcgccgggcccgccgcctg

SEQ ID NO: 139 - DNA, 67 bp, Synthetic Sequence
attttgtttaactttaagaaggagatatacatatgacgcacaccgaaccggccgcgccggccacctg

SEQ ID NO: 140 - DNA, 63 bp, Synthetic Sequence
ctacccgcagagggcggggcataagcttcctattagccctcgtgcacggtgatggccccggac

SEQ ID NO: 141 - DNA, 59 bp, Synthetic Sequence
attttgtttaactttaagaaggagatatacatatgaccgaggcgctgcccttcccgcag

SEQ ID NO: 142 - DNA, 62 bp, Synthetic Sequence
ctacccgcagagggcggggcataagcttcctattagtcgtccgtgaccgcgatcgcctgaac

SEQ ID NO: 143 - DNA, 62 bp, Synthetic Sequence
attttgtttaactttaagaaggagatatacatatgaccgcggccgcgcaggaactggaaatc

SEQ ID NO: 144 - DNA, 73 bp, Synthetic Sequence
cgatccgcactcacccgcatggtcatgaattctgtttcctataattaccaggtgaccgggaatgcgtggatac

SEQ ID NO: 145 - DNA, 68 bp, Synthetic Sequence
attttgtttaactttaagaaggagatatacatatgaccgagacctccaccgccttcccggcccaagac

SEQ ID NO: 146 - DNA, 72 bp, Synthetic Sequence
ctacccgcagagggcggggcataagcttcctattactccgtgacccgaagggccccggacgggcacagcatg

SEQ ID NO: 147 - DNA, 59 bp, Synthetic Sequence
attttgtttaactttaagaaggagatatacatatggctgcacacgccgatgagccgatc

SEQ ID NO: 148 - DNA, 75 bp, Synthetic Sequence
cgatccgcactcacccgcatggtcatgaattctgtttcctataattatgtgacgctcctttgcgcgtgggggatg

SEQ ID NO: 149 - DNA, 62 bp, Synthetic Sequence
attttgtttaactttaagaaggagatatacatatgccgggcgccttgcccctcgtcgggcac

SEQ ID NO: 150 - DNA, 76 bp, Synthetic Sequence
cgatccgcactcacccgcatggtcatgaattctgtttcctataattagttgctcggccggctgggtgcggggttac

SEQ ID NO: 151 - DNA, 59 bp, Synthetic Sequence
attttgtttaactttaagaaggagatatacatatgccggtccagctccccggcggcatc

SEQ ID NO: 152 - DNA, 72 bp, Synthetic Sequence
cgatccgcactcacccgcatggtcatgaattctgtttcctataattacccggcgccggggctggtggccgac

SEQ ID NO: 153 - DNA, 66 bp, Synthetic Sequence
attttgtttaactttaagaaggagatatacatatgacgaccgttcccgatcttcccgacgccacag

SEQ ID NO: 154 - DNA, 71 bp, Synthetic Sequence
cgatccgcactcacccgcatggtcatgaattctgtttcctataattattccgggtcgccctgccaggtcac

SEQ ID NO: 155 - DNA, 62 bp, Synthetic Sequence
attttgtttaactttaagaaggagatatacatatgcagaacaccgccgagaccggccccgac

SEQ ID NO: 156 - DNA, 72 bp, Synthetic Sequence
cgatccgcactcacccgcatggtcatgaattctgtttcctataattaccaggcgacggggagcgagatcaag

SEQ ID NO: 157 - DNA, 53 bp, Synthetic Sequence
attttgtttaactttaagaaggagatatacatatgccggaaatcatcgacctg

SEQ ID NO: 158 - DNA, 68 bp, Synthetic Sequence
cgatccgcactcacccgcatggtcatgaattctgtttcctataattaccgccaccgcaccggcaggtg

SEQ ID NO: 159 - DNA, 61 bp, Synthetic Sequence
attttgtttaactttaagaaggagatatacatatgtcagtgccgagccgcccgccggccac

SEQ ID NO: 160 - DNA, 72 bp, Synthetic Sequence
cgatccgcactcacccgcatggtcatgaattctgtttcctataattagagttggaaagtgatccgttcggtg

SEQ ID NO: 161 - DNA, 58 bp, Synthetic Sequence
attttgtttaactttaagaaggagatatacatatgaccacatcgcccaccgagtccac

SEQ ID NO: 162 - DNA, 74 bp, Synthetic Sequence
cgatccgcactcacccgcatggtcatgaattctgtttcctataattagtcctccggacgcagccgcaacggcag

SEQ ID NO: 163 - DNA, 59 bp, Synthetic Sequence
attttgtttaactttaagaaggagatatacatatgaccgccgagaaccacaccgcgcag

SEQ ID NO: 164 - DNA, 75 bp, Synthetic Sequence
cgatccgcactcacccgcatggtcatgaattctgtttcctataattaccacgccaccggaatctccgccgccatg

SEQ ID NO: 165 - DNA, 59 bp, Synthetic Sequence
attttgtttaactttaagaaggagatatacatatgccgcaggacacctcccgccggttc

SEQ ID NO: 166 - DNA, 71 bp, Synthetic Sequence
cgatccgcactcacccgcatggtcatgaattctgtttcctataattaccacaccacaggcagcctcaccac

SEQ ID NO: 167 - DNA, 63 bp, Synthetic Sequence
attttgtttaactttaagaaggagatatacatatggatgagtcgcccgtcttcgtcctggatc

SEQ ID NO: 168 - DNA, 80 bp, Synthetic Sequence
cgatccgcactcacccgcatggtcatgaattctgtttcctataattatccccctgcttccccggccggcgcggagcggag

SEQ ID NO: 169 - DNA, 60 bp, Synthetic Sequence
attttgtttaactttaagaaggagatatacatatggagactgccccgctccgccccgtac

SEQ ID NO: 170 - DNA, 72 bp, Synthetic Sequence
cgatccgcactcacccgcatggtcatgaattctgtttcctataattacggacgcgaacgagcgcgcaccgtg

SEQ ID NO: 171 - DNA, 61 bp, Synthetic Sequence
attttgtttaactttaagaaggagatatacatatgcgcgatccggtccgctacttcgagac

SEQ ID NO: 172 - DNA, 74 bp, Synthetic Sequence
cgatccgcactcacccgcatggtcatgaattctgtttcctataattaccccgcgtcgtccgaaagagccggatg

SEQ ID NO: 173 - DNA, 58 bp, Synthetic Sequence
attttgtttaactttaagaaggagatatacatatgttcacaccccgcacgtacgccac

SEQ ID NO: 174 - DNA, 78 bp, Synthetic Sequence
cgatccgcactcacccgcatggtcatgaattctgtttcctataattacgcccccacccgcaccggcaaccgccgcaac

SEQ ID NO: 175 - DNA, 65 bp, Synthetic Sequence
attttgtttaactttaagaaggagatatacatatgaccacggacgacgacgaagaagaggatcag

SEQ ID NO: 176 - DNA, 71 bp, Synthetic Sequence
cgatccgcactcacccgcatggtcatgaattctgtttcctataattaccatgcgacgggcaacgattccag

SEQ ID NO: 177 - DNA, 62 bp, Synthetic Sequence
attttgtttaactttaagaaggagatatacatatgttgatgccgctgcggcgtcaggggctg

SEQ ID NO: 178 - DNA, 72 bp, Synthetic Sequence
cgatccgcactcacccgcatggtcatgaattctgtttcctataattagccgccgaggtgcaccggcagcgac

SEQ ID NO: 179 - DNA, 58 bp, Synthetic Sequence
attttgtttaactttaagaaggagatatacatatgctcggcgacgcccggttcagctc

SEQ ID NO: 180 - DNA, 71 bp, Synthetic Sequence
cgatccgcactcacccgcatggtcatgaattctgtttcctataattaccaagtgaccgggagtgccgatac

SEQ ID NO: 181 - DNA, 62 bp, Synthetic Sequence
attttgtttaactttaagaaggagatatacatatggacacacaccccgaacccatcgattac

SEQ ID NO: 182 - DNA, 72 bp, Synthetic Sequence
cgatccgcactcacccgcatggtcatgaattctgtttcctataattaccaggtgaccggcagctcctcgatc

SEQ ID NO: 183 - DNA, 59 bp, Synthetic Sequence
attttgtttaactttaagaaggagatatacatatgacgcagccggacaccaggacgaac

SEQ ID NO: 184 - DNA, 71 bp, Synthetic Sequence
cgatccgcactcacccgcatggtcatgaattctgtttcctataattaccaggcgacgggcagcgcgtccag

SEQ ID NO: 185 - DNA, 57 bp, Synthetic Sequence
attttgtttaactttaagaaggagatatacatatgccggacgccggacgtctccctc

SEQ ID NO: 186 - DNA, 75 bp, Synthetic Sequence
cgatccgcactcacccgcatggtcatgaattctgtttcctataattacggagtgagcgtcccgccatcgggcctg

SEQ ID NO: 187 - DNA, 59 bp, Synthetic Sequence
attttgtttaactttaagaaggagatatacatatggagtcaccggagttcttccgcgac

SEQ ID NO: 188 - DNA, 72 bp, Synthetic Sequence
cgatccgcactcacccgcatggtcatgaattctgtttcctataattaacaatccgtgacctgtgcggaccag

SEQ ID NO: 189 - DNA, 69 bp, Synthetic Sequence
attttgtttaactttaagaaggagatatacatatgaagtcgtccgcgacgcggtccggggccggcggac

SEQ ID NO: 190 - DNA, 73 bp, Synthetic Sequence
cgatccgcactcacccgcatggtcatgaattctgtttcctataattacctccttccggagctgttggcacgtg

SEQ ID NO: 191 - DNA, 57 bp, Synthetic Sequence
attttgtttaactttaagaaggagatatacatatgcgcccaccccgcctacccgaac

SEQ ID NO: 192 - DNA, 70 bp, Synthetic Sequence
cgatccgcactcacccgcatggtcatgaattctgtttcctataattatcgggtggcggcctctccggcag

SEQ ID NO: 193 - DNA, 56 bp, Synthetic Sequence
attttgtttaactttaagaaggagatatacatatggaaggagtccaggcagtcttc

SEQ ID NO: 194 - DNA, 71 bp, Synthetic Sequence
cgatccgcactcacccgcatggtcatgaattctgtttcctataattacaccgcgaccagcagctcgcgcag

SEQ ID NO: 195 - DNA, 55 bp, Synthetic Sequence
attttgtttaactttaagaaggagatatacatatgcagatcgtcgtggacctcac

SEQ ID NO: 196 - DNA, 66 bp, Synthetic Sequence
gtggtggtggtggtggtgctcgagtgcggccgctaattaccctttatttcgaggcgacgccaaatc

SEQ ID NO: 197 - DNA, 59 bp, Synthetic Sequence
attttgtttaactttaagaaggagatatacatatgtccggccacggaccggcggccgtc

SEQ ID NO: 198 - DNA, 71 bp, Synthetic Sequence
cgatccgcactcacccgcatggtcatgaattctgtttcctataattacttccgtacgggcgtgaactccac

SEQ ID NO: 199 - DNA, 56 bp, Synthetic Sequence
attttgtttaactttaagaaggagatatacatatgccatgccccgcgctgcccgac

SEQ ID NO: 200 - DNA, 72 bp, Synthetic Sequence
cgatccgcactcacccgcatggtcatgaattctgtttcctataattacacgtaccggacccgcagctccttc

SEQ ID NO: 201 - DNA, 62 bp, Synthetic Sequence
attttgtttaactttaagaaggagatatacatatggacgcgcgggtccgccacagccccgag

SEQ ID NO: 202 - DNA, 71 bp, Synthetic Sequence
cgatccgcactcacccgcatggtcatgaattctgtttcctataattaggagaccaccgcgtgccggggctg

SEQ ID NO: 203 - DNA, 75 bp, Synthetic Sequence
attttgtttaactttaagaaggagatatacatatgggtatacgtggtgcggcgggcgtccgcgcggcccgcggtc

SEQ ID NO: 204 - DNA, 83 bp, Synthetic Sequence
cgatccgcactcacccgcatggtcatgaattctgtttcctataattacggtgcttcagatggcacggccggcgctgggccgtc

SEQ ID NO: 205 - DNA, 60 bp, Synthetic Sequence
attttgtttaactttaagaaggagatatacatatgggtacgcacattcctggacccgaac

SEQ ID NO: 206 - DNA, 76 bp, Synthetic Sequence
cgatccgcactcacccgcatggtcatgaattctgtttcctataattacgggctccccgcccccacctcccgccgac

SEQ ID NO: 207 - DNA, 59 bp, Synthetic Sequence
attttgtttaactttaagaaggagatatacatatgaccaccccccagcaccccgacgac

SEQ ID NO: 208 - DNA, 72 bp, Synthetic Sequence
cgatccgcactcacccgcatggtcatgaattctgtttcctataattaccggaaggccagctccccccggaag

SEQ ID NO: 209 - DNA, 64 bp, Synthetic Sequence
attttgtttaactttaagaaggagatatacatatgactttcccttttcccgaacagcccggcac

SEQ ID NO: 210 - DNA, 78 bp, Synthetic Sequence
cgatccgcactcacccgcatggtcatgaattctgtttcctataattagccgcgcagccaagccttcaacgcggcccac

SEQ ID NO: 211 - DNA, 59 bp, Synthetic Sequence
attttgtttaactttaagaaggagatatacatatgctggaacagctgcgcaggcagtac

SEQ ID NO: 212 - DNA, 73 bp, Synthetic Sequence
cgatccgcactcacccgcatggtcatgaattctgtttcctataattaggcagtaccaaccgacctacccactc

SEQ ID NO: 213 - DNA, 62 bp, Synthetic Sequence
attttgtttaactttaagaaggagatatacatatgaacaccctccgcaccgccaagctgctc

SEQ ID NO: 214 - DNA, 95 bp, Synthetic Sequence
cgatccgcactcacccgcatggtcatgaattctgtttcctataattaggcgtgcgggtacggacagcgcgccggggcgggggcggtgcccggcag

SEQ ID NO: 215 - DNA, 58 bp, Synthetic Sequence
attttgtttaactttaagaaggagatatacatatgcgtacgtacggtacggaacggag

SEQ ID NO: 216 - DNA, 72 bp, Synthetic Sequence
cgatccgcactcacccgcatggtcatgaattctgtttcctataattagcgccgtacgaccgacacccgcgac

SEQ ID NO: 217 - DNA, 71 bp, Synthetic Sequence
attttgtttaactttaagaaggagatatacatatgaccacagccgacacgatgccccttgcctacccgttc

SEQ ID NO: 218 - DNA, 65 bp, Synthetic Sequence
ctacccgcagagggcggggcataagcttcctattagggccgcggccccaccaccttctccccgtc

SEQ ID NO: 219 - DNA, 56 bp, Synthetic Sequence
attttgtttaactttaagaaggagatatacatatggcgtggctccaggacgcggac

SEQ ID NO: 220 - DNA, 68 bp, Synthetic Sequence
cgatccgcactcacccgcatggtcatgaattctgtttcctataattaccagctgaccggaagggtgag

SEQ ID NO: 221 - DNA, 57 bp, Synthetic Sequence
attttgtttaactttaagaaggagatatacatatgagccaccccgaagccctcatac

SEQ ID NO: 222 - DNA, 73 bp, Synthetic Sequence
cgatccgcactcacccgcatggtcatgaattctgtttcctataattaccagcgcacggggagccgggccggtg

SEQ ID NO: 223 - DNA, 56 bp, Synthetic Sequence
attttgtttaactttaagaaggagatatacatatgggcccgggcgcgctcaccgac

SEQ ID NO: 224 - DNA, 71 bp, Synthetic Sequence
cgatccgcactcacccgcatggtcatgaattctgtttcctataattatgtgcacgtcacctccagccgcac

SEQ ID NO: 225 - DNA, 56 bp, Synthetic Sequence
attttgtttaactttaagaaggagatatacatatggacaatccctaccccctgtac

SEQ ID NO: 226 - DNA, 67 bp, Synthetic Sequence
cgatccgcactcacccgcatggtcatgaattctgtttcctataattagtcccagtggacggatagac

SEQ ID NO: 227 - DNA, 53 bp, Synthetic Sequence
gggtcctcaacgacaggagcacgatcatgccggaaatacaggaacgcacgctg

SEQ ID NO: 228 - DNA, 56 bp, Synthetic Sequence
ttatcgccggcatggcggccccacgggtgccggggcacaactcaatttgcgggtac

SEQ ID NO: 229 - DNA, 1451 bp, Synthetic Sequence
catatgaccgaagcactgcctttcccacaagaccgcacctgtccgtacgacccaccggctggctaccagccgctgagagatagccgtccactgagccgtgttacgttgtatgatggccgtccggcgtgggtcgtgacgggccacgcagagagccgtgcactgctgacggacccgcgcttgtcggctgatcgccagaacccggcgttcccgtccccggctccgcgttttgagactctgcgtaaggtccgtaccccgctgctgggcgtggacgatccggagcacaatacgcagcgtcgtatgttgattccgtccttcagcgtgaagcgtgcagcagcactgcgcccgcgtatccaagaaatcgtggatcgcctgttggacgctatggaacagcaaggtcctccggcggaactggtttctgcgttcgcactgccggtcccgagcatggtcatctgcgccttgctgggtgtcccgtacgctgaccatgaactgtttgagggcctgagccgtactctgctgcagagcgcagacccgcaagaggtcaccgaagcccgcgataaactggaagattactttaccgcactggtggagcgtaagcgcaaagaaccgggtgacggtctgctggatgaactgattgcggagcgcctggacagcggcgagctgggccatcgtgaactggtccgtatggcgatgctgctgctggttgcgggtcatgaaaccacctccaacatgttgagcctgggcacgttcaccctgctggagcacccggagcaatttgcggcgctgcgcgctgatcctagcctgctgccggcggcagtggaagaattgctgcgtttcctgtctatcgccgacggcatggttcgtgttgcgaccgaagatatcgagatcggtggcgttacgattcgcgcggatgatggtgtgatcttcagcacgagcgtggttaatcgcgacggtgcggcgtatgcctcaccggataccctggactgggagcgtagcgcgcgtcaccatgtcgcttttggtttcggtgttcaccagtgcctgggtcagaacctggcccgtgccgagatggaaattgcatttggtgcgttattcgcccgttttccgggtctgcgtcttgcagtgcctgcggccgagattccggtgaaaccggcgcacgcgttgcaaggtctggttgagctgccggtgacctggtgataacggcggaccgccgcccacaccctgtacccgtcaacggaggagagaaaaaatgaaaattgacattgacacgagcgtttgtatcggtagcggccaatgtgttctgactgccccgggtgtttttacccaagatgatgatggtttcagcacgctgctgccgggtcgcgaagatggtacgggcgacccattagttcgtgaagccgcgcgcgcgtgcccggtgcaagcaatcgcggtgaccgacgactaataataggaagctt

SEQ ID NO: 230 - DNA, 1188 bp, Streptomyces rimosus
atgaccgaagcactgcctttcccacaagaccgcacctgtccgtacgacccaccggctggctaccagccgctgagagatagccgtccactgagccgtgttacgttgtatgatggccgtccggcgtgggtcgtgacgggccacgcagagagccgtgcactgctgacggacccgcgcttgtcggctgattggcagaacccggcgttcccgtccccggctccgcgttttgagactctgcgtaaggtccgtaccccgctgctgggcgtggacgatccggagcacaatacgcagcgtcgtatgttgattccgtccttcagcgtgaagcgtgcagcagcactgcgcccgcgtatccaagaaatcgtggatcgcctgttggacgctatggaacagcaaggtcctccggcggaactggtttctgcgttcgcactgccggtcccgagcatggtcatctgcgccttgctgggtgtcccgtacgctgaccatgaactgtttgagggcctgagccgtactctgctgcagagcgcagacccgcaagaggtcaccgaagcccgcgataaactggaagattactttaccgcactggtggagcgtaagcgcaaagaaccgggtgacggtctgctggatgaactgattgcggagcgcctggacagcggcgagctgggccatcgtgaactggtccgtatggcgatgctgctgctggttgcgggtcatgaaaccacctccaacatgttgagcctgggcacgttcaccctgctggagcacccggagcaatttgcggcgctgcgcgctgatcctagcctgctgccggcggcagtggaagaattgctgcgtttcctgtctatcgccgacggcatggttcgtgttgcgaccgaagatatcgagatcggtggcgttacgattcgcgcggatgatggtgtgatcttcagcacgagcgtggttaatcgcgacggtgcggcgtatgcctcaccggataccctggactgggagcgtagcgcgcgtcaccatgtcgcttttggtttcggtgttcaccagtgcctgggtcagaacctggcccgtgccgagatggaaattgcatttggtgcgttattcgcccgttttccgggtctgcgtcttgcagtgcctgcggccgagattccggtgaaaccggcgcacgcgttgcaaggtctggttgagctgccggtgacctggtga

SEQ ID NO: 231 - protein, 395 aa, Streptomyces rimosus
MTEALPFPQDRTCPYDPPAGYQPLRDSRPLSRVTLYDGRPAWVVTGHAESRALLTDPRLSADWQNPAFPSPAPRFETLRKVRTPLLGVDDPEHNTQRRMLIPSFSVKRAAALRPRIQEIVDRLLDAMEQQGPPAELVSAFALPVPSMVICALLGVPYADHELFEGLSRTLLQSADPQEVTEARDKLEDYFTALVERKRKEPGDGLLDELIAERLDSGELGHRELVRMAMLLLVAGHETTSNMLSLGTFTLLEHPEQFAALRADPSLLPAAVEELLRFLSIADGMVRVATEDIEIGGVTIRADDGVIFSTSVVNRDGAAYASPDTLDWERSARHHVAFGFGVHQCLGQNLARAEMEIAFGALFARFPGLRLAVPAAEIPVKPAHALQGLVELPVTW

SEQ ID NO: 232 - DNA, 1188 bp, Streptomyces rimosus
atgaccgaagcactgcctttcccacaagaccgcacctgtccgtacgacccaccggctggctaccagccgctgagagatagccgtccactgagccgtgttacgttgtatgatggccgtccggcgtgggtcgtgacgggccacgcagagagccgtgcactgctgacggacccgcgcttgtcggctgattatcagaacccggcgttcccgtccccggctccgcgttttgagactctgcgtaaggtccgtaccccgctgctgggcgtggacgatccggagcacaatacgcagcgtcgtatgttgattccgtccttcagcgtgaagcgtgcagcagcactgcgcccgcgtatccaagaaatcgtggatcgcctgttggacgctatggaacagcaaggtcctccggcggaactggtttctgcgttcgcactgccggtcccgagcatggtcatctgcgccttgctgggtgtcccgtacgctgaccatgaactgtttgagggcctgagccgtactctgctgcagagcgcagacccgcaagaggtcaccgaagcccgcgataaactggaagattactttaccgcactggtggagcgtaagcgcaaagaaccgggtgacggtctgctggatgaactgattgcggagcgcctggacagcggcgagctgggccatcgtgaactggtccgtatggcgatgctgctgctggttgcgggtcatgaaaccacctccaacatgttgagcctgggcacgttcaccctgctggagcacccggagcaatttgcggcgctgcgcgctgatcctagcctgctgccggcggcagtggaagaattgctgcgtttcctgtctatcgccgacggcatggttcgtgttgcgaccgaagatatcgagatcggtggcgttacgattcgcgcggatgatggtgtgatcttcagcacgagcgtggttaatcgcgacggtgcggcgtatgcctcaccggataccctggactgggagcgtagcgcgcgtcaccatgtcgcttttggtttcggtgttcaccagtgcctgggtcagaacctggcccgtgccgagatggaaattgcatttggtgcgttattcgcccgttttccgggtctgcgtcttgcagtgcctgcggccgagattccggtgaaaccggcgcacgcgttgcaaggtctggttgagctgccggtgacctggtga

SEQ ID NO: 233 - protein, 395 aa, Streptomyces rimosus
MTEALPFPQDRTCPYDPPAGYQPLRDSRPLSRVTLYDGRPAWVVTGHAESRALLTDPRLSADYQNPAFPSPAPRFETLRKVRTPLLGVDDPEHNTQRRMLIPSFSVKRAAALRPRIQEIVDRLLDAMEQQGPPAELVSAFALPVPSMVICALLGVPYADHELFEGLSRTLLQSADPQEVTEARDKLEDYFTALVERKRKEPGDGLLDELIAERLDSGELGHRELVRMAMLLLVAGHETTSNMLSLGTFTLLEHPEQFAALRADPSLLPAAVEELLRFLSIADGMVRVATEDIEIGGVTIRADDGVIFSTSVVNRDGAAYASPDTLDWERSARHHVAFGFGVHQCLGQNLARAEMEIAFGALFARFPGLRLAVPAAEIPVKPAHALQGLVELPVTW

SEQ ID NO: 234 - DNA, 1188 bp, Streptomyces rimosus
atgaccgaagcactgcctttcccacaagaccgcacctgtccgtacgacccaccggctggctaccagccgctgagagatagccgtccactgagccgtgttacgttgtatgatggccgtccggcgtgggtcgtgacgggccacgcagagagccgtgcactgctgacggacccgcgcttgtcggctgatcgccagaacccggcgttcccgtccccggctccgcgttttgagactctgcgtaaggtccgtaccccgctgctgggcgtggacgatccggagcacaatacgcagcgtcgtatgttgattccgtccttcagcgtgaagcgtgcagcagcactgcgcccgcgtatccaagaaatcgtggatcgcctgttggacgctatggaacagcaaggtcctccggcggaactggtttctgcgttcgcactgccggtcccgagcatggtcatctgcgccttgctgggtgtcccgtacgctgaccatgaactgtttgagggcctgagccgtactctgattcagagcgcagacccgcaagaggtcaccgaagcccgcgataaactggaagattactttaccgcactggtggagcgtaagcgcaaagaaccgggtgacggtctgctggatgaactgattgcggagcgcctggacagcggcgagctgggccatcgtgaactggtccgtatggcgatgctgctgctggttgcgggtcatgaaaccacctccaacatgttgagcctgggcacgttcaccctgctggagcacccggagcaatttgcggcgctgcgcgctgatcctagcctgctgccggcggcagtggaagaattgctgcgtttcctgtctatcgccgacggcatggttcgtgttgcgaccgaagatatcgagatcggtggcgttacgattcgcgcggatgatggtgtgatcttcagcacgagcgtggttaatcgcgacggtgcggcgtatgcctcaccggataccctggactgggagcgtagcgcgcgtcaccatgtcgcttttggtttcggtgttcaccagtgcctgggtcagaacctggcccgtgccgagatggaaattgcatttggtgcgttattcgcccgttttccgggtctgcgtcttgcagtgcctgcggccgagattccggtgaaaccggcgcacgcgttgcaaggtctggttgagctgccggtgacctggtga

SEQ ID NO: 235 - protein, 395 aa, Streptomyces rimosus
MTEALPFPQDRTCPYDPPAGYQPLRDSRPLSRVTLYDGRPAWVVTGHAESRALLTDPRLSADRQNPAFPSPAPRFETLRKVRTPLLGVDDPEHNTQRRMLIPSFSVKRAAALRPRIQEIVDRLLDAMEQQGPPAELVSAFALPVPSMVICALLGVPYADHELFEGLSRTLIQSADPQEVTEARDKLEDYFTALVERKRKEPGDGLLDELIAERLDSGELGHRELVRMAMLLLVAGHETTSNMLSLGTFTLLEHPEQFAALRADPSLLPAAVEELLRFLSIADGMVRVATEDIEIGGVTIRADDGVIFSTSVVNRDGAAYASPDTLDWERSARHHVAFGFGVHQCLGQNLARAEMEIAFGALFARFPGLRLAVPAAEIPVKPAHALQGLVELPVTW

SEQ ID NO: 236 - DNA, 1188 bp, Streptomyces rimosus
atgaccgaagcactgcctttcccacaagaccgcacctgtccgtacgacccaccggctggctaccagccgctgagagatagccgtccactgagccgtgttacgttgtatgatggccgtccggcgtgggtcgtgacgggccacgcagagagccgtgcactgctgacggacccgcgcttgtcggctgatcgccagaacccggcgttcccgtccccggctccgcgttttgagactctgcgtaaggtccgtaccccgctgctgggcgtggacgatccggagcacaatacgcagcgtcgtatgttgattccgtccttcagcgtgaagcgtgcagcagcactgcgcccgcgtatccaagaaatcgtggatcgcctgttggacgctatggaacagcaaggtcctccggcggaactggtttctgcgttcgcactgccggtcccgagcatggtcatctgcgccttgctgggtgtcccgtacgctgaccatgaactgtttgagggcctgagccgtactctgctgcagagcgcagacccgcaagaggtcaccgaagcccgcgataaactggaagattactttaccgcactggtggagcgtaagcgcaaagaaccgggtgacggtctgctggatgaactgattgcggagcgcctggacagcggcgagctgggccatcgtgaactggtccgtatggcgatgattctgctggttgcgggtcatgaaaccacctccaacatgttgagcctgggcacgttcaccctgctggagcacccggagcaatttgcggcgctgcgcgctgatcctagcctgctgccggcggcagtggaagaattgctgcgtttcctgtctatcgccgacggcatggttcgtgttgcgaccgaagatatcgagatcggtggcgttacgattcgcgcggatgatggtgtgatcttcagcacgagcgtggttaatcgcgacggtgcggcgtatgcctcaccggataccctggactgggagcgtagcgcgcgtcaccatgtcgcttttggtttcggtgttcaccagtgcctgggtcagaacctggcccgtgccgagatggaaattgcatttggtgcgttattcgcccgttttccgggtctgcgtcttgcagtgcctgcggccgagattccggtgaaaccggcgcacgcgttgcaaggtctggttgagctgccggtgacctggtga

SEQ ID NO: 237 - protein, 395 aa, Streptomyces rimosus
MTEALPFPQDRTCPYDPPAGYQPLRDSRPLSRVTLYDGRPAWVVTGHAESRALLTDPRLSADRQNPAFPSPAPRFETLRKVRTPLLGVDDPEHNTQRRMLIPSFSVKRAAALRPRIQEIVDRLLDAMEQQGPPAELVSAFALPVPSMVICALLGVPYADHELFEGLSRTLLQSADPQEVTEARDKLEDYFTALVERKRKEPGDGLLDELIAERLDSGELGHRELVRMAMILLVAGHETTSNMLSLGTFTLLEHPEQFAALRADPSLLPAAVEELLRFLSIADGMVRVATEDIEIGGVTIRADDGVIFSTSVVNRDGAAYASPDTLDWERSARHHVAFGFGVHQCLGQNLARAEMEIAFGALFARFPGLRLAVPAAEIPVKPAHALQGLVELPVTW

SEQ ID NO: 238 - DNA, 23 bp, Synthetic Sequence
gtcggctgattggcagaacccgg

SEQ ID NO: 239 - DNA, 23 bp, Synthetic Sequence
ccgggttctggcgatcagccgac

SEQ ID NO: 240 - DNA, 23 bp, Synthetic Sequence
gtcggctgattatcagaacccgg

SEQ ID NO: 241 - DNA, 23 bp, Synthetic Sequence
ccgggttctgataatcagccgac

SEQ ID NO: 242 - DNA, 23 bp, Synthetic Sequence
cccggctccgtattttgagactc

SEQ ID NO: 243 - DNA, 23 bp, Synthetic Sequence
gagtctcaaaatacggagccggg

SEQ ID NO: 244 - DNA, 23 bp, Synthetic Sequence
ccgtactctggcgcagagcgcag

SEQ ID NO: 245 - DNA, 23 bp, Synthetic Sequence
ctgcgctctgcgccagagtacgg

SEQ ID NO: 246 - DNA, 23 bp, Synthetic Sequence
ccgtactctgattcagagcgcag

SEQ ID NO: 247 - DNA, 23 bp, Synthetic Sequence
caaccagcagaatcatcgccata

SEQ ID NO: 248 - DNA, 23 bp, Synthetic Sequence
tatggcgatgattctgctggttg

SEQ ID NO: 249 - DNA, 23 bp, Synthetic Sequence
catgacccgccagcagcagcagc

SEQ ID NO: 250 - DNA, 1188 bp, Streptomyces rimosus
atgaccgaagcactgcctttcccacaagaccgcacctgtccgtacgacccaccggctggctaccagccgctgagagatagccgtccactgagccgtgttacgttgtatgatggccgtccggcgtgggtcgtgacgggccacgcagagagccgtgcactgctgacggacccgcgcttgtcggctgattggcagaacccggcgttcccgtccccggctccgtattttgagactctgcgtaaggtccgtaccccgctgctgggcgtggacgatccggagcacaatacgcagcgtcgtatgttgattccgtccttcagcgtgaagcgtgcagcagcactgcgcccgcgtatccaagaaatcgtggatcgcctgttggacgctatggaacagcaaggtcctccggcggaactggtttctgcgttcgcactgccggtcccgagcatggtcatctgcgccttgctgggtgtcccgtacgctgaccatgaactgtttgagggcctgagccgtactctgctgcagagcgcagacccgcaagaggtcaccgaagcccgcgataaactggaagattactttaccgcactggtggagcgtaagcgcaaagaaccgggtgacggtctgctggatgaactgattgcggagcgcctggacagcggcgagctgggccatcgtgaactggtccgtatggcgatgctgctgctggttgcgggtcatgaaaccacctccaacatgttgagcctgggcacgttcaccctgctggagcacccggagcaatttgcggcgctgcgcgctgatcctagcctgctgccggcggcagtggaagaattgctgcgtttcctgtctatcgccgacggcatggttcgtgttgcgaccgaagatatcgagatcggtggcgttacgattcgcgcggatgatggtgtgatcttcagcacgagcgtggttaatcgcgacggtgcggcgtatgcctcaccggataccctggactgggagcgtagcgcgcgtcaccatgtcgcttttggtttcggtgttcaccagtgcctgggtcagaacctggcccgtgccgagatggaaattgcatttggtgcgttattcgcccgttttccgggtctgcgtcttgcagtgcctgcggccgagattccggtgaaaccggcgcacgcgttgcaaggtctggttgagctgccggtgacctggtga

SEQ ID NO: 251 - protein, 395 aa, Streptomyces rimosus
MTEALPFPQDRTCPYDPPAGYQPLRDSRPLSRVTLYDGRPAWVVTGHAESRALLTDPRLSADWQNPAFPSPAPYFETLRKVRTPLLGVDDPEHNTQRRMLIPSFSVKRAAALRPRIQEIVDRLLDAMEQQGPPAELVSAFALPVPSMVICALLGVPYADHELFEGLSRTLLQSADPQEVTEARDKLEDYFTALVERKRKEPGDGLLDELIAERLDSGELGHRELVRMAMLLLVAGHETTSNMLSLGTFTLLEHPEQFAALRADPSLLPAAVEELLRFLSIADGMVRVATEDIEIGGVTIRADDGVIFSTSVVNRDGAAYASPDTLDWERSARHHVAFGFGVHQCLGQNLARAEMEIAFGALFARFPGLRLAVPAAEIPVKPAHALQGLVELPVTW

SEQ ID NO: 252 - DNA, 1188 bp, Streptomyces rimosus
atgaccgaagcactgcctttcccacaagaccgcacctgtccgtacgacccaccggctggctaccagccgctgagagatagccgtccactgagccgtgttacgttgtatgatggccgtccggcgtgggtcgtgacgggccacgcagagagccgtgcactgctgacggacccgcgcttgtcggctgattggcagaacccggcgttcccgtccccggctccgcgttttgagactctgcgtaaggtccgtaccccgctgctgggcgtggacgatccggagcacaatacgcagcgtcgtatgttgattccgtccttcagcgtgaagcgtgcagcagcactgcgcccgcgtatccaagaaatcgtggatcgcctgttggacgctatggaacagcaaggtcctccggcggaactggtttctgcgttcgcactgccggtcccgagcatggtcatctgcgccttgctgggtgtcccgtacgctgaccatgaactgtttgagggcctgagccgtactctggcgcagagcgcagacccgcaagaggtcaccgaagcccgcgataaactggaagattactttaccgcactggtggagcgtaagcgcaaagaaccgggtgacggtctgctggatgaactgattgcggagcgcctggacagcggcgagctgggccatcgtgaactggtccgtatggcgatgctgctgctggttgcgggtcatgaaaccacctccaacatgttgagcctgggcacgttcaccctgctggagcacccggagcaatttgcggcgctgcgcgctgatcctagcctgctgccggcggcagtggaagaattgctgcgtttcctgtctatcgccgacggcatggttcgtgttgcgaccgaagatatcgagatcggtggcgttacgattcgcgcggatgatggtgtgatcttcagcacgagcgtggttaatcgcgacggtgcggcgtatgcctcaccggataccctggactgggagcgtagcgcgcgtcaccatgtcgcttttggtttcggtgttcaccagtgcctgggtcagaacctggcccgtgccgagatggaaattgcatttggtgcgttattcgcccgttttccgggtctgcgtcttgcagtgcctgcggccgagattccggtgaaaccggcgcacgcgttgcaaggtctggttgagctgccggtgacctggtga

SEQ ID NO: 253 - protein, 395 aa, Streptomyces rimosus
MTEALPFPQDRTCPYDPPAGYQPLRDSRPLSRVTLYDGRPAWVVTGHAESRALLTDPRLSADWQNPAFPSPAPRFETLRKVRTPLLGVDDPEHNTQRRMLIPSFSVKRAAALRPRIQEIVDRLLDAMEQQGPPAELVSAFALPVPSMVICALLGVPYADHELFEGLSRTLAQSADPQEVTEARDKLEDYFTALVERKRKEPGDGLLDELIAERLDSGELGHRELVRMAMLLLVAGHETTSNMLSLGTFTLLEHPEQFAALRADPSLLPAAVEELLRFLSIADGMVRVATEDIEIGGVTIRADDGVIFSTSVVNRDGAAYASPDTLDWERSARHHVAFGFGVHQCLGQNLARAEMEIAFGALFARFPGLRLAVPAAEIPVKPAHALQGLVELPVTW

SEQ ID NO: 254 - DNA, 1188 bp, Streptomyces rimosus
atgaccgaagcactgcctttcccacaagaccgcacctgtccgtacgacccaccggctggctaccagccgctgagagatagccgtccactgagccgtgttacgttgtatgatggccgtccggcgtgggtcgtgacgggccacgcagagagccgtgcactgctgacggacccgcgcttgtcggctgatcgccagaacccggcgttcccgtccccggctccgtattttgagactctgcgtaaggtccgtaccccgctgctgggcgtggacgatccggagcacaatacgcagcgtcgtatgttgattccgtccttcagcgtgaagcgtgcagcagcactgcgcccgcgtatccaagaaatcgtggatcgcctgttggacgctatggaacagcaaggtcctccggcggaactggtttctgcgttcgcactgccggtcccgagcatggtcatctgcgccttgctgggtgtcccgtacgctgaccatgaactgtttgagggcctgagccgtactctggcgcagagcgcagacccgcaagaggtcaccgaagcctgggataaactggaagattactttaccgcactggtggagcgtaagcgcaaagaaccgggtgacggtctgctggatgaactgattgcggagcgcctggacagcggcgagctgggccatcgtgaactggtccgtatggcgatgctgctgctggttgcgggtcatgaaaccacctccaacatgttgagcctgggcacgttcaccctgctggagcacccggagcaatttgcggcgctgcgcgctgatcctagcctgctgccggcggcagtggaagaattgctgcgtttcctgtctatcgccgacggcatggttcgtgttgcgaccgaagatatcgagatcggtggcgttacgattcgcgcggatgatggtgtgatcttcagcacgagcgtggttaatcgcgacggtgcggcgtatgcctcaccggataccctggactgggagcgtagcgcgcgtcaccatgtcgcttttggtttcggtgttcaccagtgcctgggtcagaacctggcccgtgccgagatggaaattgcatttggtgcgttattcgcccgttttccgggtctgcgtcttgcagtgcctgcggccgagattccggtgaaaccggcgcacgcgttgcaaggtctggttgagctgccggtgacctggtga

SEQ ID NO: 255 - protein, 395 aa, Streptomyces rimosus
MTEALPFPQDRTCPYDPPAGYQPLRDSRPLSRVTLYDGRPAWVVTGHAESRALLTDPRLSADRQNPAFPSPAPYFETLRKVRTPLLGVDDPEHNTQRRMLIPSFSVKRAAALRPRIQEIVDRLLDAMEQQGPPAELVSAFALPVPSMVICALLGVPYADHELFEGLSRTLAQSADPQEVTEAWDKLEDYFTALVERKRKEPGDGLLDELIAERLDSGELGHRELVRMAMLLLVAGHETTSNMLSLGTFTLLEHPEQFAALRADPSLLPAAVEELLRFLSIADGMVRVATEDIEIGGVTIRADDGVIFSTSVVNRDGAAYASPDTLDWERSARHHVAFGFGVHQCLGQNLARAEMEIAFGALFARFPGLRLAVPAAEIPVKPAHALQGLVELPVTW

SEQ ID NO: 256 - DNA, 1188 bp, Streptomyces rimosus
atgaccgaagcactgcctttcccacaagaccgcacctgtccgtacgacccaccggctggctaccagccgctgagagatagccgtccactgagccgtgttacgttgtatgatggccgtccggcgtgggtcgtgacgggccacgcagagagccgtgcactgctgacggacccgcgcttgtcggctgattggcagaacccggcgttcccgtccccggctccgtattttgagactctgcgtaaggtccgtaccccgctgctgggcgtggacgatccggagcacaatacgcagcgtcgtatgttgattccgtccttcagcgtgaagcgtgcagcagcactgcgcccgcgtatccaagaaatcgtggatcgcctgttggacgctatggaacagcaaggtcctccggcggaactggtttctgcgttcgcactgccggtcccgagcatggtcatctgcgccttgctgggtgtcccgtacgctgaccatgaactgtttgagggcctgagccgtactctggcgcagagcgcagacccgcaagaggtcaccgaagcccgcgataaactggaagattactttaccgcactggtggagcgtaagcgcaaagaaccgggtgacggtctgctggatgaactgattgcggagcgcctggacagcggcgagctgggccatcgtgaactggtccgtatggcgatgctgctgctggttgcgggtcatgaaaccacctccaacatgttgagcctgggcacgttcaccctgctggagcacccggagcaatttgcggcgctgcgcgctgatcctagcctgctgccggcggcagtggaagaattgctgcgtttcctgtctatcgccgacggcatggttcgtgttgcgaccgaagatatcgagatcggtggcgttacgattcgcgcggatgatggtgtgatcttcagcacgagcgtggttaatcgcgacggtgcggcgtatgcctcaccggataccctggactgggagcgtagcgcgcgtcaccatgtcgcttttggtttcggtgttcaccagtgcctgggtcagaacctggcccgtgccgagatggaaattgcatttggtgcgttattcgcccgttttccgggtctgcgtcttgcagtgcctgcggccgagattccggtgaaaccggcgcacgcgttgcaaggtctggttgagctgccggtgacctggtga

SEQ ID NO: 257 - protein, 395 aa, Streptomyces rimosus
MTEALPFPQDRTCPYDPPAGYQPLRDSRPLSRVTLYDGRPAWVVTGHAESRALLTDPRLSADWQNPAFPSPAPYFETLRKVRTPLLGVDDPEHNTQRRMLIPSFSVKRAAALRPRIQEIVDRLLDAMEQQGPPAELVSAFALPVPSMVICALLGVPYADHELFEGLSRTLAQSADPQEVTEARDKLEDYFTALVERKRKEPGDGLLDELIAERLDSGELGHRELVRMAMLLLVAGHETTSNMLSLGTFTLLEHPEQFAALRADPSLLPAAVEELLRFLSIADGMVRVATEDIEIGGVTIRADDGVIFSTSVVNRDGAAYASPDTLDWERSARHHVAFGFGVHQCLGQNLARAEMEIAFGALFARFPGLRLAVPAAEIPVKPAHALQGLVELPVTW